European Patent Application EP 4 215 608 A1, published July 26, 2023. Title: Targeted Deaminase and Base Editing Using the Same. Applicant: Institute for Basic Science. The sequence listing filed with the application follows.

SEQUENCE LISTING (571 sequences)

SEQ ID NO: 1 - protein, 138 aa, Artificial Sequence
  Deaminase
GSYALGPYQISAPQLPAYNGQTVGTFYYVNDAGGLESKVFSSGGPTPYPNYANAGHVEGQSALFMRDNGISEGLVFHNNPEGTCGFCVNMTETLLPENAKMTVVPPEGAIPVKRGATGETKVFTGNSNSPKSPTKGGC

SEQ ID NO: 2 - protein, 123 aa, Artificial Sequence
  Zinc Finger Protein
GIHGVPAAMAERPFQCRICMRNFSDRSNLSRHIRTHTGEKPFACDICGRKFAISSNLNSHTKIHTGSQKPFQCRICMRNFSRSDNLARHIRTHTGEKPFACDICGRKFATSGNLTRHTKIHLR

SEQ ID NO: 3 - protein, 122 aa, Artificial Sequence
  Zinc Finger Protein
GIHGVPAAMAERPFQCRICMRNFSRSDNLSVHIRTHTGEKPFACDICGRKFAQKINLQVHTKIHTGEKPFQCRICMRNFSRSDVLSEHIRTHTGEKPFACDICGRKFAQRNHRTTHTKIHLR

SEQ ID NO: 4 - DNA, 408 bp, Artificial Sequence
  TALE
gatatagctgatttgaggaccctcgggtactcacagcagcaacaagaaaaaatcaaaccaaaggtacgtagcacggttgcccaacatcatgaagccctagttggtcacggatttactcatgcccatattgttgcactgagtcaacaccctgctgcattaggcacagtggctgtgaaatatcaagatatgattgctgctcttcctgaggccacacacgaggcaattgtgggtgttggaaaacaatggtctggtgcgcgagcgcttgaagctctcctaaccgtagctggagagttgagaggcccaccgcttcagcttgacacagggcagctgttgaagatagcaaagagggggggtgtaactgctgttgaagcagtccatgcatggagaaatgcattaactggagctcca

SEQ ID NO: 5 - DNA, 411 bp, Artificial Sequence
  TALE
gatattgctgatcttcgaacattgggttattctcagcagcaacaagagaaaatcaaaccgaaagtccgttcaaccgtagctcaacatcatgaagcccttgttggtcatggatttactcatgctcacattgttgctctaagtcagcaccctgccgcgctaggcacagttgccgtcaagtatcaagatatgatagctgctttacctgaagcaacccacgaggcaatagtgggggttgggaagaggggtgcaggcgccagggcactggaggcactcttaacagtagctggagaacttcggggaccaccattgcagcttgatactggacaactcttgaagatcgcaaaaagagggggtgtgactgctgtggaagctgttcatgcatggagaaatgctttgacgggagcacccctg

SEQ ID NO: 6 - DNA, 123 bp, Artificial Sequence
  TALE
agcatagttgctcagctaagtagacctgatccagcacttgctgcattgacgaacgatcatctcgtagcgctggcttgtttgggcggcaggccagccttggacgccgtgaagaaaggattaggt

SEQ ID NO: 7 - DNA, 123 bp, Artificial Sequence
  TALE
tcgatagtagcacaattaagcaggcctgaccctgcacttgctgctcttacaaatgatcatcttgttgctctggcctgtttgggtgggcgtcccgcgttggatgctgttaagaaaggacttggt

SEQ ID NO: 8 - protein, 5 aa, Artificial Sequence
  Synthetic Sequence
TGEKQ

SEQ ID NO: 9 - protein, 10 aa, Artificial Sequence
  Synthetic Sequence
SGAQGSTLDF

SEQ ID NO: 10 - protein, 16 aa, Artificial Sequence
  Synthetic Sequence
SGSETPGTSESATPES

SEQ ID NO: 11 - protein, 33 aa, Artificial Sequence
  Synthetic Sequence
GSGGSSGGSSGSETPGTSESATPESSGGSSGGS

SEQ ID NO: 12 - protein, 138 aa, Artificial Sequence
  A1341D KRKKA
GSYALGPYQISAPQLPAYNGQTVGTFYYVNDAGGLESKVFSSGGPTPYPNYDNAGHVEGQSALFMRDNGISEGLVFHNNPEGTCGFCVNMTETLLPENAKMTVVPPEGAIPVKRGATGETKVFTGNSNSPKSPTAGGC

SEQ ID NO: 13 - protein, 138 aa, Artificial Sequence
  AAAAA
GSYALGPYQISAPQLPAYNGQTVGTFYYVNDAGGLESKVFSSGGPTPYPNYANAGHVEGQSALFMRDNGISEGLVFHNNPEGTCGFCVNMTETLLPENAKMTVVPPEGAIPVAAGATGETAVFTGNSNSPASPTAGGC

SEQ ID NO: 14 - protein, 138 aa, Artificial Sequence
  AAAAK
GSYALGPYQISAPQLPAYNGQTVGTFYYVNDAGGLESKVFSSGGPTPYPNYANAGHVEGQSALFMRDNGISEGLVFHNNPEGTCGFCVNMTETLLPENAKMTVVPPEGAIPVAAGATGETAVFTGNSNSPASPTKGGC

SEQ ID NO: 15 - protein, 138 aa, Artificial Sequence
  AAKAA
GSYALGPYQISAPQLPAYNGQTVGTFYYVNDAGGLESKVFSSGGPTPYPNYANAGHVEGQSALFMRDNGISEGLVFHNNPEGTCGFCVNMTETLLPENAKMTVVPPEGAIPVAAGATGETKVFTGNSNSPASPTAGGC

SEQ ID NO: 16 - protein, 138 aa, Artificial Sequence
  AAKAK
GSYALGPYQISAPQLPAYNGQTVGTFYYVNDAGGLESKVFSSGGPTPYPNYANAGHVEGQSALFMRDNGISEGLVFHNNPEGTCGFCVNMTETLLPENAKMTVVPPEGAIPVAAGATGETKVFTGNSNSPASPTKGGC

SEQ ID NO: 17 - protein, 138 aa, Artificial Sequence
  KAAAA
GSYALGPYQISAPQLPAYNGQTVGTFYYVNDAGGLESKVFSSGGPTPYPNYANAGHVEGQSALFMRDNGISEGLVFHNNPEGTCGFCVNMTETLLPENAKMTVVPPEGAIPVKAGATGETAVFTGNSNSPASPTAGGC

SEQ ID NO: 18 - protein, 138 aa, Artificial Sequence
  E1347A
GSYALGPYQISAPQLPAYNGQTVGTFYYVNDAGGLESKVFSSGGPTPYPNYANAGHVAGQSALFMRDNGISEGLVFHNNPEGTCGFCVNMTETLLPENAKMTVVPPEGAIPVKRGATGETKVFTGNSNSPKSPTKGGC

SEQ ID NO: 19 - protein, 138 aa, Artificial Sequence
  GSVG
GSYALGPYQISAPQLPAYNGQTVGTFYYVNDAGGLEGKVFSSGGPTPYPNYANAGHVESQSALFMRDNGISEGLVFHNNPEGTCGFCVNMTETLLPENAKMTVVPPEGVIPVKRGATGETKVFTGNSNGPKSPTKGGC

SEQ ID NO: 20 - protein, 138 aa, Artificial Sequence
  SSVG
GSYALGPYQISAPQLPAYNGQTVGTFYYVNDAGGLESKVFSSGGPTPYPNYANAGHVESQSALFMRDNGISEGLVFHNNPEGTCGFCVNMTETLLPENAKMTVVPPEGVIPVKRGATGETKVFTGNSNGPKSPTKGGC

SEQ ID NO: 21 - protein, 138 aa, Artificial Sequence
  GSAG
GSYALGPYQISAPQLPAYNGQTVGTFYYVNDAGGLEGKVFSSGGPTPYPNYANAGHVESQSALFMRDNGISEGLVFHNNPEGTCGFCVNMTETLLPENAKMTVVPPEGAIPVKRGATGETKVFTGNSNGPKSPTKGGC

SEQ ID NO: 22 - protein, 138 aa, Artificial Sequence
  GSVS
GSYALGPYQISAPQLPAYNGQTVGTFYYVNDAGGLEGKVFSSGGPTPYPNYANAGHVESQSALFMRDNGISEGLVFHNNPEGTCGFCVNMTETLLPENAKMTVVPPEGVIPVKRGATGETKVFTGNSNSPKSPTKGGC

SEQ ID NO: 23 - protein, 44 aa, Artificial Sequence
  Wild-type DddAtox G1333-N
GSYALGPYQISAPQLPAYNGQTVGTFYYVNDAGGLESKVFSSGG

SEQ ID NO: 24 - protein, 94 aa, Artificial Sequence
  Wild-type G1333-C
PTPYPNYANAGHVEGQSALFMRDNGISEGLVFHNNPEGTCGFCVNMTETLLPENAKMTVVPPEGAIPVKRGATGETKVFTGNSNSPKSPTKGGC

SEQ ID NO: 25 - protein, 108 aa, Artificial Sequence
  Wild-type DddAtox G1397-N
GSYALGPYQISAPQLPAYNGQTVGTFYYVNDAGGLESKVFSSGGPTPYPNYANAGHVEGQSALFMRDNGISEGLVFHNNPEGTCGFCVNMTETLLPENAKMTVVPPEG

SEQ ID NO: 26 - protein, 30 aa, Artificial Sequence
  Wild-type DddAtox G1397-C
AIPVKRGATGETKVFTGNSNSPKSPTKGGC

SEQ ID NO: 27 - DNA, 138 bp, Artificial Sequence
  Wild-type DddAtox G1333-N
ggctctggttcctacgccctgggtccatatcagattagtgctccccaactccccgcctacaacggtcagacagtggggaccttttactatgtcaacgacgccgggggattggaatccaaggttttctctagcggtggg

SEQ ID NO: 28 - DNA, 282 bp, Artificial Sequence
  Wild-type G1333-C
ccaacaccttatcctaactacgctaacgccgggcacgtcgaggggcagtcagctctttttatgagagataacggcattagcgaagggcttgtgttccataataatcctgagggcacctgtggcttctgtgtaaatatgaccgaaacacttctgcctgagaacgctaaaatgactgtcgtaccacccgaaggcgcaatcccagttaaacggggcgcaaccggcgaaaccaaagtattcaccggaaacagcaatagtccaaagtcccccaccaagggaggttgc

SEQ ID NO: 29 - DNA, 324 bp, Artificial Sequence
  Wild-type DddAtox G1397-N
ggtagctacgcacttggtccttaccagattagcgcaccccaactccccgcctataatggtcaaaccgtcgggaccttttactacgtaaacgatgctggtgggctggaatccaaagtattctcctcagggggccctacaccctaccccaactacgccaatgctggtcatgtagaagggcagtcagcactgtttatgcgcgataatggtataagcgaggggttggtcttccataacaacccagagggtacttgtggcttctgtgtgaatatgactgaaacccttctgcccgaaaatgccaagatgactgtcgtcccacctgaaggc

SEQ ID NO: 30 - DNA, 90 bp, Artificial Sequence
  Wild-type DddAtox G1397-C
gccatacctgtgaagcggggagcaacaggggagacaaaggtgttcacaggcaactctaacagtccaaagagccccaccaaaggcgggtgt

SEQ ID NO: 31 - protein, 44 aa, Artificial Sequence
  Deaminase Variant
GSAALGPYQISAPQLPAYNGQTVGTFYYVNDAGGLESKVFSSGG

SEQ ID NO: 32 - DNA, 138 bp, Artificial Sequence
  Deaminase Variant
ggctctggttccgcagccctgggtccatatcagattagtgctccccaactccccgcctacaacggtcagacagtggggaccttttactatgtcaacgacgccgggggattggaatccaaggttttctctagcggtggg

SEQ ID NO: 33 - protein, 44 aa, Artificial Sequence
  Deaminase Variant
GSYAAGPYQISAPQLPAYNGQTVGTFYYVNDAGGLESKVFSSGG

SEQ ID NO: 34 - DNA, 138 bp, Artificial Sequence
  Deaminase Variant
ggctctggttcctacgccgcaggtccatatcagattagtgctccccaactccccgcctacaacggtcagacagtggggaccttttactatgtcaacgacgccgggggattggaatccaaggttttctctagcggtggg

SEQ ID NO: 35 - protein, 44 aa, Artificial Sequence
  Deaminase Variant
GSYALGPYQASAPQLPAYNGQTVGTFYYVNDAGGLESKVFSSGG

SEQ ID NO: 36 - DNA, 138 bp, Artificial Sequence
  Deaminase Variant
ggctctggttcctacgccctgggtccatatcaggcaagtgctccccaactccccgcctacaacggtcagacagtggggaccttttactatgtcaacgacgccgggggattggaatccaaggttttctctagcggtggg

SEQ ID NO: 37 - protein, 44 aa, Artificial Sequence
  Deaminase Variant
GSYALGPYQIAAPQLPAYNGQTVGTFYYVNDAGGLESKVFSSGG

SEQ ID NO: 38 - DNA, 138 bp, Artificial Sequence
  Deaminase Variant
ggctctggttcctacgccctgggtccatatcagattgcagctccccaactccccgcctacaacggtcagacagtggggaccttttactatgtcaacgacgccgggggattggaatccaaggttttctctagcggtggg

SEQ ID NO: 39 - protein, 44 aa, Artificial Sequence
  Deaminase Variant
GSYALGPYQISAPQLPAYNGQTAGTFYYVNDAGGLESKVFSSGG

SEQ ID NO: 40 - DNA, 138 bp, Artificial Sequence
  Deaminase Variant
ggctctggttcctacgccctgggtccatatcagattagtgctccccaactccccgcctacaacggtcagacagcagggaccttttactatgtcaacgacgccgggggattggaatccaaggttttctctagcggtggg

SEQ ID NO: 41 - protein, 44 aa, Artificial Sequence
  Deaminase Variant
GSYALGPYQISAPQLPAYNGQTVATFYYVNDAGGLESKVFSSGG

SEQ ID NO: 42 - DNA, 138 bp, Artificial Sequence
  Deaminase Variant
ggctctggttcctacgccctgggtccatatcagattagtgctccccaactccccgcctacaacggtcagacagtggcaaccttttactatgtcaacgacgccgggggattggaatccaaggttttctctagcggtggg

SEQ ID NO: 43 - protein, 44 aa, Artificial Sequence
  Deaminase Variant
GSYALGPYQISAPQLPAYNGQTVGAFYYVNDAGGLESKVFSSGG

SEQ ID NO: 44 - DNA, 138 bp, Artificial Sequence
  Deaminase Variant
ggctctggttcctacgccctgggtccatatcagattagtgctccccaactccccgcctacaacggtcagacagtgggggcattttactatgtcaacgacgccgggggattggaatccaaggttttctctagcggtggg

SEQ ID NO: 45 - protein, 44 aa, Artificial Sequence
  Deaminase Variant
GSYALGPYQISAPQLPAYNGQTVGTAYYVNDAGGLESKVFSSGG

SEQ ID NO: 46 - DNA, 138 bp, Artificial Sequence
  Deaminase Variant
ggctctggttcctacgccctgggtccatatcagattagtgctccccaactccccgcctacaacggtcagacagtggggaccgcatactatgtcaacgacgccgggggattggaatccaaggttttctctagcggtggg

SEQ ID NO: 47 - protein, 44 aa, Artificial Sequence
  Deaminase Variant
GSYALGPYQISAPQLPAYNGQTVGTFAYVNDAGGLESKVFSSGG

SEQ ID NO: 48 - DNA, 138 bp, Artificial Sequence
  Deaminase Variant
ggctctggttcctacgccctgggtccatatcagattagtgctccccaactccccgcctacaacggtcagacagtggggacctttgcatatgtcaacgacgccgggggattggaatccaaggttttctctagcggtggg

SEQ ID NO: 49 - protein, 44 aa, Artificial Sequence
  Deaminase Variant
GSYALGPYQISAPQLPAYNGQTVGTFYAVNDAGGLESKVFSSGG

SEQ ID NO: 50 - DNA, 138 bp, Artificial Sequence
  Deaminase Variant
ggctctggttcctacgccctgggtccatatcagattagtgctccccaactccccgcctacaacggtcagacagtggggaccttttacgcagtcaacgacgccgggggattggaatccaaggttttctctagcggtggg

SEQ ID NO: 51 - protein, 44 aa, Artificial Sequence
  Deaminase Variant
GSYALGPYQISAPQLPAYNGQTVGTFYYANDAGGLESKVFSSGG

SEQ ID NO: 52 - DNA, 138 bp, Artificial Sequence
  Deaminase Variant
ggctctggttcctacgccctgggtccatatcagattagtgctccccaactccccgcctacaacggtcagacagtggggaccttttactatgcaaacgacgccgggggattggaatccaaggttttctctagcggtggg

SEQ ID NO: 53 - protein, 44 aa, Artificial Sequence
  Deaminase Variant
GSYALGPYQISAPQLPAYNGQTVGTFYYVNDAGGLESAVFSSGG

SEQ ID NO: 54 - DNA, 138 bp, Artificial Sequence
  Deaminase Variant
ggctctggttcctacgccctgggtccatatcagattagtgctccccaactccccgcctacaacggtcagacagtggggaccttttactatgtcaacgacgccgggggattggaatccgcagttttctctagcggtggg

SEQ ID NO: 55 - protein, 44 aa, Artificial Sequence
  Deaminase Variant
GSYALGPYQISAPQLPAYNGQTVGTFYYVNDAGGLESKVASSGG

SEQ ID NO: 56 - DNA, 138 bp, Artificial Sequence
  Deaminase Variant
ggctctggttcctacgccctgggtccatatcagattagtgctccccaactccccgcctacaacggtcagacagtggggaccttttactatgtcaacgacgccgggggattggaatccaaggttgcatctagcggtggg

SEQ ID NO: 57 - protein, 44 aa, Artificial Sequence
  Deaminase Variant
GSYALGPYQISAPQLPAYNGQTVGTFYYVNDAGGLESKVFASGG

SEQ ID NO: 58 - DNA, 138 bp, Artificial Sequence
  Deaminase Variant
ggctctggttcctacgccctgggtccatatcagattagtgctccccaactccccgcctacaacggtcagacagtggggaccttttactatgtcaacgacgccgggggattggaatccaaggttttcgcaagcggtggg

SEQ ID NO: 59 - protein, 94 aa, Artificial Sequence
  Deaminase Variant
PTPYPNYANAGHAEGQSALFMRDNGISEGLVFHNNPEGTCGFCVNMTETLLPENAKMTVVPPEGAIPVKRGATGETKVFTGNSNSPKSPTKGGC

SEQ ID NO: 60 - DNA, 282 bp, Artificial Sequence
  Deaminase Variant
ccaacaccttatcctaactacgctaacgccgggcacgcagaggggcagtcagctctttttatgagagataacggcattagcgaagggcttgtgttccataataatcctgagggcacctgtggcttctgtgtaaatatgaccgaaacacttctgcctgagaacgctaaaatgactgtcgtaccacccgaaggcgcaatcccagttaaacggggcgcaaccggcgaaaccaaagtattcaccggaaacagcaatagtccaaagtcccccaccaagggaggttgc

SEQ ID NO: 61 - protein, 94 aa, Artificial Sequence
  Deaminase Variant
PTPYPNYANAGHVEGASALFMRDNGISEGLVFHNNPEGTCGFCVNMTETLLPENAKMTVVPPEGAIPVKRGATGETKVFTGNSNSPKSPTKGGC

SEQ ID NO: 62 - DNA, 282 bp, Artificial Sequence
  Deaminase Variant
ccaacaccttatcctaactacgctaacgccgggcacgtcgagggggcatcagctctttttatgagagataacggcattagcgaagggcttgtgttccataataatcctgagggcacctgtggcttctgtgtaaatatgaccgaaacacttctgcctgagaacgctaaaatgactgtcgtaccacccgaaggcgcaatcccagttaaacggggcgcaaccggcgaaaccaaagtattcaccggaaacagcaatagtccaaagtcccccaccaagggaggttgc

SEQ ID NO: 63 - protein, 94 aa, Artificial Sequence
  Deaminase Variant
PTPYPNYANAGHVEGQAALFMRDNGISEGLVFHNNPEGTCGFCVNMTETLLPENAKMTVVPPEGAIPVKRGATGETKVFTGNSNSPKSPTKGGC

SEQ ID NO: 64 - DNA, 282 bp, Artificial Sequence
  Deaminase Variant
ccaacaccttatcctaactacgctaacgccgggcacgtcgaggggcaggcagctctttttatgagagataacggcattagcgaagggcttgtgttccataataatcctgagggcacctgtggcttctgtgtaaatatgaccgaaacacttctgcctgagaacgctaaaatgactgtcgtaccacccgaaggcgcaatcccagttaaacggggcgcaaccggcgaaaccaaagtattcaccggaaacagcaatagtccaaagtcccccaccaagggaggttgc

SEQ ID NO: 65 - protein, 94 aa, Artificial Sequence
  Deaminase Variant
PTPYPNYANAGHVEGQSALAMRDNGISEGLVFHNNPEGTCGFCVNMTETLLPENAKMTVVPPEGAIPVKRGATGETKVFTGNSNSPKSPTKGGC

SEQ ID NO: 66 - DNA, 282 bp, Artificial Sequence
  Deaminase Variant
ccaacaccttatcctaactacgctaacgccgggcacgtcgaggggcagtcagctcttgcaatgagagataacggcattagcgaagggcttgtgttccataataatcctgagggcacctgtggcttctgtgtaaatatgaccgaaacacttctgcctgagaacgctaaaatgactgtcgtaccacccgaaggcgcaatcccagttaaacggggcgcaaccggcgaaaccaaagtattcaccggaaacagcaatagtccaaagtcccccaccaagggaggttgc

SEQ ID NO: 67 - protein, 94 aa, Artificial Sequence
  Deaminase Variant
PTPYPNYANAGHVEGQSALFARDNGISEGLVFHNNPEGTCGFCVNMTETLLPENAKMTVVPPEGAIPVKRGATGETKVFTGNSNSPKSPTKGGC

SEQ ID NO: 68 - DNA, 282 bp, Artificial Sequence
  Deaminase Variant
ccaacaccttatcctaactacgctaacgccgggcacgtcgaggggcagtcagctctttttgcaagagataacggcattagcgaagggcttgtgttccataataatcctgagggcacctgtggcttctgtgtaaatatgaccgaaacacttctgcctgagaacgctaaaatgactgtcgtaccacccgaaggcgcaatcccagttaaacggggcgcaaccggcgaaaccaaagtattcaccggaaacagcaatagtccaaagtcccccaccaagggaggttgc

SEQ ID NO: 69 - protein, 94 aa, Artificial Sequence
  Deaminase Variant
PTPYPNYANAGHVEGQSALFMRDNGISAGLVFHNNPEGTCGFCVNMTETLLPENAKMTVVPPEGAIPVKRGATGETKVFTGNSNSPKSPTKGGC

SEQ ID NO: 70 - DNA, 282 bp, Artificial Sequence
  Deaminase Variant
ccaacaccttatcctaactacgctaacgccgggcacgtcgaggggcagtcagctctttttatgagagataacggcattagcgcagggcttgtgttccataataatcctgagggcacctgtggcttctgtgtaaatatgaccgaaacacttctgcctgagaacgctaaaatgactgtcgtaccacccgaaggcgcaatcccagttaaacggggcgcaaccggcgaaaccaaagtattcaccggaaacagcaatagtccaaagtcccccaccaagggaggttgc

SEQ ID NO: 71 - protein, 94 aa, Artificial Sequence
  Deaminase Variant
PTPYPNYANAGHVEGQSALFMRDNGISEALVFHNNPEGTCGFCVNMTETLLPENAKMTVVPPEGAIPVKRGATGETKVFTGNSNSPKSPTKGGC

SEQ ID NO: 72 - DNA, 282 bp, Artificial Sequence
  Deaminase Variant
ccaacaccttatcctaactacgctaacgccgggcacgtcgaggggcagtcagctctttttatgagagataacggcattagcgaagcacttgtgttccataataatcctgagggcacctgtggcttctgtgtaaatatgaccgaaacacttctgcctgagaacgctaaaatgactgtcgtaccacccgaaggcgcaatcccagttaaacggggcgcaaccggcgaaaccaaagtattcaccggaaacagcaatagtccaaagtcccccaccaagggaggttgc

SEQ ID NO: 73 - protein, 94 aa, Artificial Sequence
  Deaminase Variant
PTPYPNYANAGHVEGQSALFMRDNGISEGAVFHNNPEGTCGFCVNMTETLLPENAKMTVVPPEGAIPVKRGATGETKVFTGNSNSPKSPTKGGC

SEQ ID NO: 74 - DNA, 282 bp, Artificial Sequence
  Deaminase Variant
ccaacaccttatcctaactacgctaacgccgggcacgtcgaggggcagtcagctctttttatgagagataacggcattagcgaaggggcagtgttccataataatcctgagggcacctgtggcttctgtgtaaatatgaccgaaacacttctgcctgagaacgctaaaatgactgtcgtaccacccgaaggcgcaatcccagttaaacggggcgcaaccggcgaaaccaaagtattcaccggaaacagcaatagtccaaagtcccccaccaagggaggttgc

SEQ ID NO: 75 - protein, 94 aa, Artificial Sequence
  Deaminase Variant
PTPYPNYANAGHVEGQSALFMRDNGISEGLAFHNNPEGTCGFCVNMTETLLPENAKMTVVPPEGAIPVKRGATGETKVFTGNSNSPKSPTKGGC

SEQ ID NO: 76 - DNA, 282 bp, Artificial Sequence
  Deaminase Variant
ccaacaccttatcctaactacgctaacgccgggcacgtcgaggggcagtcagctctttttatgagagataacggcattagcgaagggcttgcattccataataatcctgagggcacctgtggcttctgtgtaaatatgaccgaaacacttctgcctgagaacgctaaaatgactgtcgtaccacccgaaggcgcaatcccagttaaacggggcgcaaccggcgaaaccaaagtattcaccggaaacagcaatagtccaaagtcccccaccaagggaggttgc

SEQ ID NO: 77 - protein, 94 aa, Artificial Sequence
  Deaminase Variant
PTPYPNYANAGHVEGQSALFMRDNGISEGLVAHNNPEGTCGFCVNMTETLLPENAKMTVVPPEGAIPVKRGATGETKVFTGNSNSPKSPTKGGC

SEQ ID NO: 78 - DNA, 282 bp, Artificial Sequence
  Deaminase Variant
ccaacaccttatcctaactacgctaacgccgggcacgtcgaggggcagtcagctctttttatgagagataacggcattagcgaagggcttgtggcacataataatcctgagggcacctgtggcttctgtgtaaatatgaccgaaacacttctgcctgagaacgctaaaatgactgtcgtaccacccgaaggcgcaatcccagttaaacggggcgcaaccggcgaaaccaaagtattcaccggaaacagcaatagtccaaagtcccccaccaagggaggttgc

SEQ ID NO: 79 - protein, 94 aa, Artificial Sequence
  Deaminase Variant
PTPYPNYANAGHVEGQSALFMRDNGISEGLVFANNPEGTCGFCVNMTETLLPENAKMTVVPPEGAIPVKRGATGETKVFTGNSNSPKSPTKGGC

SEQ ID NO: 80 - DNA, 282 bp, Artificial Sequence
  Deaminase Variant
ccaacaccttatcctaactacgctaacgccgggcacgtcgaggggcagtcagctctttttatgagagataacggcattagcgaagggcttgtgttcgcaaataatcctgagggcacctgtggcttctgtgtaaatatgaccgaaacacttctgcctgagaacgctaaaatgactgtcgtaccacccgaaggcgcaatcccagttaaacggggcgcaaccggcgaaaccaaagtattcaccggaaacagcaatagtccaaagtcccccaccaagggaggttgc

SEQ ID NO: 81 - protein, 94 aa, Artificial Sequence
  Deaminase Variant
PTPYPNYANAGHVEGQSALFMRDNGISEGLVFHNNPEGTCGFCVNMTETLLPENAAMTVVPPEGAIPVKRGATGETKVFTGNSNSPKSPTKGGC

SEQ ID NO: 82 - DNA, 282 bp, Artificial Sequence
  Deaminase Variant
ccaacaccttatcctaactacgctaacgccgggcacgtcgaggggcagtcagctctttttatgagagataacggcattagcgaagggcttgtgttccataataatcctgagggcacctgtggcttctgtgtaaatatgaccgaaacacttctgcctgagaacgctgcaatgactgtcgtaccacccgaaggcgcaatcccagttaaacggggcgcaaccggcgaaaccaaagtattcaccggaaacagcaatagtccaaagtcccccaccaagggaggttgc

SEQ ID NO: 83 - protein, 94 aa, Artificial Sequence
  Deaminase Variant
PTPYPNYANAGHVEGQSALFMRDNGISEGLVFHNNPEGTCGFCVNMTETLLPENAKATVVPPEGAIPVKRGATGETKVFTGNSNSPKSPTKGGC

SEQ ID NO: 84 - DNA, 282 bp, Artificial Sequence
  Deaminase Variant
ccaacaccttatcctaactacgctaacgccgggcacgtcgaggggcagtcagctctttttatgagagataacggcattagcgaagggcttgtgttccataataatcctgagggcacctgtggcttctgtgtaaatatgaccgaaacacttctgcctgagaacgctaaagcaactgtcgtaccacccgaaggcgcaatcccagttaaacggggcgcaaccggcgaaaccaaagtattcaccggaaacagcaatagtccaaagtcccccaccaagggaggttgc

SEQ ID NO: 85 - protein, 94 aa, Artificial Sequence
  Deaminase Variant
PTPYPNYANAGHVEGQSALFMRDNGISEGLVFHNNPEGTCGFCVNMTETLLPENAKMAVVPPEGAIPVKRGATGETKVFTGNSNSPKSPTKGGC

SEQ ID NO: 86 - DNA, 282 bp, Artificial Sequence
  Deaminase Variant
ccaacaccttatcctaactacgctaacgccgggcacgtcgaggggcagtcagctctttttatgagagataacggcattagcgaagggcttgtgttccataataatcctgagggcacctgtggcttctgtgtaaatatgaccgaaacacttctgcctgagaacgctaaaatggcagtcgtaccacccgaaggcgcaatcccagttaaacggggcgcaaccggcgaaaccaaagtattcaccggaaacagcaatagtccaaagtcccccaccaagggaggttgc

SEQ ID NO: 87 - protein, 94 aa, Artificial Sequence
  Deaminase Variant
PTPYPNYANAGHVEGQSALFMRDNGISEGLVFHNNPEGTCGFCVNMTETLLPENAKMTVAPPEGAIPVKRGATGETKVFTGNSNSPKSPTKGGC

SEQ ID NO: 88 - DNA, 282 bp, Artificial Sequence
  Deaminase Variant
ccaacaccttatcctaactacgctaacgccgggcacgtcgaggggcagtcagctctttttatgagagataacggcattagcgaagggcttgtgttccataataatcctgagggcacctgtggcttctgtgtaaatatgaccgaaacacttctgcctgagaacgctaaaatgactgtcgcaccacccgaaggcgcaatcccagttaaacggggcgcaaccggcgaaaccaaagtattcaccggaaacagcaatagtccaaagtcccccaccaagggaggttgc

SEQ ID NO: 89 - protein, 108 aa, Artificial Sequence
  Deaminase Variant
GSYALGPYQISAPQLPAYNGQTVGTFYYVNDAGGLESKVFSSGGPTPYPNYANAGHVEGQSALFMRDNGISEGLVFHNNPEGTCGFAVNMTETLLPENAKMTVVPPEG

SEQ ID NO: 90 - DNA, 324 bp, Artificial Sequence
  Deaminase Variant
ggtagctacgcacttggtccttaccagattagcgcaccccaactccccgcctataatggtcaaaccgtcgggaccttttactacgtaaacgatgctggtgggctggaatccaaagtattctcctcagggggccctacaccctaccccaactacgccaatgctggtcatgtagaagggcagtcagcactgtttatgcgcgataatggtataagcgaggggttggtcttccataacaacccagagggtacttgtggcttcgcagtgaatatgactgaaacccttctgcccgaaaatgccaagatgactgtcgtcccacctgaaggc

SEQ ID NO: 91 - protein, 108 aa, Artificial Sequence
  Deaminase Variant
GSYALGPYQISAPQLPAYNGQTVGTFYYVNDAGGLESKVFSSGGPTPYPNYANAGHVEGQSALFMRDNGISEGLVFHNNPEGTCGFCANMTETLLPENAKMTVVPPEG

SEQ ID NO: 92 - DNA, 324 bp, Artificial Sequence
  Deaminase Variant
ggtagctacgcacttggtccttaccagattagcgcaccccaactccccgcctataatggtcaaaccgtcgggaccttttactacgtaaacgatgctggtgggctggaatccaaagtattctcctcagggggccctacaccctaccccaactacgccaatgctggtcatgtagaagggcagtcagcactgtttatgcgcgataatggtataagcgaggggttggtcttccataacaacccagagggtacttgtggcttctgtgcaaatatgactgaaacccttctgcccgaaaatgccaagatgactgtcgtcccacctgaaggc

SEQ ID NO: 93 - protein, 108 aa, Artificial Sequence
  Deaminase Variant
GSYALGPYQISAPQLPAYNGQTVGTFYYVNDAGGLESKVFSSGGPTPYPNYANAGHVEGQSALFMRDNGISEGLVFHNNPEGTCGFCVNMAETLLPENAKMTVVPPEG

SEQ ID NO: 94 - DNA, 324 bp, Artificial Sequence
  Deaminase Variant
ggtagctacgcacttggtccttaccagattagcgcaccccaactccccgcctataatggtcaaaccgtcgggaccttttactacgtaaacgatgctggtgggctggaatccaaagtattctcctcagggggccctacaccctaccccaactacgccaatgctggtcatgtagaagggcagtcagcactgtttatgcgcgataatggtataagcgaggggttggtcttccataacaacccagagggtacttgtggcttctgtgtgaatatggcagaaacccttctgcccgaaaatgccaagatgactgtcgtcccacctgaaggc

SEQ ID NO: 95 - protein, 108 aa, Artificial Sequence
  Deaminase Variant
GSYALGPYQISAPQLPAYNGQTVGTFYYVNDAGGLESKVFSSGGPTPYPNYANAGHVEGQSALFMRDNGISEGLVFHNNPEGTCGFCVNMTATLLPENAKMTVVPPEG

SEQ ID NO: 96 - DNA, 324 bp, Artificial Sequence
  Deaminase Variant
ggtagctacgcacttggtccttaccagattagcgcaccccaactccccgcctataatggtcaaaccgtcgggaccttttactacgtaaacgatgctggtgggctggaatccaaagtattctcctcagggggccctacaccctaccccaactacgccaatgctggtcatgtagaagggcagtcagcactgtttatgcgcgataatggtataagcgaggggttggtcttccataacaacccagagggtacttgtggcttctgtgtgaatatgactgcaacccttctgcccgaaaatgccaagatgactgtcgtcccacctgaaggc

SEQ ID NO: 97 - protein, 108 aa, Artificial Sequence
  Deaminase Variant
GSYALGPYQISAPQLPAYNGQTVGTFYYVNDAGGLESKVFSSGGPTPYPNYANAGHVEGQSALFMRDNGISEGLVFHNNPEGTCGFCVNMTETLAPENAKMTVVPPEG

SEQ ID NO: 98 - DNA, 324 bp, Artificial Sequence
  Deaminase Variant
ggtagctacgcacttggtccttaccagattagcgcaccccaactccccgcctataatggtcaaaccgtcgggaccttttactacgtaaacgatgctggtgggctggaatccaaagtattctcctcagggggccctacaccctaccccaactacgccaatgctggtcatgtagaagggcagtcagcactgtttatgcgcgataatggtataagcgaggggttggtcttccataacaacccagagggtacttgtggcttctgtgtgaatatgactgaaacccttgcacccgaaaatgccaagatgactgtcgtcccacctgaaggc

SEQ ID NO: 99 - protein, 108 aa, Artificial Sequence
  Deaminase Variant
GSYALGPYQISAPQLPAYNGQTVGTFYYVNDAGGLESKVFSSGGPTPYPNYANAGHVEGQSALFMRDNGISEGLVFHNNPEGTCGFCVNMTETLLPENAAMTVVPPEG

SEQ ID NO: 100 - DNA, 324 bp, Artificial Sequence
  Deaminase Variant
ggtagctacgcacttggtccttaccagattagcgcaccccaactccccgcctataatggtcaaaccgtcgggaccttttactacgtaaacgatgctggtgggctggaatccaaagtattctcctcagggggccctacaccctaccccaactacgccaatgctggtcatgtagaagggcagtcagcactgtttatgcgcgataatggtataagcgaggggttggtcttccataacaacccagagggtacttgtggcttctgtgtgaatatgactgaaacccttctgcccgaaaatgccgcaatgactgtcgtcccacctgaaggc

SEQ ID NO: 101 - protein, 108 aa, Artificial Sequence
  Deaminase Variant
GSYALGPYQISAPQLPAYNGQTVGTFYYVNDAGGLESKVFSSGGPTPYPNYANAGHVEGQSALFMRDNGISEGLVFHNNPEGTCGFCVNMTETLLPENAKATVVPPEG

SEQ ID NO: 102 - DNA, 324 bp, Artificial Sequence
  Deaminase Variant
ggtagctacgcacttggtccttaccagattagcgcaccccaactccccgcctataatggtcaaaccgtcgggaccttttactacgtaaacgatgctggtgggctggaatccaaagtattctcctcagggggccctacaccctaccccaactacgccaatgctggtcatgtagaagggcagtcagcactgtttatgcgcgataatggtataagcgaggggttggtcttccataacaacccagagggtacttgtggcttctgtgtgaatatgactgaaacccttctgcccgaaaatgccaaggcaactgtcgtcccacctgaaggc

SEQ ID NO: 103 - protein, 108 aa, Artificial Sequence
  Deaminase Variant
GSYALGPYQISAPQLPAYNGQTVGTFYYVNDAGGLESKVFSSGGPTPYPNYANAGHVEGQSALFMRDNGISEGLVFHNNPEGTCGFCVNMTETLLPENAKMAVVPPEG

SEQ ID NO: 104 - DNA, 324 bp, Artificial Sequence
  Deaminase Variant
ggtagctacgcacttggtccttaccagattagcgcaccccaactccccgcctataatggtcaaaccgtcgggaccttttactacgtaaacgatgctggtgggctggaatccaaagtattctcctcagggggccctacaccctaccccaactacgccaatgctggtcatgtagaagggcagtcagcactgtttatgcgcgataatggtataagcgaggggttggtcttccataacaacccagagggtacttgtggcttctgtgtgaatatgactgaaacccttctgcccgaaaatgccaagatggcagtcgtcccacctgaaggc

SEQ ID NO: 105 - protein, 108 aa, Artificial Sequence
  Deaminase Variant
GSYALGPYQISAPQLPAYNGQTVGTFYYVNDAGGLESKVFSSGGPTPYPNYANAGHVEGQSALFMRDNGISEGLVFHNNPEGTCGFCVNMTETLLPENAKMTAVPPEG

SEQ ID NO: 106 - DNA, 324 bp, Artificial Sequence
  Deaminase Variant
ggtagctacgcacttggtccttaccagattagcgcaccccaactccccgcctataatggtcaaaccgtcgggaccttttactacgtaaacgatgctggtgggctggaatccaaagtattctcctcagggggccctacaccctaccccaactacgccaatgctggtcatgtagaagggcagtcagcactgtttatgcgcgataatggtataagcgaggggttggtcttccataacaacccagagggtacttgtggcttctgtgtgaatatgactgaaacccttctgcccgaaaatgccaagatgactgcagtcccacctgaaggc

SEQ ID NO: 107 - protein, 30 aa, Artificial Sequence
  Deaminase Variant
AIPVKRGATGETAVFTGNSNSPKSPTKGGC

SEQ ID NO: 108 - DNA, 90 bp, Artificial Sequence
  Deaminase Variant
gccatacctgtgaagcggggagcaacaggggagacagcagtgttcacaggcaactctaacagtccaaagagccccaccaaaggcgggtgt

SEQ ID NO: 109 - protein, 30 aa, Artificial Sequence
  Deaminase Variant
AIPVKRGATGETKAFTGNSNSPKSPTKGGC

SEQ ID NO: 110 - DNA, 90 bp, Artificial Sequence
  Deaminase Variant
gccatacctgtgaagcggggagcaacaggggagacaaaggcattcacaggcaactctaacagtccaaagagccccaccaaaggcgggtgt

SEQ ID NO: 111 - protein, 30 aa, Artificial Sequence
  Deaminase Variant
AIPVKRGATGETKVATGNSNSPKSPTKGGC

SEQ ID NO: 112 - DNA, 90 bp, Artificial Sequence
  Deaminase Variant
gccatacctgtgaagcggggagcaacaggggagacaaaggtggcaacaggcaactctaacagtccaaagagccccaccaaaggcgggtgt

SEQ ID NO: 113 - protein, 30 aa, Artificial Sequence
  Deaminase Variant
AIPVKRGATGETKVFAGNSNSPKSPTKGGC

SEQ ID NO: 114 - DNA, 90 bp, Artificial Sequence
  Deaminase Variant
gccatacctgtgaagcggggagcaacaggggagacaaaggtgttcgcaggcaactctaacagtccaaagagccccaccaaaggcgggtgt

SEQ ID NO: 115 - protein, 24 aa, Artificial Sequence
  Linker
SGTPHEVGVYTLSGTPHEVGVYTL

SEQ ID NO: 116 - DNA, 19 bp, Artificial Sequence
  Primer
catcaatgggcgtggatag

SEQ ID NO: 117 - DNA, 19 bp, Artificial Sequence
  Primer
catcaatgggcgtggatag

SEQ ID NO: 118 - DNA, 20 bp, Artificial Sequence
  Primer
gacacctactcagacaatgc

SEQ ID NO: 119 - DNA, 12 bp, Artificial Sequence
  Left-ZFD DNA binding region
gtcatcctcatc

SEQ ID NO: 120 - DNA, 12 bp, Artificial Sequence
  Synthetic Sequence
aaactgcaaaag

SEQ ID NO: 121 - DNA, 3 bp, Artificial Sequence
  Synthetic Sequence
tcg

SEQ ID NO: 122 - DNA, 4 bp, Artificial Sequence
  Synthetic Sequence
ctga

SEQ ID NO: 123 - DNA, 5 bp, Artificial Sequence
  Synthetic Sequence
ctgat

SEQ ID NO: 124 - DNA, 6 bp, Artificial Sequence
  Synthetic Sequence
ctgatc

SEQ ID NO: 125 - DNA, 7 bp, Artificial Sequence
  Synthetic Sequence
ctgatcg

SEQ ID NO: 126 - DNA, 8 bp, Artificial Sequence
  Synthetic Sequence
ctgatcga

SEQ ID NO: 127 - DNA, 9 bp, Artificial Sequence
  Synthetic Sequence
ctgatcgat

SEQ ID NO: 128 - DNA, 10 bp, Artificial Sequence
  Synthetic Sequence
ctgatcgatc

SEQ ID NO: 129 - DNA, 11 bp, Artificial Sequence
  Synthetic Sequence
ctgatcgatcg

SEQ ID NO: 130 - DNA, 12 bp, Artificial Sequence
  Synthetic Sequence
ctgatcgatcga

SEQ ID NO: 131 - DNA, 13 bp, Artificial Sequence
  Synthetic Sequence
ctgatcgatcgat

SEQ ID NO: 132 - DNA, 14 bp, Artificial Sequence
  Synthetic Sequence
ctgatcgatcgatc

SEQ ID NO: 133 - DNA, 15 bp, Artificial Sequence
  Synthetic Sequence
ctgatcgatcgatcg

SEQ ID NO: 134 - DNA, 16 bp, Artificial Sequence
  Synthetic Sequence
ctgatcgatcgatcga

SEQ ID NO: 135 - DNA, 17 bp, Artificial Sequence
  Synthetic Sequence
ctgatcgatcgatcgat

SEQ ID NO: 136 - DNA, 18 bp, Artificial Sequence
  Synthetic Sequence
ctgatcgatcgatcgatc

SEQ ID NO: 137 - DNA, 19 bp, Artificial Sequence
  Synthetic Sequence
ctgatcgatcgatcgatcg

SEQ ID NO: 138 - DNA, 20 bp, Artificial Sequence
  Synthetic Sequence
ctgatcgatcgatcgatcga

SEQ ID NO: 139 - DNA, 21 bp, Artificial Sequence
  Synthetic Sequence
ctgatcgatcgatcgatcgat

SEQ ID NO: 140 - DNA, 22 bp, Artificial Sequence
  Synthetic Sequence
ctgatcgatcgatcgatcgatc

SEQ ID NO: 141 - DNA, 23 bp, Artificial Sequence
  Synthetic Sequence
ctgatcgatcgatcgatcgatcg

SEQ ID NO: 142 - DNA, 24 bp, Artificial Sequence
  Synthetic Sequence
ctgatcgatcgatcgatcgatcga

SEQ ID NO: 143 - DNA, 33 bp, Artificial Sequence
  Synthetic Sequence
gtttactcaatcctctgatcagggtgagcatca

SEQ ID NO: 144 - protein, 11 aa, Artificial Sequence
  Synthetic Sequence
VYSILWSGWAS

SEQ ID NO: 145 - DNA, 33 bp, Artificial Sequence
  Synthetic Sequence
gtttactcaatcctctgattagggtgagcatca

SEQ ID NO: 146 - protein, 11 aa, Artificial Sequence
  Synthetic Sequence
VYSILWLGWAS

SEQ ID NO: 147 - DNA, 33 bp, Artificial Sequence
  Synthetic Sequence
gtttactcaatcctctaatcagggtgagcatca

SEQ ID NO: 148 - protein, 10 aa, Artificial Sequence
  Synthetic Sequence
VYSILSGWAS

SEQ ID NO: 149 - DNA, 39 bp, Artificial Sequence
  Synthetic Sequence
ctacgcctaatctactccacctcaatcacactactcccc

SEQ ID NO: 150 - DNA, 39 bp, Artificial Sequence
  Synthetic Sequence
ctacgcctaatctactttacctcaatcacactactcccc

SEQ ID NO: 151 - protein, 13 aa, Artificial Sequence
  Synthetic Sequence
LRLIYFTSITLLP

SEQ ID NO: 152 - DNA, 39 bp, Artificial Sequence; identical to SEQ ID NO: 149
  Synthetic Sequence

SEQ ID NO: 153 - protein, 13 aa, Artificial Sequence
  Synthetic Sequence
LRLIYSTSITLLP

SEQ ID NO: 154 - DNA, 39 bp, Artificial Sequence
  Synthetic Sequence
ctacgcctaatctactttatttcaatcacactactcccc

SEQ ID NO: 155 - protein, 13 aa, Artificial Sequence
  Synthetic Sequence
LRLIYFISITLLP

SEQ ID NO: 156 - DNA, 39 bp, Artificial Sequence
  Synthetic Sequence
ctacgcctaatctacttcacctcaatcacactactcccc

SEQ ID NO: 157 - protein, 13 aa, Artificial Sequence
  Synthetic Sequence
LRLIYFTSITLLP

SEQ ID NO: 158 - DNA, 39 bp, Artificial Sequence
  Synthetic Sequence
ctacgcctaatctactttatctcaatcacactactcccc

SEQ ID NO: 159 - protein, 13 aa, Artificial Sequence
  Synthetic Sequence
LRLIYFISITLLP

SEQ ID NO: 160 - DNA, 39 bp, Artificial Sequence
  Synthetic Sequence
ctacgcctaatctactttaccttaatcacactactcccc

SEQ ID NO: 161 - protein, 13 aa, Artificial Sequence
  Synthetic Sequence
LRLIYFTLITLLP

SEQ ID NO: 162 - DNA, 917 bp, Artificial Sequence
  Synthetic Sequence
ctagcaacgattgtacaattgcttctttaaaaaaggaagaaagaaagaaagaaaagaatcaacatcagcgttaacaaacggccccgttacggcccaaacggtcatatagagtaacggcgttaagcgttgaaagactcctatcgaaatacgtaaccgcaaacgtgtcatagtcagatcccctcttccttcaccgcctcaaacacaaaaataatcttctacagcctatatatacaacccccccttctatctctcctttctcacaattcatcatctttctttctctacccccaattttaagaaatcctctcttctcctcttcattttcaaggtaaatctctctctctctctctctctctgttattccttgttttaattaggtatgtattattgctagtttgttaatctgcttatcttatgtatgccttatgtgaatatctttatcttgttcatctcatccgtttagaagctataaatttgttgatttgactgtgtatctacacgtggttatgtttatatctaatcagatatgaatttcttcatattgttgcgtttgtgtgtaccaatccgaaatcgttgatttttttcatttaatcgtgtagctaattgtacgtatacatatggatctacgtatcaattgttcatctgtttgtgtttgtatgtatacagatctgaaaacatcacttctctcatctgattgtgttgttacatacatagatatagatctgttatatcattttttttattaattgtgtatatatatatgtgcatagatctggattacatgattgtgattatttacatgattttgttatttacgtatgtatatatgtagatctggactttttggagttgttgacttgattgtatttgtgtgtgtatatgtgtgttctgatcttgatatgttatgtatgtgcagc

SEQ ID NO: 163 - DNA, 469 bp, Artificial Sequence
  Synthetic Sequence
caggcctcccagctttcgtccgtatcatcggtttcgacaacgttcgtcaagttcaatgcatcagtttcattgcccacacaccagaatcctactaagtttgagtattatggcattggaaaagctgttttcttctatcatttgttctgcttgtaatttactgtgttctttcagtttttgttttcggacatcaaaatgcaaatggatggataagagttaataaatgatatggtccttttgttcattctcaaattattattatctgttgtttttactttaatgggttgaatttaagtaagaaaggaactaacagtgtgatattaaggtgcaatgttagacatataaaacagtctttcacctctctttggttatgtcttgaattggtttgtttcttcacttatctgtgtaatcaagtttactatgagtctatgatcaagtaattatgcaatcaagttaagtacagtataggctt

SEQ ID NO: 164 - DNA, 19 bp, Artificial Sequence
  Synthetic Sequence
taatacgactcactatagg

SEQ ID NO: 165 - protein, 308 aa, Artificial Sequence
  Synthetic Sequence
MLQLCSTFRPQLLLPCQFRFTNGVLIPQINYVASNSVVNIRPMIRCQRASGGRGGANRSKPAKPQVKEGSNKTVIEGLVTESLPNGMFRVDLENGDNILGYICGKIRKNFIRILPGDKVKVEMSVYDSTKGRIIFRMSSRDYPYDVPDYAGYPYDVPDYAGYPYDVPDYAMDIADLRTLGYSQQQQEKIKPKVRSTVAQHHEALVGHGFTHAHIVALSQHPAALGTVAVKYQDMIAALPEATHEAIVGVGKQWSGARALEALLTVAGELRGPPLQLDTGQLLKIAKRGGVTAVEAVHAWRNALTGAPL

SEQ ID NO: 166 - protein, 240 aa, Artificial Sequence
  Synthetic Sequence
MASSMLSSATMVASPAQATMVAPFNGLKSSAAFPATRKANNDITSITSNGGRVNCMQVWPPIGKKKFETLSYLPDLTDSEDYKDHDGDYKDHDIDYKDDDDKMDIADLRTLGYSQQQQEKIKPKVRSTVAQHHEALVGHGFTHAHIVALSQHPAALGTVAVKYQDMIAALPEATHEAIVGVGKRGAGARALEALLTVAGELRGPPLQLDTGQLLKIAKRGGVTAVEAVHAWRNALTGAPL

SEQ ID NO: 167 - protein, 244 aa, Artificial Sequence
  Synthetic Sequence
MAMAVFRREGRRLLPSIAARPIAAIRSPLSSDQEEGLLGVRSISTQVVRNRMKSVKNIQKITKAMKMVAASKLRAVQYPYDVPDYAGYPYDVPDYAGYPYDVPDYAMDIADLRTLGYSQQQQEKIKPKVRSTVAQHHEALVGHGFTHAHIVALSQHPAALGTVAVKYQDMIAALPEATHEAIVGVGKQWSGARALEALLTVAGELRGPPLQLDTGQLLKIAKRGGVTAVEAVHAWRNALTGAPL

SEQ ID NO: 168 - protein, 196 aa, Artificial Sequence
  Synthetic Sequence
MFKQASRLLSRSVAAASSKSVTTRAFSTELPSTLDSDYKDHDGDYKDHDIDYKDDDDKMDIADLRTLGYSQQQQEKIKPKVRSTVAQHHEALVGHGFTHAHIVALSQHPAALGTVAVKYQDMIAALPEATHEAIVGVGKRGAGARALEALLTVAGELRGPPLQLDTGQLLKIAKRGGVTAVEAVHAWRNALTGAPL

SEQ ID NO: 169 - protein, 195 aa, Artificial Sequence
  Synthetic Sequence
GLTPEQVVAIASNGGGKQALESIVAQLSRPDPALAALTNDHLVALACLGGRPALDAVKKGLGGSGSYALGPYQISAPQLPAYNGQTVGTFYYVNDAGGLESKVFSSGGSGGSTNLSDIIEKETGKQLVIQESILMLPEEVEEVIGNKPESDILVHTAYDESTDENVMLLTSDAPEYKPWALVIQDSNGENKIKML

SEQ ID NO: 170 - protein, 245 aa, Artificial Sequence
  Synthetic Sequence
GLTPEQVVAIASNGGGKQALESIVAQLSRPDPALAALTNDHLVALACLGGRPALDAVKKGLGGSPTPYPNYANAGHVEGQSALFMRDNGISEGLVFHNNPEGTCGFCVNMTETLLPENAKMTVVPPEGAIPVKRGATGETKVFTGNSNSPKSPTKGGCSGGSTNLSDIIEKETGKQLVIQESILMLPEEVEEVIGNKPESDILVHTAYDESTDENVMLLTSDAPEYKPWALVIQDSNGENKIKML

SEQ ID NO: 171 - protein, 259 aa, Artificial Sequence
  Synthetic Sequence
GLTPEQVVAIASNGGGKQALESIVAQLSRPDPALAALTNDHLVALACLGGRPALDAVKKGLGGSGSYALGPYQISAPQLPAYNGQTVGTFYYVNDAGGLESKVFSSGGPTPYPNYANAGHVEGQSALFMRDNGISEGLVFHNNPEGTCGFCVNMTETLLPENAKMTVVPPEGSGGSTNLSDIIEKETGKQLVIQESILMLPEEVEEVIGNKPESDILVHTAYDESTDENVMLLTSDAPEYKPWALVIQDSNGENKIKML

SEQ ID NO: 172 - protein, 181 aa, Artificial Sequence
  Synthetic Sequence
GLTPEQVVAIASNGGGKQALESIVAQLSRPDPALAALTNDHLVALACLGGRPALDAVKKGLGGSAIPVKRGATGETKVFTGNSNSPKSPTKGGCSGGSTNLSDIIEKETGKQLVIQESILMLPEEVEEVIGNKPESDILVHTAYDESTDENVMLLTSDAPEYKPWALVIQDSNGENKIKML

SEQ ID NO: 173 - protein, 68 aa, Artificial Sequence
  Synthetic Sequence
NLTPAQVVAIASNNGGKQALETVQRLLPVLCQAHGLTPDQVVAIASNNGGKQALETVQRLLPVLCQDH

SEQ ID NO: 174 - protein, 68 aa, Artificial Sequence
  Synthetic Sequence
GLTPEQVVAIASNNGGKQALETVQRLLPVLCQAHGLTPDQVVAIASNNGGKQALETVQRLLPVLCQDH

SEQ ID NO: 175 - protein, 68 aa, Artificial Sequence
  Synthetic Sequence
GLTPAQVVAIASNIGGKQALETVQRLLPVLCQAHGLTPEQVVAIASNNGGKQALETVQRLLPVLCQAH

SEQ ID NO: 176 - protein, 68 aa, Artificial Sequence
  Synthetic Sequence
GLTPEQVVAIASNGGGKQALETVQRLLPVLCQAHGLTPDQVVAIASNIGGKQALETVQRLLPVLCQAH

SEQ ID NO: 177 - protein, 68 aa, Artificial Sequence
  Synthetic Sequence
GLTPAQVVAIASHDGGKQALETVQRLLPVLCQAHGLTPAQVVAIASNNGGKQALETVQRLLPVLCQDH

SEQ ID NO: 178 - protein, 68 aa, Artificial Sequence
  Synthetic Sequence
GLTPEQVVAIASNGGGKQALETVQRLLPVLCQAHGLTPAQVVAIASNGGGKQALETVQRLLPVLCQDH

SEQ ID NO: 179 - protein, 68 aa, Artificial Sequence
  Synthetic Sequence
GLTPAQVVAIASHDGGKQALETVQRLLPVLCQAHGLTPDQVVAIASNNGGKQALETVQRLLPVLCQDH

SEQ ID NO: 180 - protein, 68 aa, Artificial Sequence
  Synthetic Sequence
GLTPDQVVAIASHDGGKQALETVQRLLPVLCQDHGLTPAQVVAIASNIGGKQALETVQRLLPVLCQDH

SEQ ID NO: 181 - protein, 68 aa, Artificial Sequence
  Synthetic Sequence
GLTPDQVVAIASNIGGKQALETVQRLLPVLCQDHGLTPDQVVAIASNNGGKQALETVQRLLPVLCQAH

SEQ ID NO: 182 - protein, 68 aa, Artificial Sequence
  Synthetic Sequence
NLTPAQVVAIASNGGGKQALETVQRLLPVLCQAHGLTPDQVVAIASNNGGKQALETVQRLLPVLCQAH

SEQ ID NO: 183 - protein, 68 aa, Artificial Sequence
  Synthetic Sequence
GLTPAQVVAIASNGGGKQALETVQRLLPVLCQDHGLTPAQVVAIASNNGGKQALETVQRLLPVLCQAH

SEQ ID NO: 184 - protein, 68 aa, Artificial Sequence
  Synthetic Sequence
GLTPDQVVAIASHDGGKQALETVQRLLPVLCQDHGLTPAQVVAIASNNGGKQALETVQRLLPVLCQAH

SEQ ID NO: 185 - protein, 68 aa, Artificial Sequence
  Synthetic Sequence
GLTPEQVVAIASNNGGKQALETVQRLLPVLCQAHGLTPAQVVAIASNNGGKQALETVQRLLPVLCQDH

SEQ ID NO: 186 - protein, 68 aa, Artificial Sequence
  Synthetic Sequence
GLTPDQVVAIASHDGGKQALETVQRLLPVLCQAHGLTPAQVVAIASHDGGKQALETVQRLLPVLCQAH

SEQ ID NO: 187 - protein, 68 aa, Artificial Sequence
  Synthetic Sequence
GLTPDQVVAIASHDGGKQALETVQRLLPVLCQDHGLTPDQVVAIASHDGGKQALETVQRLLPVLCQDH

SEQ ID NO: 188 - protein, 68 aa, Artificial Sequence
  Synthetic Sequence
GLTPDQVVAIASHDGGKQALETVQRLLPVLCQDHGLTPDQVVAIASNNGGKQALETVQRLLPVLCQDH

SEQ ID NO: 189 - protein, 68 aa, Artificial Sequence
  Synthetic Sequence
GLTPAQVVAIASNGGGKQALETVQRLLPVLCQAHGLTPAQVVAIASHDGGKQALETVQRLLPVLCQDH

SEQ ID NO: 190 - protein, 68 aa, Artificial Sequence
  Synthetic Sequence
GLTPEQVVAIASNIGGKQALETVQRLLPVLCQAHGLTPAQVVAIASNIGGKQALETVQRLLPVLCQDH

SEQ ID NO: 191 - protein, 68 aa, Artificial Sequence
  Synthetic Sequence
NLTPAQVVAIASNNGGKQALETVQRLLPVLCQAHGLTPDQVVAIASHDGGKQALETVQRLLPVLCQDH

SEQ ID NO: 192 - protein, 68 aa, Artificial Sequence
  Synthetic Sequence
GLTPAQVVAIASNIGGKQALETVQRLLPVLCQAHGLTPDQVVAIASNIGGKQALETVQRLLPVLCQDH

SEQ ID NO: 193 - protein, 68 aa, Artificial Sequence
  Synthetic Sequence
GLTPDQVVAIASHDGGKQALETVQRLLPVLCQDHGLTPAQVVAIASNIGGKQALETVQRLLPVLCQAH

SEQ ID NO: 194 - protein, 68 aa, Artificial Sequence
  Synthetic Sequence
GLTPAQVVAIASNNGGKQALETVQRLLPVLCQAHGLTPDQVVAIASNNGGKQALETVQRLLPVLCQDH

SEQ ID NO: 195 - protein, 68 aa, Artificial Sequence
  Synthetic Sequence
GLTPAQVVAIASNIGGKQALETVQRLLPVLCQAHGLTPDQVVAIASNNGGKQALETVQRLLPVLCQAH

SEQ ID NO: 196 - protein, 68 aa, Artificial Sequence
  Synthetic Sequence
GLTPAQVVAIASHDGGKQALETVQRLLPVLCQDHGLTPDQVVAIASNGGGKQALETVQRLLPVLCQAH

SEQ ID NO: 197 - protein, 68 aa, Artificial Sequence
  Synthetic Sequence
GLTPEQVVAIASNNGGKQALETVQRLLPVLCQAHGLTPDQVVAIASNIGGKQALETVQRLLPVLCQDH

SEQ ID NO: 198 - protein, 68 aa, Artificial Sequence
  Synthetic Sequence
GLTPDQVVAIASNIGGKQALETVQRLLPVLCQAHGLTPDQVVAIASNGGGKQALETVQRLLPVLCQAH

SEQ ID NO: 199 - protein, 68 aa, Artificial Sequence
  Synthetic Sequence
GLTPDQVVAIASNIGGKQALETVQRLLPVLCQDHGLTPDQVVAIASNGGGKQALETVQRLLPVLCQAH

SEQ ID NO: 200 - protein, 68 aa, Artificial Sequence
  Synthetic Sequence
NLTPAQVVAIASNIGGKQALETVQRLLPVLCQAHGLTPEQVVAIASNNGGKQALETVQRLLPVLCQAH

SEQ ID NO: 201 - protein, 68 aa, Artificial Sequence
  Synthetic Sequence
GLTPDQVVAIASNGGGKQALETVQRLLPVLCQDHGLTPDQVVAIASNGGGKQALETVQRLLPVLCQDH

SEQ ID NO: 202 - protein, 68 aa, Artificial Sequence
  Synthetic Sequence
GLTPEQVVAIASNGGGKQALETVQRLLPVLCQAHGLTPDQVVAIASHDGGKQALETVQRLLPVLCQAH

SEQ ID NO: 203 - protein, 68 aa, Artificial Sequence; identical to SEQ ID NO: 188
  Synthetic Sequence

SEQ ID NO: 204 - protein, 68 aa, Artificial Sequence
  Synthetic Sequence
GLTPAQVVAIASNGGGKQALETVQRLLPVLCQAHGLTPAQVVAIASHDGGKQALETVQRLLPVLCQAH

SEQ ID NO: 205 - protein, 68 aa, Artificial Sequence
  Synthetic Sequence
GLTPAQVVAIASNGGGKQALETVQRLLPVLCQDHGLTPDQVVAIASNNGGKQALETVQRLLPVLCQDH

SEQ ID NO: 206 - protein, 68 aa, Artificial Sequence
  Synthetic Sequence
GLTPAQVVAIASNNGGKQALETVQRLLPVLCQDHGLTPAQVVAIASNNGGKQALETVQRLLPVLCQDH

SEQ ID NO: 207 - protein, 68 aa, Artificial Sequence
  Synthetic Sequence
GLTPDQVVAIASNGGGKQALETVQRLLPVLCQAHGLTPEQVVAIASNIGGKQALETVQRLLPVLCQAH

SEQ ID NO: 208 - protein, 68 aa, Artificial Sequence
  Synthetic Sequence
GLTPAQVVAIASNGGGKQALETVQRLLPVLCQAHGLTPAQVVAIASNNGGKQALETVQRLLPVLCQDH

SEQ ID NO: 209 - protein, 68 aa, Artificial Sequence
  Synthetic Sequence
NLTPDQVVAIASNIGGKQALETVQRLLPVLCQAHGLTPAQVVAIASNIGGKQALETVQRLLPVLCQDH

SEQ ID NO: 210 - protein, 68 aa, Artificial Sequence
  Synthetic Sequence
GLTPAQVVAIASNIGGKQALETVQRLLPVLCQAHGLTPAQVVAIASNGGGKQALETVQRLLPVLCQAH

SEQ ID NO: 211 - protein, 68 aa, Artificial Sequence
  Synthetic Sequence
GLTPAQVVAIASNNGGKQALETVQRLLPVLCQDHGLTPAQVVAIASNIGGKQALETVQRLLPVLCQDH

SEQ ID NO: 212 - protein, 68 aa, Artificial Sequence
  Synthetic Sequence
GLTPAQVVAIASNIGGKQALETVQRLLPVLCQAHGLTPDQVVAIASNGGGKQALETVQRLLPVLCQAH

SEQ ID NO: 213 - protein, 68 aa, Artificial Sequence
  Synthetic Sequence
GLTPDQVVAIASNGGGKQALETVQRLLPVLCQAHGLTPAQVVAIASHDGGKQALETVQRLLPVLCQDH

SEQ ID NO: 214 - protein, 68 aa, Artificial Sequence
  Synthetic Sequence
GLTPDQVVAIASHDGGKQALETVQRLLPVLCQAHGLTPDQVVAIASNIGGKQALETVQRLLPVLCQAH

SEQ ID NO: 215 - protein, 68 aa, Artificial Sequence
  Synthetic Sequence
GLTPDQVVAIASNIGGKQALETVQRLLPVLCQAHGLTPAQVVAIASNIGGKQALETVQRLLPVLCQDH

SEQ ID NO: 216 - protein, 68 aa, Artificial Sequence; identical to SEQ ID NO: 192
  Synthetic Sequence

SEQ ID NO: 217 - protein, 68 aa, Artificial Sequence; identical to SEQ ID NO: 189
  Synthetic Sequence

SEQ ID NO: 218 - protein, 68 aa, Artificial Sequence
  Synthetic Sequence
NLTPEQVVAIASNNGGKQALETVQRLLPVLCQAHGLTPDQVVAIASNIGGKQALETVQRLLPVLCQDH

SEQ ID NO: 219 - protein, 68 aa, Artificial Sequence
  Synthetic Sequence
GLTPDQVVAIASNIGGKQALETVQRLLPVLCQAHGLTPDQVVAIASHDGGKQALETVQRLLPVLCQDH

SEQ ID NO: 220 - protein, 68 aa, Artificial Sequence
  Synthetic Sequence
GLTPDQVVAIASNNGGKQALETVQRLLPVLCQDHGLTPAQVVAIASNGGGKQALETVQRLLPVLCQAH

SEQ ID NO: 221 - protein, 68 aa, Artificial Sequence
  Synthetic Sequence
GLTPDQVVAIASNIGGKQALETVQRLLPVLCQDHGLTPDQVVAIASHDGGKQALETVQRLLPVLCQDH

SEQ ID NO: 222 - protein, 68 aa, Artificial Sequence
  Synthetic Sequence
GLTPAQVVAIASNIGGKQALETVQRLLPVLCQAHGLTPAQVVAIASNNGGKQALETVQRLLPVLCQAH

SEQ ID NO: 223 - protein, 68 aa, Artificial Sequence
  Synthetic Sequence
GLTPDQVVAIASNNGGKQALETVQRLLPVLCQDHGLTPAQVVAIASNIGGKQALETVQRLLPVLCQAH

SEQ ID NO: 224 - protein, 68 aa, Artificial Sequence; identical to SEQ ID NO: 215
  Synthetic Sequence

SEQ ID NO: 225 - protein, 68 aa, Artificial Sequence
  Synthetic Sequence
GLTPAQVVAIASNIGGKQALETVQRLLPVLCQAHGLTPAQVVAIASHDGGKQALETVQRLLPVLCQDH

SEQ ID NO: 226 - protein, 34 aa, Artificial Sequence
  Synthetic Sequence
GLTPAQVVAIASHDGGKQALETVQRLLPVLCQAH

SEQ ID NO: 227 - protein, 68 aa, Artificial Sequence
  Synthetic Sequence
NLTPDQVVAIASNGGGKQALETVQRLLPVLCQAHGLTPDQVVAIASNIGGKQALETVQRLLPVLCQDH

SEQ ID NO: 228 - protein, 68 aa, Artificial Sequence
  Synthetic Sequence
GLTPDQVVAIASNGGGKQALETVQRLLPVLCQAHGLTPEQVVAIASNGGGKQALETVQRLLPVLCQAH

SEQ ID NO: 229 - protein, 68 aa, Artificial Sequence
  Synthetic Sequence
GLTPAQVVAIASNNGGKQALETVQRLLPVLCQDHGLTPDQVVAIASNNGGKQALETVQRLLPVLCQDH

SEQ ID NO: 230 - protein, 68 aa, Artificial Sequence
  Synthetic Sequence
GLTPAQVVAIASNGGGKQALETVQRLLPVLCQAHGLTPEQVVAIASNGGGKQALETVQRLLPVLCQAH

SEQ ID NO: 231 - protein, 68 aa, Artificial Sequence
  Synthetic Sequence
GLTPDQVVAIASNIGGKQALETVQRLLPVLCQAHGLTPAQVVAIASHDGGKQALETVQRLLPVLCQDH

SEQ ID NO: 232 - protein, 68 aa, Artificial Sequence
  Synthetic Sequence
GLTPDQVVAIASNGGGKQALETVQRLLPVLCQAHGLTPDQVVAIASNIGGKQALETVQRLLPVLCQDH

SEQ ID NO: 233 - protein, 68 aa, Artificial Sequence; identical to SEQ ID NO: 232
  Synthetic Sequence

SEQ ID NO: 234 - protein, 68 aa, Artificial Sequence; identical to SEQ ID NO: 206
  Synthetic Sequence

SEQ ID NO: 235 - protein, 34 aa, Artificial Sequence
  Synthetic Sequence
GLTPDQVVAIASNNGGKQALETVQRLLPVLCQDH

SEQ ID NO: 236 - protein, 68 aa, Artificial Sequence
  Synthetic Sequence
NLTPEQVVAIASNGGGKQALETVQRLLPVLCQAHGLTPAQVVAIASNIGGKQALETVQRLLPVLCQDH

SEQ ID NO: 237 - protein, 68 aa, Artificial Sequence
  Synthetic Sequence
GLTPAQVVAIASNIGGKQALETVQRLLPVLCQAHGLTPDQVVAIASNIGGKQALETVQRLLPVLCQAH

SEQ ID NO: 238 - protein, 68 aa, Artificial Sequence
  Synthetic Sequence
GLTPAQVVAIASNIGGKQALETVQRLLPVLCQDHGLTPAQVVAIASNIGGKQALETVQRLLPVLCQAH

SEQ ID NO: 239 - protein, 68 aa, Artificial Sequence
  Synthetic Sequence
GLTPEQVVAIASNIGGKQALETVQRLLPVLCQAHGLTPAQVVAIASNGGGKQALETVQRLLPVLCQAH

SEQ ID NO: 240 - protein, 68 aa, Artificial Sequence
  Synthetic Sequence
GLTPAQVVAIASNNGGKQALETVQRLLPVLCQAHGLTPAQVVAIASNIGGKQALETVQRLLPVLCQDH

SEQ ID NO: 241 - protein, 68 aa, Artificial Sequence; identical to SEQ ID NO: 181
  Synthetic Sequence

SEQ ID NO: 242 - protein, 68 aa, Artificial Sequence
  Synthetic Sequence
GLTPAQVVAIASHDGGKQALETVQRLLPVLCQAHGLTPDQVVAIASHDGGKQALETVQRLLPVLCQDH

SEQ ID NO: 243 - protein, 68 aa, Artificial Sequence
  Synthetic Sequence
GLTPDQVVAIASHDGGKQALETVQRLLPVLCQDHGLTPDQVVAIASNIGGKQALETVQRLLPVLCQAH

SEQ ID NO: 244 - protein, 68 aa, Artificial Sequence; identical to SEQ ID NO: 218
  Synthetic Sequence

SEQ ID NO: 245 - protein, 68 aa, Artificial Sequence
  Synthetic Sequence
GLTPDQVVAIASNIGGKQALETVQRLLPVLCQAHGLTPDQVVAIASNIGGKQALETVQRLLPVLCQAH

SEQ ID NO: 246 - protein, 68 aa, Artificial Sequence; identical to SEQ ID NO: 238
  Synthetic Sequence

SEQ ID NO: 247 - protein, 68 aa, Artificial Sequence; identical to SEQ ID NO: 239
  Synthetic Sequence

SEQ ID NO: 248 - protein, 68 aa, Artificial Sequence; identical to SEQ ID NO: 240
  Synthetic Sequence

SEQ ID NO: 249 - protein, 68 aa, Artificial Sequence; identical to SEQ ID NO: 181
  Synthetic Sequence

SEQ ID NO: 250 - protein, 68 aa, Artificial Sequence
  Synthetic Sequence
GLTPAQVVAIASHDGGKQALETVQRLLPVLCQDHGLTPAQVVAIASHDGGKQALETVQRLLPVLCQAH

SEQ ID NO: 251 - protein, 68 aa, Artificial Sequence
  Synthetic Sequence
GLTPAQVVAIASHDGGKQALETVQRLLPVLCQDHGLTPDQVVAIASNIGGKQALETVQRLLPVLCQAH

SEQ ID NO: 252 - protein, 68 aa, Artificial Sequence
  Synthetic Sequence
NLTPDQVVAIASHDGGKQALETVQRLLPVLCQDHGLTPDQVVAIASNNGGKQALETVQRLLPVLCQDH

SEQ ID NO: 253 - protein, 68 aa, Artificial Sequence; identical to SEQ ID NO: 230
  Synthetic Sequence

SEQ ID NO: 254 - protein, 68 aa, Artificial Sequence
  Synthetic Sequence
GLTPDQVVAIASHDGGKQALETVQRLLPVLCQDHGLTPDQVVAIASNGGGKQALETVQRLLPVLCQAH

SEQ ID NO: 255 - protein, 69 aa, Artificial Sequence
  Synthetic Sequence
GLTPDQVVAIASNNGGKQALETVQRLLPVLCQAHGLTPAQVVAIASNGGGKQALETVQRLLPVLCQDHG

SEQ ID NO: 256 - protein, 67 aa, Artificial Sequence
  Synthetic Sequence
LTPAQVVAIASNIGGKQALETVQRLLPVLCQAHGLTPEQVVAIASNGGGKQALETVQRLLPVLCQAH

SEQ ID NO: 257 - protein, 68 aa, Artificial Sequence; identical to SEQ ID NO: 254
  Synthetic Sequence

SEQ ID NO: 258 - protein, 68 aa, Artificial Sequence
  Synthetic Sequence
GLTPAQVVAIASNNGGKQALETVQRLLPVLCQAHGLTPAQVVAIASNIGGKQALETVQRLLPVLCQAH

SEQ ID NO: 259 - protein, 34 aa, Artificial Sequence
  Synthetic Sequence
GLTPDQVVAIASNNGGKQALETVQRLLPVLCQAH

SEQ ID NO: 260 - protein, 68 aa, Artificial Sequence
  Synthetic Sequence
NLTPDQVVAIASNIGGKQALETVQRLLPVLCQAHGLTPDQVVAIASNIGGKQALETVQRLLPVLCQDH

SEQ ID NO: 261 - protein, 68 aa, Artificial Sequence; identical to SEQ ID NO: 213
  Synthetic Sequence

SEQ ID NO: 262 - protein, 68 aa, Artificial Sequence; identical to SEQ ID NO: 214
  Synthetic Sequence

SEQ ID NO: 263 - protein, 68 aa, Artificial Sequence
  Synthetic Sequence
GLTPEQVVAIASHDGGKQALETVQRLLPVLCQAHGLTPAQVVAIASNNGGKQALETVQRLLPVLCQAH

SEQ ID NO: 264 - protein, 68 aa, Artificial Sequence; identical to SEQ ID NO: 237
  Synthetic Sequence

SEQ ID NO: 265 - protein, 68 aa, Artificial Sequence; identical to SEQ ID NO: 238
  Synthetic Sequence

SEQ ID NO: 266 - protein, 68 aa, Artificial Sequence
  Synthetic Sequence
GLTPDQVVAIASNIGGKQALETVQRLLPVLCQDHGLTPDQVVAIASHDGGKQALETVQRLLPVLCQAH

SEQ ID NO: 267 - protein, 68 aa, Artificial Sequence
  Synthetic Sequence
GLTPAQVVAIASNNGGKQALETVQRLLPVLCQDHGLTPDQVVAIASNIGGKQALETVQRLLPVLCQAH

SEQ ID NO: 268 - DNA, 19 bp, Artificial Sequence
  Synthetic Sequence
catcaatgggcgtggatag

SEQ ID NO: 269 - protein, 136 aa, Artificial Sequence
  Synthetic Sequence
DIADLRTLGYSQQQQEKIKPKVRSTVAQHHEALVGHGFTHAHIVALSQHPAALGTVAVKYQDMIAALPEATHEAIVGVGKQWSGARALEALLTVAGELRGPPLQLDTGQLLKIAKRGGVTAVEAVHAWRNALTGAP

SEQ ID NO: 270 - protein, 137 aa, Artificial Sequence
  Synthetic Sequence
DIADLRTLGYSQQQQEKIKPKVRSTVAQHHEALVGHGFTHAHIVALSQHPAALGTVAVKYQDMIAALPEATHEAIVGVGKRGAGARALEALLTVAGELRGPPLQLDTGQLLKIAKRGGVTAVEAVHAWRNALTGAPL

SEQ ID NO: 271 - protein, 41 aa, Artificial Sequence
  Synthetic Sequence
SIVAQLSRPDPALAALTNDHLVALACLGGRPALDAVKKGLG

SEQ ID NO: 272 - protein, 94 aa, Artificial Sequence; identical to SEQ ID NO: 24
  Synthetic Sequence

SEQ ID NO: 273 - protein, 108 aa, Artificial Sequence; identical to SEQ ID NO: 25
  Synthetic Sequence

SEQ ID NO: 274 - protein, 49 aa, Artificial Sequence
  Synthetic Sequence
MLGFVGRVAAAPASGALRRLTPSASLPPAQLLLRAAPTAVHPVRDYAAQ

SEQ ID NO: 275 - protein, 8 aa, Artificial Sequence
  Synthetic Sequence
DYKDDDDK

SEQ ID NO: 276 - protein, 9 aa, Artificial Sequence
  Synthetic Sequence
YPYDVPDYA

SEQ ID NO: 277 - DNA, 19 bp, Artificial Sequence
  Synthetic Sequence
ttttcctactggtccgatt

SEQ ID NO: 278 - DNA, 19 bp, Artificial Sequence
  Synthetic Sequence
ttgcaggtattaattgctt

SEQ ID NO: 279 - DNA, 20 bp, Artificial Sequence
  Synthetic Sequence
ttccctaaacataaactcat

SEQ ID NO: 280 - DNA, 19 bp, Artificial Sequence
  Synthetic Sequence
ttaaaataaagttattatt

SEQ ID NO: 281 - DNA, 19 bp, Artificial Sequence
  Synthetic Sequence
ttcctaacagggttctact

SEQ ID NO: 282 - DNA, 17 bp, Artificial Sequence
  Synthetic Sequence
ttgttgttggagaatat

SEQ ID NO: 283 - protein, 199 aa, Artificial Sequence
  Synthetic Sequence
MALSRAVCGTSRQLAPVLGYLGSRQKHSLPDYPYDVPDYAGYPYDVPDYAGYPYDVPDYAGIRIQDLRTLGYSQQQQEKIKPKVRSTVAQHHEALVGHGFTHAHIVALSQHPAALGTVAVKYQDMIAALPEATHEAIVGVGKQWSGARALEALLTVAGELRGPPLQLDTGQLLKIAKRGGVTAVEAVHAWRNALTGAPL

SEQ ID NO: 284 - protein, 191 aa, Artificial Sequence
  Synthetic Sequence
MASVLTPLLLRGLTGSARRLPVPRAKIHSLDYKDHDGDYKDHDIDYKDDDDKGIRIQDLRTLGYSQQQQEKIKPKVRSTVAQHHEALVGHGFTHAHIVALSQHPAALGTVAVKYQDMIAALPEATHEAIVGVGKQWSGARALEALLTVAGELRGPPLQLDTGQLLKIAKRGGVTAVEAVHAWRNALTGAPL

SEQ ID NO: 285 - protein, 197 aa, Artificial Sequence
  Synthetic Sequence
GLTPEQVVAIASNGGGKQALESIVAQLSRPDPALAALTNDHLVALACLGGRPALDAVKKGLGGSGSGSYALGPYQISAPQLPAYNGQTVGTFYYVNDAGGLESKVFSSGGSGGSTNLSDIIEKETGKQLVIQESILMLPEEVEEVIGNKPESDILVHTAYDESTDENVMLLTSDAPEYKPWALVIQDSNGENKIKML

SEQ ID NO: 286 - protein, 247 aa, Artificial Sequence
  Synthetic Sequence
GLTPEQVVAIASNGGGKQALESIVAQLSRPDPALAALTNDHLVALACLGGRPALDAVKKGLGGSGSPTPYPNYANAGHVEGQSALFMRDNGISEGLVFHNNPEGTCGFCVNMTETLLPENAKMTVVPPEGAIPVKRGATGETKVFTGNSNSPKSPTKGGCSGGSTNLSDIIEKETGKQLVIQESILMLPEEVEEVIGNKPESDILVHTAYDESTDENVMLLTSDAPEYKPWALVIQDSNGENKIKML

SEQ ID NO: 287 - protein, 261 aa, Artificial Sequence
  Synthetic Sequence
GLTPEQVVAIASNGGGKQALESIVAQLSRPDPALAALTNDHLVALACLGGRPALDAVKKGLGGSGSGSYALGPYQISAPQLPAYNGQTVGTFYYVNDAGGLESKVFSSGGPTPYPNYANAGHVEGQSALFMRDNGISEGLVFHNNPEGTCGFCVNMTETLLPENAKMTVVPPEGSGGSTNLSDIIEKETGKQLVIQESILMLPEEVEEVIGNKPESDILVHTAYDESTDENVMLLTSDAPEYKPWALVIQDSNGENKIKML

SEQ ID NO: 288 - protein, 183 aa, Artificial Sequence
  Synthetic Sequence
GLTPEQVVAIASNGGGKQALESIVAQLSRPDPALAALTNDHLVALACLGGRPALDAVKKGLGGSGSAIPVKRGATGETKVFTGNSNSPKSPTKGGCSGGSTNLSDIIEKETGKQLVIQESILMLPEEVEEVIGNKPESDILVHTAYDESTDENVMLLTSDAPEYKPWALVIQDSNGENKIKML

SEQ ID NO: 289 - protein, 577 aa, Artificial Sequence
  Synthetic Sequence
NLTPDQVVAIASNGGGKQALETVQRLLPVLCQAHGLTPAQVVAIASNGGGKQALETVQRLLPVLCQAHGLTPEQVVAIASNGGGKQALETVQRLLPVLCQAHGLTPDQVVAIASHDGGKQALETVQRLLPVLCQAHGLTPAQVVAIASHDGGKQALETVQRLLPVLCQDHGLTPAQVVAIASNGGGKQALETVQRLLPVLCQDHGLTPEQVVAIASNIGGKQALETVQRLLPVLCQAHGLTPDQVVAIASHDGGKQALETVQRLLPVLCQAHGLTPDQVVAIASNGGGKQALETVQRLLPVLCQAHGLTPAQVVAIASNNGGKQALETVQRLLPVLCQDHGLTPAQVVAIASNNGGKQALETVQRLLPVLCQDHGLTPDQVVAIASNGGGKQALETVQRLLPVLCQAHGLTPAQVVAIASHDGGKQALETVQRLLPVLCQDHGLTPDQVVAIASHDGGKQALETVQRLLPVLCQAHGLTPEQVVAIASNNGGKQALETVQRLLPVLCQAHGLTPEQVVAIASNIGGKQALETVQRLLPVLCQAHGLTPDQVVAIASNGGGKQALETVQRLLPVLCQD

SEQ ID NO: 290 - protein, 577 aa, Artificial Sequence
  Synthetic Sequence
NLTPEQVVAIASNGGGKQALETVQRLLPVLCQAHGLTPAQVVAIASNIGGKQALETVQRLLPVLCQDHGLTPAQVVAIASNIGGKQALETVQRLLPVLCQAHGLTPDQVVAIASNIGGKQALETVQRLLPVLCQAHGLTPDQVVAIASNIGGKQALETVQRLLPVLCQDHGLTPDQVVAIASNGGGKQALETVQRLLPVLCQAHGLTPDQVVAIASNIGGKQALETVQRLLPVLCQAHGLTPAQVVAIASNIGGKQALETVQRLLPVLCQDHGLTPAQVVAIASNIGGKQALETVQRLLPVLCQAHGLTPAQVVAIASNNGGKQALETVQRLLPVLCQDHGLTPEQVVAIASNGGGKQALETVQRLLPVLCQAHGLTPAQVVAIASNGGGKQALETVQRLLPVLCQDHGLTPAQVVAIASNIGGKQALETVQRLLPVLCQAHGLTPDQVVAIASNGGGKQALETVQRLLPVLCQAHGLTPDQVVAIASNGGGKQALETVQRLLPVLCQAHGLTPEQVVAIASNIGGKQALETVQRLLPVLCQAHGLTPDQVVAIASNGGGKQALETVQRLLPVLCQD

SEQ ID NO: 291 - protein, 577 aa, Artificial Sequence
  Synthetic Sequence
NLTPAQVVAIASNGGGKQALETVQRLLPVLCQAHGLTPDQVVAIASNNGGKQALETVQRLLPVLCQAHGLTPAQVVAIASHDGGKQALETVQRLLPVLCQAHGLTPAQVVAIASNIGGKQALETVQRLLPVLCQAHGLTPAQVVAIASNNGGKQALETVQRLLPVLCQDHGLTPAQVVAIASNNGGKQALETVQRLLPVLCQAHGLTPDQVVAIASNGGGKQALETVQRLLPVLCQAHGLTPDQVVAIASNIGGKQALETVQRLLPVLCQDHGLTPDQVVAIASNGGGKQALETVQRLLPVLCQAHGLTPEQVVAIASNGGGKQALETVQRLLPVLCQAHGLTPAQVVAIASNIGGKQALETVQRLLPVLCQDHGLTPAQVVAIASNIGGKQALETVQRLLPVLCQAHGLTPEQVVAIASNGGGKQALETVQRLLPVLCQAHGLTPAQVVAIASNGGGKQALETVQRLLPVLCQAHGLTPDQVVAIASNNGGKQALETVQRLLPVLCQDHGLTPDQVVAIASHDGGKQALETVQRLLPVLCQAHGLTPAQVVAIASNGGGKQALETVQRLLPVLCQD

SEQ ID NO: 292 - protein, 577 aa, Artificial Sequence
  Synthetic Sequence
NLTPAQVVAIASNGGGKQALETVQRLLPVLCQDHGLTPAQVVAIASHDGGKQALETVQRLLPVLCQAHGLTPEQVVAIASHDGGKQALETVQRLLPVLCQAHGLTPEQVVAIASNGGGKQALETVQRLLPVLCQAHGLTPAQVVAIASNIGGKQALETVQRLLPVLCQDHGLTPAQVVAIASNIGGKQALETVQRLLPVLCQAHGLTPEQVVAIASHDGGKQALETVQRLLPVLCQAHGLTPAQVVAIASNIGGKQALETVQRLLPVLCQAHGLTPAQVVAIASNNGGKQALETVQRLLPVLCQAHGLTPAQVVAIASNNGGKQALETVQRLLPVLCQDHGLTPAQVVAIASNNGGKQALETVQRLLPVLCQDHGLTPDQVVAIASNGGGKQALETVQRLLPVLCQAHGLTPEQVVAIASNGGGKQALETVQRLLPVLCQAHGLTPDQVVAIASHDGGKQALETVQRLLPVLCQDHGLTPDQVVAIASNGGGKQALETVQRLLPVLCQAHGLTPEQVVAIASNIGGKQALETVQRLLPVLCQAHGLTPAQVVAIASHDGGKQALETVQRLLPVLCQD

SEQ ID NO: 293 - protein, 611 aa, Artificial Sequence
  Synthetic Sequence
NLTPAQVVAIASNGGGKQALETVQRLLPVLCQDHGLTPAQVVAIASHDGGKQALETVQRLLPVLCQAHGLTPEQVVAIASHDGGKQALETVQRLLPVLCQAHGLTPDQVVAIASHDGGKQALETVQRLLPVLCQAHGLTPDQVVAIASNGGGKQALETVQRLLPVLCQDHGLTPAQVVAIASNIGGKQALETVQRLLPVLCQDHGLTPDQVVAIASNIGGKQALETVQRLLPVLCQAHGLTPDQVVAIASNIGGKQALETVQRLLPVLCQAHGLTPAQVVAIASHDGGKQALETVQRLLPVLCQAHGLTPAQVVAIASNIGGKQALETVQRLLPVLCQDHGLTPAQVVAIASNGGGKQALETVQRLLPVLCQDHGLTPDQVVAIASNIGGKQALETVQRLLPVLCQDHGLTPDQVVAIASNIGGKQALETVQRLLPVLCQAHGLTPDQVVAIASNIGGKQALETVQRLLPVLCQAHGLTPAQVVAIASHDGGKQALETVQRLLPVLCQAHGLTPAQVVAIASNGGGKQALETVQRLLPVLCQDHGLTPEQVVAIASHDGGKQALETVQRLLPVLCQAHGLTPAQVVAIASNIGGKQALETVQRLLPVLCQD

SEQ ID NO: 294 - protein, 509 aa, Artificial Sequence
  Synthetic Sequence
NLTPAQVVAIASNGGGKQALETVQRLLPVLCQAHGLTPDQVVAIASNNGGKQALETVQRLLPVLCQAHGLTPAQVVAIASNGGGKQALETVQRLLPVLCQDHGLTPAQVVAIASNGGGKQALETVQRLLPVLCQAHGLTPDQVVAIASNNGGKQALETVQRLLPVLCQAHGLTPAQVVAIASNGGGKQALETVQRLLPVLCQDHGLTPEQVVAIASNGGGKQALETVQRLLPVLCQAHGLTPAQVVAIASNNGGKQALETVQRLLPVLCQDHGLTPDQVVAIASNNGGKQALETVQRLLPVLCQAHGLTPDQVVAIASNIGGKQALETVQRLLPVLCQDHGLTPAQVVAIASNNGGKQALETVQRLLPVLCQDHGLTPAQVVAIASNIGGKQALETVQRLLPVLCQAHGLTPEQVVAIASNIGGKQALETVQRLLPVLCQAHGLTPDQVVAIASNGGGKQALETVQRLLPVLCQDHGLTPDQVVAIASNIGGKQALETVQRLLPVLCQA

SEQ ID NO: 295 - DNA, 28 bp, Artificial Sequence
  Synthetic Sequence
agtggggaccgcatactatgtcaacgac

SEQ ID NO: 296 - DNA, 18 bp, Artificial Sequence
  Synthetic Sequence
gtctgaccgttgtaggcg

SEQ ID NO: 297 - DNA, 30 bp, Artificial Sequence
  Synthetic Sequence
atccaaggttgcatctagcggtgggtccgg

SEQ ID NO: 298 - DNA, 18 bp, Artificial Sequence
  Synthetic Sequence
tccaatcccccggcgtcg

SEQ ID NO: 299 - DNA, 33 bp, Artificial Sequence
  Synthetic Sequence
cagacagtggcaaccttttactatgtcaacgac

SEQ ID NO: 300 - DNA, 18 bp, Artificial Sequence
  Synthetic Sequence
accgttgtaggcggggag

SEQ ID NO: 301 - DNA, 30 bp, Artificial Sequence
  Synthetic Sequence
tccatatcaggcaagtgctccccaactccc

SEQ ID NO: 302 - DNA, 18 bp, Artificial Sequence
  Synthetic Sequence
cccagggcgtaggaacca

SEQ ID NO: 303 - DNA, 36 bp, Artificial Sequence
  Synthetic Sequence
attggaatccgcagttttctctagcggtgggtccgg

SEQ ID NO: 304 - DNA, 18 bp, Artificial Sequence
  Synthetic Sequence
cccccggcgtcgttgaca

SEQ ID NO: 305 - DNA, 36 bp, Artificial Sequence
  Synthetic Sequence
ctctggttcctacgccgcaggtccatatcagattag

SEQ ID NO: 306 - DNA, 36 bp, Artificial Sequence
  Synthetic Sequence
ctaatctgatatggacctgcggcgtaggaaccagag

SEQ ID NO: 307 - DNA, 30 bp, Artificial Sequence
  Synthetic Sequence
atatcagattgcagctccccaactccccgc

SEQ ID NO: 308 - DNA, 18 bp, Artificial Sequence
  Synthetic Sequence
ggacccagggcgtaggaa

SEQ ID NO: 309 - DNA, 24 bp, Artificial Sequence
  Synthetic Sequence
caaggttttcgcaagcggtgggtc

SEQ ID NO: 310 - DNA, 18 bp, Artificial Sequence
  Synthetic Sequence
gattccaatcccccggcg

SEQ ID NO: 311 - DNA, 30 bp, Artificial Sequence
  Synthetic Sequence
ggtcagacagtgggggcattttactatgtc

SEQ ID NO: 312 - DNA, 30 bp, Artificial Sequence
  Synthetic Sequence
gacatagtaaaatgcccccactgtctgacc

SEQ ID NO: 313 - DNA, 28 bp, Artificial Sequence
  Synthetic Sequence
ggtcagacagcagggaccttttactatg

SEQ ID NO: 314 - DNA, 18 bp, Artificial Sequence
  Synthetic Sequence
gttgtaggcggggagttg

SEQ ID NO: 315 - DNA, 25 bp, Artificial Sequence
  Synthetic Sequence
ttttactatgcaaacgacgccgggg

SEQ ID NO: 316 - DNA, 18 bp, Artificial Sequence
  Synthetic Sequence
ggtccccactgtctgacc

SEQ ID NO: 317 - DNA, 42 bp, Artificial Sequence
  Synthetic Sequence
ctctggttccgcagccctgggtccatatcagattagtgctcc

SEQ ID NO: 318 - DNA, 18 bp, Artificial Sequence
  Synthetic Sequence
ccagagccccccaacccc

SEQ ID NO: 319 - DNA, 31 bp, Artificial Sequence
  Synthetic Sequence
cagtggggacctttgcatatgtcaacgacgc

SEQ ID NO: 320 - DNA, 31 bp, Artificial Sequence
  Synthetic Sequence
gcgtcgttgacatatgcaaaggtccccactg

SEQ ID NO: 321 - DNA, 28 bp, Artificial Sequence
  Synthetic Sequence
gaccttttacgcagtcaacgacgccggg

SEQ ID NO: 322 - DNA, 18 bp, Artificial Sequence
  Synthetic Sequence
cccactgtctgaccgttg

SEQ ID NO: 323 - DNA, 36 bp, Artificial Sequence
  Synthetic Sequence
tgtggcttcgcagtgaatatgactgaaacccttctg

SEQ ID NO: 324 - DNA, 32 bp, Artificial Sequence
  Synthetic Sequence
catattcactgcgaagccacaagtaccctctg

SEQ ID NO: 325 - DNA, 36 bp, Artificial Sequence
  Synthetic Sequence
gtgtgaatatgactgcaacccttctgcccgaaaatg

SEQ ID NO: 326 - DNA, 36 bp, Artificial Sequence
  Synthetic Sequence
cattttcgggcagaagggttgcagtcatattcacac

SEQ ID NO: 327 - DNA, 35 bp, Artificial Sequence
  Synthetic Sequence
gaaaatgccgcaatgactgtcgtcccacctgaagg

SEQ ID NO: 328 - DNA, 31 bp, Artificial Sequence
  Synthetic Sequence
gacagtcattgcggcattttcgggcagaagg

SEQ ID NO: 329 - DNA, 32 bp, Artificial Sequence
  Synthetic Sequence
gaaacccttgcacccgaaaatgccaagatgac

SEQ ID NO: 330 - DNA, 40 bp, Artificial Sequence
  Synthetic Sequence
attttcgggtgcaagggtttcagtcatattcacacagaag

SEQ ID NO: 331 - DNA, 32 bp, Artificial Sequence
  Synthetic Sequence
aatgccaaggcaactgtcgtcccacctgaagg

SEQ ID NO: 332 - DNA, 34 bp, Artificial Sequence
  Synthetic Sequence
gacgacagttgccttggcattttcgggcagaagg

SEQ ID NO: 333 - DNA, 34 bp, Artificial Sequence
  Synthetic Sequence
gtgaatatggcagaaacccttctgcccgaaaatg

SEQ ID NO: 334 - DNA, 35 bp, Artificial Sequence
  Synthetic Sequence
aagggtttctgccatattcacacagaagccacaag

SEQ ID NO: 335 - DNA, 35 bp, Artificial Sequence
  Synthetic Sequence
cgaaaatgccaagatggcagtcgtcccacctgaag

SEQ ID NO: 336 - DNA, 35 bp, Artificial Sequence
  Synthetic Sequence
cttcaggtgggacgactgccatcttggcattttcg

SEQ ID NO: 337 - DNA, 36 bp, Artificial Sequence
  Synthetic Sequence
ggtacttgtggcttctgtgcaaatatgactgaaacc

SEQ ID NO: 338 - DNA, 36 bp, Artificial Sequence
  Synthetic Sequence
ggtttcagtcatatttgcacagaagccacaagtacc

SEQ ID NO: 339 - DNA, 35 bp, Artificial Sequence
  Synthetic Sequence
gaaaatgccaagatgactgcagtcccacctgaagg

SEQ ID NO: 340 - DNA, 35 bp, Artificial Sequence
  Synthetic Sequence
ccttcaggtgggactgcagtcatcttggcattttc

SEQ ID NO: 341 - DNA, 35 bp, Artificial Sequence
  Synthetic Sequence
ggcattagcgcagggcttgtgttccataataatcc

SEQ ID NO: 342 - DNA, 42 bp, Artificial Sequence
  Synthetic Sequence
cacaagccctgcgctaatgccgttatctctcataaaaagagc

SEQ ID NO: 343 - DNA, 40 bp, Artificial Sequence
  Synthetic Sequence
gtcagctcttgcaatgagagataacggcattagcgaaggg

SEQ ID NO: 344 - DNA, 18 bp, Artificial Sequence
  Synthetic Sequence
tgcccctcgacgtgcccg

SEQ ID NO: 345 - DNA, 35 bp, Artificial Sequence
  Synthetic Sequence
gggcttgtggcacataataatcctgagggcacctg

SEQ ID NO: 346 - DNA, 32 bp, Artificial Sequence
  Synthetic Sequence
gattattatgtgccacaagcccttcgctaatg

SEQ ID NO: 347 - DNA, 23 bp, Artificial Sequence
  Synthetic Sequence
cattagcgaagcacttgtgttcc

SEQ ID NO: 348 - DNA, 20 bp, Artificial Sequence
  Synthetic Sequence
ccgttatctctcataaaaag

SEQ ID NO: 349 - DNA, 30 bp, Artificial Sequence
  Synthetic Sequence
gcttgtgttcgcaaataatcctgagggcac

SEQ ID NO: 350 - DNA, 18 bp, Artificial Sequence
  Synthetic Sequence
ccttcgctaatgccgtta

SEQ ID NO: 351 - DNA, 23 bp, Artificial Sequence
  Synthetic Sequence
tgagaacgctgcaatgactgtcg

SEQ ID NO: 352 - DNA, 18 bp, Artificial Sequence
  Synthetic Sequence
ggcagaagtgtttcggtc

SEQ ID NO: 353 - DNA, 37 bp, Artificial Sequence
  Synthetic Sequence
tagcgaaggggcagtgttccataataatcctgagggc

SEQ ID NO: 354 - DNA, 35 bp, Artificial Sequence
  Synthetic Sequence
atggaacactgccccttcgctaatgccgttatctc

SEQ ID NO: 355 - DNA, 36 bp, Artificial Sequence
  Synthetic Sequence
agctctttttgcaagagataacggcattagcgaagg

SEQ ID NO: 356 - DNA, 18 bp, Artificial Sequence
  Synthetic Sequence
gactgcccctcgacgtgc

SEQ ID NO: 357 - DNA, 26 bp, Artificial Sequence
  Synthetic Sequence
gaacgctaaagcaactgtcgtaccac

SEQ ID NO: 358 - DNA, 18 bp, Artificial Sequence
  Synthetic Sequence
tcaggcagaagtgtttcg

SEQ ID NO: 359 - DNA, 40 bp, Artificial Sequence
  Synthetic Sequence
cgtcgagggggcatcagctctttttatgagagataacggc

SEQ ID NO: 360 - DNA, 18 bp, Artificial Sequence
  Synthetic Sequence
tgcccggcgttagcgtag

SEQ ID NO: 361 - DNA, 25 bp, Artificial Sequence
  Synthetic Sequence
cgaggggcaggcagctctttttatg

SEQ ID NO: 362 - DNA, 18 bp, Artificial Sequence
  Synthetic Sequence
acgtgcccggcgttagcg

SEQ ID NO: 363 - DNA, 23 bp, Artificial Sequence
  Synthetic Sequence
cgctaaaatggcagtcgtaccac

SEQ ID NO: 364 - DNA, 20 bp, Artificial Sequence
  Synthetic Sequence
ttctcaggcagaagtgtttc

SEQ ID NO: 365 - DNA, 22 bp, Artificial Sequence
  Synthetic Sequence
gccgggcacgcagaggggcagt

SEQ ID NO: 366 - DNA, 26 bp, Artificial Sequence
  Synthetic Sequence
gttagcgtagttaggataaggtgttg

SEQ ID NO: 367 - DNA, 27 bp, Artificial Sequence
  Synthetic Sequence
cgaagggcttgcattccataataatcc

SEQ ID NO: 368 - DNA, 18 bp, Artificial Sequence
  Synthetic Sequence
ctaatgccgttatctctc

SEQ ID NO: 369 - DNA, 23 bp, Artificial Sequence
  Synthetic Sequence
aatgactgtcgcaccacccgaag

SEQ ID NO: 370 - DNA, 20 bp, Artificial Sequence
  Synthetic Sequence
ttagcgttctcaggcagaag

SEQ ID NO: 371 - DNA, 36 bp, Artificial Sequence
  Synthetic Sequence
acaaaggtggcaacaggcaactctaacagtccaaag

SEQ ID NO: 372 - DNA, 36 bp, Artificial Sequence
  Synthetic Sequence
gttgcctgttgccacctttgtctcccctgttgctcc

SEQ ID NO: 373 - DNA, 31 bp, Artificial Sequence
  Synthetic Sequence
caacaggggagacagcagtgttcacaggcaa

SEQ ID NO: 374 - DNA, 31 bp, Artificial Sequence
  Synthetic Sequence
ttgcctgtgaacactgctgtctcccctgttg

SEQ ID NO: 375 - DNA, 36 bp, Artificial Sequence
  Synthetic Sequence
ggagacaaaggtgttcgcaggcaactctaacagtcc

SEQ ID NO: 376 - DNA, 36 bp, Artificial Sequence
  Synthetic Sequence
ggactgttagagttgcctgcgaacacctttgtctcc

SEQ ID NO: 377 - DNA, 34 bp, Artificial Sequence
  Synthetic Sequence
gagacaaaggcattcacaggcaactctaacagtc

SEQ ID NO: 378 - DNA, 33 bp, Artificial Sequence
  Synthetic Sequence
gcctgtgaatgcctttgtctcccctgttgctcc

SEQ ID NO: 379 - protein, 138 aa, Artificial Sequence; identical to SEQ ID NO: 18
  Synthetic Sequence

SEQ ID NO: 380 - DNA, 51 bp, Artificial Sequence
  Synthetic Sequence
cccaagcttgccaccatgggatccggcagctacgccctgggtccgtatcag

SEQ ID NO: 381 - DNA, 49 bp, Artificial Sequence
  Synthetic Sequence
cccgggagtctcgctgccgctgcaaccgcctttggtcgggctcttcggg

SEQ ID NO: 382 - DNA, 110 bp, Artificial Sequence
  Synthetic Sequence
cccgggagtctcgctgccgctgcaaccgcctttggtcgggctcttcgggctgttgctgttaccggtaaacactttggtttcaccggtagcgccgcgcgccactggaatgg

SEQ ID NO: 383 - DNA, 108 bp, Artificial Sequence
  Synthetic Sequence
cccgggagtctcgctgccgctgcaaccgcctttggtcgggctcttcgggctgttgctgttaccggtaaacactttggtttcaccggtagcgccggccttcttcactgg

SEQ ID NO: 384 - DNA, 110 bp, Artificial Sequence
  Synthetic Sequence
cccgggagtctcgctgccgctgcaaccgcctttggtcgggctcttcgggctgttgctgttaccggtaaacactttggtttcaccggtagcgccggccgccactggaatgg

SEQ ID NO: 385 - DNA, 84 bp, Artificial Sequence
  Synthetic Sequence
cccgggagtctcgctgccgctgcaaccgcctttggtcgggctcttcgggctgttgctgttaccggtaaacacggcggtttcacc

SEQ ID NO: 386 - DNA, 58 bp, Artificial Sequence
  Synthetic Sequence
cccgggagtctcgctgccgctgcaaccgcctttggtcgggctggccgggctgttgctg

SEQ ID NO: 387 - DNA, 49 bp, Artificial Sequence
  Synthetic Sequence
cccgggagtctcgctgccgctgcaaccgccggcggtcgggctcttcggg

SEQ ID NO: 388 - DNA, 46 bp, Artificial Sequence
  Synthetic Sequence
ctatgccaatgccggtcatgtggccggtcagagcgccctgttcatg

SEQ ID NO: 389 - DNA, 46 bp, Artificial Sequence
  Synthetic Sequence
catgaacagggcgctctgaccggccacatgaccggcattggcatag

SEQ ID NO: 390 - DNA, 88 bp, Artificial Sequence
  Synthetic Sequence
tgagccagctgggcggcgacagcggcagcgagactcccgggacctcagagtccgccacacccgaaagtggcagctacgccctgggtcc

SEQ ID NO: 391 - DNA, 50 bp, Artificial Sequence
  Synthetic Sequence
aatagggccctctagatgcatgctcgagttagcaaccgcctttggtcggg

SEQ ID NO: 392 - DNA, 50 bp, Artificial Sequence
  Synthetic Sequence
tgaagaaaggtctgggcggatccggcagctacgccctgggtccgtatcag

SEQ ID NO: 393 - DNA, 50 bp, Artificial Sequence
  Synthetic Sequence
tgaagaaaggcctgggtggatccggcagctacgccctgggtccgtatcag

SEQ ID NO: 394 - DNA, 50 bp, Artificial Sequence
  Synthetic Sequence
tcagattagttgagccgccagagcaaccgcctttggtcgggctcttcggg

SEQ ID NO: 395 - DNA, 34 bp, Artificial Sequence
  Synthetic Sequence
tctggcggctcaactaatctgagcgacatcattg

SEQ ID NO: 396 - DNA, 29 bp, Artificial Sequence
  Synthetic Sequence
cagatccgaaaatggatatacaagctccc

SEQ ID NO: 397 - DNA, 20 bp, Artificial Sequence
  Synthetic Sequence
ggcccagactgagcacgtga

SEQ ID NO: 398 - DNA, 20 bp, Artificial Sequence
  Synthetic Sequence
ggccacactagcgttgctgc

SEQ ID NO: 399 - DNA, 20 bp, Artificial Sequence
  Synthetic Sequence
gccatagatggtggaccgaa

SEQ ID NO: 400 - DNA, 20 bp, Artificial Sequence
  Synthetic Sequence
ccatctatggctctcggctg

SEQ ID NO: 401 - DNA, 20 bp, Artificial Sequence
  Synthetic Sequence
ccgcagccgagagccataga

SEQ ID NO: 402 - DNA, 20 bp, Artificial Sequence
  Synthetic Sequence
ggaatcccttctgcagcacc

SEQ ID NO: 403 - DNA, 20 bp, Artificial Sequence
  Synthetic Sequence
cttgccccacagggcagtaa

SEQ ID NO: 404 - DNA, 20 bp, Artificial Sequence
  Synthetic Sequence
tgcccctccctccctggccc

SEQ ID NO: 405 - DNA, 20 bp, Artificial Sequence
  Synthetic Sequence
ccctggcccaggtgaaggtg

SEQ ID NO: 406 - DNA, 21 bp, Artificial Sequence
  Synthetic Sequence
gtgaaggtgtggttccagaac

SEQ ID NO: 407 - DNA, 20 bp, Artificial Sequence
  Synthetic Sequence
aaagtacaaacggcagaagc

SEQ ID NO: 408 - DNA, 21 bp, Artificial Sequence
  Synthetic Sequence
gtggtagcggaactcactaag

SEQ ID NO: 409 - DNA, 20 bp, Artificial Sequence
  Synthetic Sequence
cacccagcctgctctgcctt

SEQ ID NO: 410 - protein, 434 aa, Artificial Sequence
  Synthetic Sequence
MLGFVGRVAAAPASGALRRLTPSASLPPAQLLLRAAPTAVHPVRDYAAQDYKDDDDKVDEMTKKFGTLTIHDTEKAAEFGIRIPGEKPFQCRICMRNFSDSGNLRVHIRTHTGEKPYKCPDCGKSFSQSSSLIRHQRTHTGEKPYECDHCGKSFSQSSHLNVHKRTHTGEKPYRCKYCDRSFSISSNLQRHVRNIHLRSGTPHEVGVYTLSGTPHEVGVYTLAIPVKRGATGETKVFTGNSNSPKSPTKGGCSGSETPGTSESATPESSEVEFSHEYWMRHALTLAKRARDEREVPVGAVLVLNNRVIGEGWNRAIGLHDPTAHAEIMALRQGGLVMQNYRLIDATLYVTFEPCVMCAGAMIHSRIGRVVFGVRNSKRGAAGSLMNVLNYPGMNHRVEITEGILADECAALLCDFYRMPRQVFNAQKKAQSSIN

SEQ ID NO: 411 - protein, 339 aa, Artificial Sequence
  Synthetic Sequence
MLGFVGRVAAAPASGALRRLTPSASLPPAQLLLRAAPTAVHPVRDYAAQDYKDDDDKVDEMTKKFGTLTIHDTEKAAEFGIRIPGEKPFQCRICMRNFSDSGNLRVHIRTHTGEKPYKCPDCGKSFSQSSSLIRHQRTHTGEKPYECDHCGKSFSQSSHLNVHKRTHTGEKPYRCKYCDRSFSISSNLQRHVRNIHLRSGTPHEVGVYTLSGTPHEVGVYTLAIPVKRGATGETKVFTGNSNSPKSPTKGGCSGGSTNLSDIIEKETGKQLVIQESILMLPEEVEEVIGNKPESDILVHTAYDESTDENVMLLTSDAPEYKPWALVIQDSNGENKIKML

SEQ ID NO: 412 - protein, 419 aa, Artificial Sequence
  Synthetic Sequence
MLGFVGRVAAAPASGALRRLTPSASLPPAQLLLRAAPTAVHPVRDYAAQYPYDVPDYAVDEMTKKFGTLTIHDTEKAAEFGIHGVPAAMGGSYALGPYQISAPQLPAYNGQTVGTFYYVNDAGGLESKVFSSGGPTPYPNYANAGHVEGQSALFMRDNGISEGLVFHNNPEGTCGFCVNMTETLLPENAKMTVVPPEGSGTPHEVGVYTLSGTPHEVGVYTLYKCPECGKSFSTKNSLTEHQRTHTGEKPYKCPECGKSFSSKKALTEHQRTHTGEKPYECNYCGKTFSVSSTLIRHQRIHTGEKPYRCKYCDRSFSISSNLQRHVRNIHLRSGGSTNLSDIIEKETGKQLVIQESILMLPEEVEEVIGNKPESDILVHTAYDESTDENVMLLTSDAPEYKPWALVIQDSNGENKIKML

SEQ ID NO: 413 - protein, 380 aa, Artificial Sequence
  Synthetic Sequence
MAPKKKRKVGIHGVPAAMGGSYALGPYQISAPQLPAYNGQTVGTFYYVNDAGGLESKVFSSGGPTPYPNYANAGHVEGQSALFMRDNGISEGLVFHNNPEGTCGFCVNMTETLLPENAKMTVVPPEGSGTPHEVGVYTLSGTPHEVGVYTLFQCRICMRKFATSGSLTRHTKIHTGEKPFQCRICMRNFSRSDHLSTHIRTHTGEKPFACDICGRKFATSSNRTKHTKIHTHPRAPIPKPFQCRICMRNFSRSDNLSEHIRTHTGEKPFACDICGRKFAWHSSLRVHTKIHLRSGGSTNLSDIIEKETGKQLVIQESILMLPEEVEEVIGNKPESDILVHTAYDESTDENVMLLTSDAPEYKPWALVIQDSNGENKIKML

SEQ ID NO: 414 - protein, 396 aa, Artificial Sequence
  Synthetic Sequence
MAPKKKRKVGIHGVPAAMAERPFQCRICMRNFSRSDHLSTHIRTHTGEKPFACDICGRKFADRSHLARHTKIHTGSQKPFQCRICMRKFALKQHLNEHTKIHTGEKPFQCRICMRNFSQSGNLARHIRTHTGEKPFACDICGRKFAHNSSLKDHTKIHLRSGTPHEVGVYTLSGTPHEVGVYTLAIPVKRGATGETKVFTGNSNSPKSPTKGGCSGSETPGTSESATPESSEVEFSHEYWMRHALTLAKRARDEREVPVGAVLVLNNRVIGEGWNRAIGLHDPTAHAEIMALRQGGLVMQNYRLIDATLYVTFEPCVMCAGAMIHSRIGRVVFGVRNSKRGAAGSLMNVLNYPGMNHRVEITEGILADECAALLCDFYRMPRQVFNAQKKAQSSIN

SEQ ID NO: 415 - protein, 911 aa, Artificial Sequence
  Synthetic Sequence
MALSRAVCGTSRQLAPVLGYLGSRQKHSLPDYPYDVPDYAGYPYDVPDYAGYPYDVPDYAGIRIQDLRTLGYSQQQQEKIKPKVRSTVAQHHEALVGHGFTHAHIVALSQHPAALGTVAVKYQDMIAALPEATHEAIVGVGKQWSGARALEALLTVAGELRGPPLQLDTGQLLKIAKRGGVTAVEAVHAWRNALTGAPLNLTPDQVVAIASHDGGKQALETVQRLLPVLCQAHGLTPDQVVAIASNGGGKQALETVQRLLPVLCQDHGLTPAQVVAIASNIGGKQALETVQRLLPVLCQDHGLTPDQVVAIASNNGGKQALETVQRLLPVLCQAHGLTPDQVVAIASHDGGKQALETVQRLLPVLCQDHGLTPDQVVAIASHDGGKQALETVQRLLPVLCQAHGLTPAQVVAIASNGGGKQALETVQRLLPVLCQDHGLTPAQVVAIASNIGGKQALETVQRLLPVLCQAHGLTPDQVVAIASNNGGKQALETVQRLLPVLCQAHGLTPAQVVAIASHDGGKQALETVQRLLPVLCQDHGLTPDQVVAIASHDGGKQALETVQRLLPVLCQAHGLTPEQVVAIASNNGGKQALETVQRLLPVLCQAHGLTPAQVVAIASNGGGKQALETVQRLLPVLCQAHGLTPAQVVAIASNGGGKQALETVQRLLPVLCQAHGLTPEQVVAIASNGGGKQALESIVAQLSRPDPALAALLVGSGSYALGPYQISAPQLPAYNGQTVGTFYYVNDAGGLESKVFSSGGPTPYPNYANAGHVEGQSALFMRDNGISEGLVFHNNPEGTCGFCVNMTETLLPENAKMTVVPPEGSGGSTNLSDIIEKETGKQLVIQESILMLPEEVEEVIGNKPESDILVHTAYDESTDENVMLLTSDAPEYKPWALVIQDSNGENKIKML

SEQ ID NO: 416 - protein, 833 aa, Artificial Sequence
  Synthetic Sequence
MALSRAVCGTSRQLAPVLGYLGSRQKHSLPDYPYDVPDYAGYPYDVPDYAGYPYDVPDYAGIRIQDLRTLGYSQQQQEKIKPKVRSTVAQHHEALVGHGFTHAHIVALSQHPAALGTVAVKYQDMIAALPEATHEAIVGVGKQWSGARALEALLTVAGELRGPPLQLDTGQLLKIAKRGGVTAVEAVHAWRNALTGAPLNLTPDQVVAIASHDGGKQALETVQRLLPVLCQAHGLTPDQVVAIASNGGGKQALETVQRLLPVLCQDHGLTPAQVVAIASNIGGKQALETVQRLLPVLCQDHGLTPDQVVAIASNNGGKQALETVQRLLPVLCQAHGLTPDQVVAIASHDGGKQALETVQRLLPVLCQDHGLTPDQVVAIASHDGGKQALETVQRLLPVLCQAHGLTPAQVVAIASNGGGKQALETVQRLLPVLCQDHGLTPAQVVAIASNIGGKQALETVQRLLPVLCQAHGLTPDQVVAIASNNGGKQALETVQRLLPVLCQAHGLTPAQVVAIASHDGGKQALETVQRLLPVLCQDHGLTPDQVVAIASHDGGKQALETVQRLLPVLCQAHGLTPEQVVAIASNNGGKQALETVQRLLPVLCQAHGLTPAQVVAIASNGGGKQALETVQRLLPVLCQAHGLTPAQVVAIASNGGGKQALETVQRLLPVLCQAHGLTPEQVVAIASNGGGKQALESIVAQLSRPDPALAALLVGSAIPVKRGATGETKVFTGNSNSPKSPTKGGCSGGSTNLSDIIEKETGKQLVIQESILMLPEEVEEVIGNKPESDILVHTAYDESTDENVMLLTSDAPEYKPWALVIQDSNGENKIKML

SEQ ID NO: 417 - protein, 1005 aa, Artificial Sequence
  Synthetic Sequence
MASVLTPLLLRGLTGSARRLPVPRAKIHSLDYKDHDGDYKDHDIDYKDDDDKGIRIQDLRTLGYSQQQQEKIKPKVRSTVAQHHEALVGHGFTHAHIVALSQHPAALGTVAVKYQDMIAALPEATHEAIVGVGKQWSGARALEALLTVAGELRGPPLQLDTGQLLKIAKRGGVTAVEAVHAWRNALTGAPLNLTPDQVVAIASNNGGKQALETVQRLLPVLCQDHGLTPAQVVAIASNIGGKQALETVQRLLPVLCQAHGLTPEQVVAIASNNGGKQALETVQRLLPVLCQAHGLTPDQVVAIASNGGGKQALETVQRLLPVLCQAHGLTPAQVVAIASNGGGKQALETVQRLLPVLCQAHGLTPEQVVAIASNGGGKQALETVQRLLPVLCQAHGLTPAQVVAIASNNGGKQALETVQRLLPVLCQDHGLTPAQVVAIASNIGGKQALETVQRLLPVLCQAHGLTPEQVVAIASNGGGKQALETVQRLLPVLCQAHGLTPDQVVAIASNNGGKQALETVQRLLPVLCQAHGLTPAQVVAIASHDGGKQALETVQRLLPVLCQDHGLTPDQVVAIASNGGGKQALETVQRLLPVLCQAHGLTPDQVVAIASHDGGKQALETVQRLLPVLCQAHGLTPDQVVAIASNIGGKQALETVQRLLPVLCQAHGLTPAQVVAIASHDGGKQALETVQRLLPVLCQAHGLTPAQVVAIASHDGGKQALETVQRLLPVLCQDHGLTPAQVVAIASHDGGKQALETVQRLLPVLCQAHGLTPEQVVAIASNGGGKQALESIVAQLSRPDPALAALLVGSGSYALGPYQISAPQLPAYNGQTVGTFYYVNDAGGLESKVFSSGGPTPYPNYANAGHVEGQSALFMRDNGISEGLVFHNNPEGTCGFCVNMTETLLPENAKMTVVPPEGSGGSTNLSDIIEKETGKQLVIQESILMLPEEVEEVIGNKPESDILVHTAYDESTDENVMLLTSDAPEYKPWALVIQDSNGENKIKML

SEQ ID NO: 418 - protein, 927 aa, Artificial Sequence
  Synthetic Sequence
MASVLTPLLLRGLTGSARRLPVPRAKIHSLDYKDHDGDYKDHDIDYKDDDDKGIRIQDLRTLGYSQQQQEKIKPKVRSTVAQHHEALVGHGFTHAHIVALSQHPAALGTVAVKYQDMIAALPEATHEAIVGVGKQWSGARALEALLTVAGELRGPPLQLDTGQLLKIAKRGGVTAVEAVHAWRNALTGAPLNLTPDQVVAIASNNGGKQALETVQRLLPVLCQDHGLTPAQVVAIASNIGGKQALETVQRLLPVLCQAHGLTPEQVVAIASNNGGKQALETVQRLLPVLCQAHGLTPDQVVAIASNGGGKQALETVQRLLPVLCQAHGLTPAQVVAIASNGGGKQALETVQRLLPVLCQAHGLTPEQVVAIASNGGGKQALETVQRLLPVLCQAHGLTPAQVVAIASNNGGKQALETVQRLLPVLCQDHGLTPAQVVAIASNIGGKQALETVQRLLPVLCQAHGLTPEQVVAIASNGGGKQALETVQRLLPVLCQAHGLTPDQVVAIASNNGGKQALETVQRLLPVLCQAHGLTPAQVVAIASHDGGKQALETVQRLLPVLCQDHGLTPDQVVAIASNGGGKQALETVQRLLPVLCQAHGLTPDQVVAIASHDGGKQALETVQRLLPVLCQAHGLTPDQVVAIASNIGGKQALETVQRLLPVLCQAHGLTPAQVVAIASHDGGKQALETVQRLLPVLCQAHGLTPAQVVAIASHDGGKQALETVQRLLPVLCQDHGLTPAQVVAIASHDGGKQALETVQRLLPVLCQAHGLTPEQVVAIASNGGGKQALESIVAQLSRPDPALAALLVGSAIPVKRGATGETKVFTGNSNSPKSPTKGGCSGGSTNLSDIIEKETGKQLVIQESILMLPEEVEEVIGNKPESDILVHTAYDESTDENVMLLTSDAPEYKPWALVIQDSNGENKIKML

SEQ ID NO: 419 - protein, 988 aa, Artificial Sequence
  Synthetic Sequence
MALSRAVCGTSRQLAPVLGYLGSRQKHSLPDYPYDVPDYAGYPYDVPDYAGYPYDVPDYAMDIADLRTLGYSQQQQEKIKPKVRSTVAQHHEALVGHGFTHAHIVALSQHPAALGTVAVKYQDMIAALPEATHEAIVGVGKQWSGARALEALLTVAGELRGPPLQLDTGQLLKIAKRGGVTAVEAVHAWRNALTGAPLNLTPEQVVAIASNNGGKQALETVQALLPVLCQAHGLTPQQVVAIASHDGGKQALETVQRLLPVLCQAHGLTPQQVVAIASNGGGKQALETVQRLLPVLCQAHGLTPEQVVAIASNIGGKQALETVQALLPVLCQAHGLTPEQVVAIASNNGGKQALETVQALLPVLCQAHGLTPEQVVAIASNGGGKQALETVQALLPVLCQAHGLTPEQVVAIASNIGGKQALETVQRLLPVLCQAHGLTPEQVVAIASNIGGKQALETVQALLPVLCQAHGLTPEQVVAIASHDGGKQALETVQRLLPVLCQAHGLTPEQVVAIASHDGGKQALETVQALLPVLCQAHGLTPEQVVAIASNIGGKQALETVQALLPVLCQAHGLTPEQVVAIASHDGGKQALETVQALLPVLCQAHGLTPEQVVAIASNNGGKQALETVQRLLPVLCQAHGLTPQQVVAIASNGGGKQALETVQRLLPVLCQAHGLTPEQVVAIASNGGGKQALETVQALLPVLCQAHGLTPEQVVAIASHDGGKQALETVQALLPVLCQAHGLTPQQVVAIASNGGGRPALESIVAQLSRPDPALAALTNDHLVALACLGGRPALDAVKKGLGGSSGSETPGTSESATPESSEVEFSHEYWMRHALTLAKRARDEREVPVGAVLVLNNRVIGEGWNRAIGLHDPTAHAEIMALRQGGLVMQNYRLIDATLYVTFEPCVMCAGAMIHSRIGRVVFGVRNSKRGAAGSLMNVLNYPGMNHRVEITEGILADECAALLCDFYRMPRQVFNAQKKAQSSIN

SEQ ID NO: 420 - protein, 980 aa, Artificial Sequence
  Synthetic Sequence
MASVLTPLLLRGLTGSARRLPVPRAKIHSLDYKDHDGDYKDHDIDYKDDDDKMDIADLRTLGYSQQQQEKIKPKVRSTVAQHHEALVGHGFTHAHIVALSQHPAALGTVAVKYQDMIAALPEATHEAIVGVGKQWSGARALEALLTVAGELRGPPLQLDTGQLLKIAKRGGVTAVEAVHAWRNALTGAPLNLTPEQVVAIASHDGGKQALETVQALLPVLCQAHGLTPQQVVAIASHDGGKQALETVQRLLPVLCQAHGLTPQQVVAIASNGGGKQALETVQRLLPVLCQAHGLTPEQVVAIASNNGGKQALETVQALLPVLCQAHGLTPEQVVAIASNGGGKQALETVQALLPVLCQAHGLTPEQVVAIASNIGGKQALETVQALLPVLCQAHGLTPEQVVAIASNIGGKQALETVQRLLPVLCQAHGLTPEQVVAIASNNGGKQALETVQALLPVLCQAHGLTPEQVVAIASNGGGKQALETVQRLLPVLCQAHGLTPEQVVAIASNIGGKQALETVQRLLPVLCQAHGLTPEQVVAIASNNGGKQALETVQALLPVLCQAHGLTPEQVVAIASNNGGKQALETVQALLPVLCQAHGLTPEQVVAIASNIGGKQALETVQALLPVLCQAHGLTPEQVVAIASNNGGKQALETVQRLLPVLCQAHGLTPQQVVAIASNIGGKQALETVQRLLPVLCQAHGLTPQQVVAIASNNGGKQALETVQRLLPVLCQAHGLTPQQVVAIASNGGGRPALESIVAQLSRPDPALAALTNDHLVALACLGGRPALDAVKKGLGGSSGSETPGTSESATPESSEVEFSHEYWMRHALTLAKRARDEREVPVGAVLVLNNRVIGEGWNRAIGLHDPTAHAEIMALRQGGLVMQNYRLIDATLYVTFEPCVMCAGAMIHSRIGRVVFGVRNSKRGAAGSLMNVLNYPGMNHRVEITEGILADECAALLCDFYRMPRQVFNAQKKAQSSIN

SEQ ID NO: 421 - protein, 942 aa, Artificial Sequence
  Synthetic Sequence
MALSRAVCGTSRQLAPVLGYLGSRQKHSLPDYPYDVPDYAGYPYDVPDYAGYPYDVPDYAGIRIQDLRTLGYSQQQQEKIKPKVRSTVAQHHEALVGHGFTHAHIVALSQHPAALGTVAVKYQDMIAALPEATHEAIVGVGKQWSGARALEALLTVAGELRGPPLQLDTGQLLKIAKRGGVTAVEAVHAWRNALTGAPLNLTPDQVVAIASHDGGKQALETVQRLLPVLCQAHGLTPDQVVAIASNGGGKQALETVQRLLPVLCQDHGLTPAQVVAIASNIGGKQALETVQRLLPVLCQDHGLTPDQVVAIASNNGGKQALETVQRLLPVLCQAHGLTPDQVVAIASHDGGKQALETVQRLLPVLCQDHGLTPDQVVAIASHDGGKQALETVQRLLPVLCQAHGLTPAQVVAIASNGGGKQALETVQRLLPVLCQDHGLTPAQVVAIASNIGGKQALETVQRLLPVLCQAHGLTPDQVVAIASNNGGKQALETVQRLLPVLCQAHGLTPAQVVAIASHDGGKQALETVQRLLPVLCQDHGLTPDQVVAIASHDGGKQALETVQRLLPVLCQAHGLTPEQVVAIASNNGGKQALETVQRLLPVLCQAHGLTPAQVVAIASNGGGKQALETVQRLLPVLCQAHGLTPAQVVAIASNGGGKQALETVQRLLPVLCQAHGLTPEQVVAIASNGGGKQALESIVAQLSRPDPALAALLVGSGSYALGPYQISAPQLPAYNGQTVGTFYYVNDAGGLESKVFSSGGSGSETPGTSESATPESSEVEFSHEYWMRHALTLAKRARDEREVPVGAVLVLNNRVIGEGWNRAIGLHDPTAHAEIMALRQGGLVMQNYRLIDATLYVTFEPCVMCAGAMIHSRIGRVVFGVRNSKRGAAGSLMNVLNYPGMNHRVEITEGILADECAALLCDFYRMPRQVFNAQKKAQSSIN

SEQ ID NO: 422 - protein, 992 aa, Artificial Sequence
  Synthetic Sequence
MALSRAVCGTSRQLAPVLGYLGSRQKHSLPDYPYDVPDYAGYPYDVPDYAGYPYDVPDYAGIRIQDLRTLGYSQQQQEKIKPKVRSTVAQHHEALVGHGFTHAHIVALSQHPAALGTVAVKYQDMIAALPEATHEAIVGVGKQWSGARALEALLTVAGELRGPPLQLDTGQLLKIAKRGGVTAVEAVHAWRNALTGAPLNLTPDQVVAIASHDGGKQALETVQRLLPVLCQAHGLTPDQVVAIASNGGGKQALETVQRLLPVLCQDHGLTPAQVVAIASNIGGKQALETVQRLLPVLCQDHGLTPDQVVAIASNNGGKQALETVQRLLPVLCQAHGLTPDQVVAIASHDGGKQALETVQRLLPVLCQDHGLTPDQVVAIASHDGGKQALETVQRLLPVLCQAHGLTPAQVVAIASNGGGKQALETVQRLLPVLCQDHGLTPAQVVAIASNIGGKQALETVQRLLPVLCQAHGLTPDQVVAIASNNGGKQALETVQRLLPVLCQAHGLTPAQVVAIASHDGGKQALETVQRLLPVLCQDHGLTPDQVVAIASHDGGKQALETVQRLLPVLCQAHGLTPEQVVAIASNNGGKQALETVQRLLPVLCQAHGLTPAQVVAIASNGGGKQALETVQRLLPVLCQAHGLTPAQVVAIASNGGGKQALETVQRLLPVLCQAHGLTPEQVVAIASNGGGKQALESIVAQLSRPDPALAALLVGSPTPYPNYANAGHVEGQSALFMRDNGISEGLVFHNNPEGTCGFCVNMTETLLPENAKMTVVPPEGAIPVKRGATGETKVFTGNSNSPKSPTKGGCSGSETPGTSESATPESSEVEFSHEYWMRHALTLAKRARDEREVPVGAVLVLNNRVIGEGWNRAIGLHDPTAHAEIMALRQGGLVMQNYRLIDATLYVTFEPCVMCAGAMIHSRIGRVVFGVRNSKRGAAGSLMNVLNYPGMNHRVEITEGILADECAALLCDFYRMPRQVFNAQKKAQSSIN

SEQ ID NO: 423 - protein, 1036 aa, Artificial Sequence
  Synthetic Sequence
MASVLTPLLLRGLTGSARRLPVPRAKIHSLDYKDHDGDYKDHDIDYKDDDDKGIRIQDLRTLGYSQQQQEKIKPKVRSTVAQHHEALVGHGFTHAHIVALSQHPAALGTVAVKYQDMIAALPEATHEAIVGVGKQWSGARALEALLTVAGELRGPPLQLDTGQLLKIAKRGGVTAVEAVHAWRNALTGAPLNLTPDQVVAIASNNGGKQALETVQRLLPVLCQDHGLTPAQVVAIASNIGGKQALETVQRLLPVLCQAHGLTPEQVVAIASNNGGKQALETVQRLLPVLCQAHGLTPDQVVAIASNGGGKQALETVQRLLPVLCQAHGLTPAQVVAIASNGGGKQALETVQRLLPVLCQAHGLTPEQVVAIASNGGGKQALETVQRLLPVLCQAHGLTPAQVVAIASNNGGKQALETVQRLLPVLCQDHGLTPAQVVAIASNIGGKQALETVQRLLPVLCQAHGLTPEQVVAIASNGGGKQALETVQRLLPVLCQAHGLTPDQVVAIASNNGGKQALETVQRLLPVLCQAHGLTPAQVVAIASHDGGKQALETVQRLLPVLCQDHGLTPDQVVAIASNGGGKQALETVQRLLPVLCQAHGLTPDQVVAIASHDGGKQALETVQRLLPVLCQAHGLTPDQVVAIASNIGGKQALETVQRLLPVLCQAHGLTPAQVVAIASHDGGKQALETVQRLLPVLCQAHGLTPAQVVAIASHDGGKQALETVQRLLPVLCQDHGLTPAQVVAIASHDGGKQALETVQRLLPVLCQAHGLTPEQVVAIASNGGGKQALESIVAQLSRPDPALAALLVGSGSYALGPYQISAPQLPAYNGQTVGTFYYVNDAGGLESKVFSSGGSGSETPGTSESATPESSEVEFSHEYWMRHALTLAKRARDEREVPVGAVLVLNNRVIGEGWNRAIGLHDPTAHAEIMALRQGGLVMQNYRLIDATLYVTFEPCVMCAGAMIHSRIGRVVFGVRNSKRGAAGSLMNVLNYPGMNHRVEITEGILADECAALLCDFYRMPRQVFNAQKKAQSSIN

SEQ ID NO: 424 - protein, 1086 aa, Artificial Sequence
  Synthetic Sequence
MASVLTPLLLRGLTGSARRLPVPRAKIHSLDYKDHDGDYKDHDIDYKDDDDKGIRIQDLRTLGYSQQQQEKIKPKVRSTVAQHHEALVGHGFTHAHIVALSQHPAALGTVAVKYQDMIAALPEATHEAIVGVGKQWSGARALEALLTVAGELRGPPLQLDTGQLLKIAKRGGVTAVEAVHAWRNALTGAPLNLTPDQVVAIASNNGGKQALETVQRLLPVLCQDHGLTPAQVVAIASNIGGKQALETVQRLLPVLCQAHGLTPEQVVAIASNNGGKQALETVQRLLPVLCQAHGLTPDQVVAIASNGGGKQALETVQRLLPVLCQAHGLTPAQVVAIASNGGGKQALETVQRLLPVLCQAHGLTPEQVVAIASNGGGKQALETVQRLLPVLCQAHGLTPAQVVAIASNNGGKQALETVQRLLPVLCQDHGLTPAQVVAIASNIGGKQALETVQRLLPVLCQAHGLTPEQVVAIASNGGGKQALETVQRLLPVLCQAHGLTPDQVVAIASNNGGKQALETVQRLLPVLCQAHGLTPAQVVAIASHDGGKQALETVQRLLPVLCQDHGLTPDQVVAIASNGGGKQALETVQRLLPVLCQAHGLTPDQVVAIASHDGGKQALETVQRLLPVLCQAHGLTPDQVVAIASNIGGKQALETVQRLLPVLCQAHGLTPAQVVAIASHDGGKQALETVQRLLPVLCQAHGLTPAQVVAIASHDGGKQALETVQRLLPVLCQDHGLTPAQVVAIASHDGGKQALETVQRLLPVLCQAHGLTPEQVVAIASNGGGKQALESIVAQLSRPDPALAALLVGSPTPYPNYANAGHVEGQSALFMRDNGISEGLVFHNNPEGTCGFCVNMTETLLPENAKMTVVPPEGAIPVKRGATGETKVFTGNSNSPKSPTKGGCSGSETPGTSESATPESSEVEFSHEYWMRHALTLAKRARDEREVPVGAVLVLNNRVIGEGWNRAIGLHDPTAHAEIMALRQGGLVMQNYRLIDATLYVTFEPCVMCAGAMIHSRIGRVVFGVRNSKRGAAGSLMNVLNYPGMNHRVEITEGILADECAALLCDFYRMPRQVFNAQKKAQSSIN

SEQ ID NO: 425 - protein, 952 aa, Artificial Sequence
  Synthetic Sequence
MALSRAVCGTSRQLAPVLGYLGSRQKHSLPDYPYDVPDYAGYPYDVPDYAGYPYDVPDYAGIRIQDLRTLGYSQQQQEKIKPKVRSTVAQHHEALVGHGFTHAHIVALSQHPAALGTVAVKYQDMIAALPEATHEAIVGVGKQWSGARALEALLTVAGELRGPPLQLDTGQLLKIAKRGGVTAVEAVHAWRNALTGAPLNLTPDQVVAIASHDGGKQALETVQRLLPVLCQAHGLTPDQVVAIASNGGGKQALETVQRLLPVLCQDHGLTPAQVVAIASNIGGKQALETVQRLLPVLCQDHGLTPDQVVAIASNNGGKQALETVQRLLPVLCQAHGLTPDQVVAIASHDGGKQALETVQRLLPVLCQDHGLTPDQVVAIASHDGGKQALETVQRLLPVLCQAHGLTPAQVVAIASNGGGKQALETVQRLLPVLCQDHGLTPAQVVAIASNIGGKQALETVQRLLPVLCQAHGLTPDQVVAIASNNGGKQALETVQRLLPVLCQAHGLTPAQVVAIASHDGGKQALETVQRLLPVLCQDHGLTPDQVVAIASHDGGKQALETVQRLLPVLCQAHGLTPEQVVAIASNNGGKQALETVQRLLPVLCQAHGLTPAQVVAIASNGGGKQALETVQRLLPVLCQAHGLTPAQVVAIASNGGGKQALETVQRLLPVLCQAHGLTPEQVVAIASNGGGKQALESIVAQLSRPDPALAALTNDHLVALACLGGRPALDAVKKGLLVGSAIPVKRGATGETKVFTGNSNSPKSPTKGGCSGSETPGTSESATPESSEVEFSHEYWMRHALTLAKRARDEREVPVGAVLVLNNRVIGEGWNRAIGLHDPTAHAEIMALRQGGLVMQNYRLIDATLYVTFEPCVMCAGAMIHSRIGRVVFGVRNSKRGAAGSLMNVLNYPGMNHRVEITEGILADECAALLCDFYRMPRQVFNAQKKAQSSIN

SEQ ID NO: 426 - protein, 1047 aa, Artificial Sequence
  Synthetic Sequence
MASVLTPLLLRGLTGSARRLPVPRAKIHSLDYKDHDGDYKDHDIDYKDDDDKGIRIQDLRTLGYSQQQQEKIKPKVRSTVAQHHEALVGHGFTHAHIVALSQHPAALGTVAVKYQDMIAALPEATHEAIVGVGKQWSGARALEALLTVAGELRGPPLQLDTGQLLKIAKRGGVTAVEAVHAWRNALTGAPLNLTPDQVVAIASNNGGKQALETVQRLLPVLCQDHGLTPAQVVAIASNIGGKQALETVQRLLPVLCQAHGLTPEQVVAIASNNGGKQALETVQRLLPVLCQAHGLTPDQVVAIASNGGGKQALETVQRLLPVLCQAHGLTPAQVVAIASNGGGKQALETVQRLLPVLCQAHGLTPEQVVAIASNGGGKQALETVQRLLPVLCQAHGLTPAQVVAIASNNGGKQALETVQRLLPVLCQDHGLTPAQVVAIASNIGGKQALETVQRLLPVLCQAHGLTPEQVVAIASNGGGKQALETVQRLLPVLCQAHGLTPDQVVAIASNNGGKQALETVQRLLPVLCQAHGLTPAQVVAIASHDGGKQALETVQRLLPVLCQDHGLTPDQVVAIASNGGGKQALETVQRLLPVLCQAHGLTPDQVVAIASHDGGKQALETVQRLLPVLCQAHGLTPDQVVAIASNIGGKQALETVQRLLPVLCQAHGLTPAQVVAIASHDGGKQALETVQRLLPVLCQAHGLTPAQVVAIASHDGGKQALETVQRLLPVLCQDHGLTPAQVVAIASHDGGKQALETVQRLLPVLCQAHGLTPEQVVAIASNGGGKQALESIVAQLSRPDPALAALTNDHLVALACLGGRPALDAVKKGLGGSGSAIPVKRGATGETKVFTGNSNSPKSPTKGGCSGSETPGTSESATPESSEVEFSHEYWMRHALTLAKRARDEREVPVGAVLVLNNRVIGEGWNRAIGLHDPTAHAEIMALRQGGLVMQNYRLIDATLYVTFEPCVMCAGAMIHSRIGRVVFGVRNSKRGAAGSLMNVLNYPGMNHRVEITEGILADECAALLCDFYRMPRQVFNAQKKAQSSIN

SEQ ID NO: 427 - protein, 785 aa, Artificial Sequence
  Synthetic Sequence
MALSRAVCGTSRQLAPVLGYLGSRQKHSLPDYPYDVPDYAGYPYDVPDYAGYPYDVPDYAGIRIQDLRTLGYSQQQQEKIKPKVRSTVAQHHEALVGHGFTHAHIVALSQHPAALGTVAVKYQDMIAALPEATHEAIVGVGKQWSGARALEALLTVAGELRGPPLQLDTGQLLKIAKRGGVTAVEAVHAWRNALTGAPLNLTPDQVVAIASHDGGKQALETVQRLLPVLCQAHGLTPDQVVAIASNGGGKQALETVQRLLPVLCQDHGLTPAQVVAIASNIGGKQALETVQRLLPVLCQDHGLTPDQVVAIASNNGGKQALETVQRLLPVLCQAHGLTPDQVVAIASHDGGKQALETVQRLLPVLCQDHGLTPDQVVAIASHDGGKQALETVQRLLPVLCQAHGLTPAQVVAIASNGGGKQALETVQRLLPVLCQDHGLTPAQVVAIASNIGGKQALETVQRLLPVLCQAHGLTPDQVVAIASNNGGKQALETVQRLLPVLCQAHGLTPAQVVAIASHDGGKQALETVQRLLPVLCQDHGLTPDQVVAIASHDGGKQALETVQRLLPVLCQAHGLTPEQVVAIASNNGGKQALETVQRLLPVLCQAHGLTPAQVVAIASNGGGKQALETVQRLLPVLCQAHGLTPAQVVAIASNGGGKQALETVQRLLPVLCQAHGLTPEQVVAIASNGGGKQALESIVAQLSRPDPALAALTNDHLVALACLGGRPALDAVKKGLGGSGSGSYALGPYQISAPQLPAYNGQTVGTFYYVNDAGGLESKVFSSGG

SEQ ID NO: 428 - protein, 835 aa, Artificial Sequence
  Synthetic Sequence
MALSRAVCGTSRQLAPVLGYLGSRQKHSLPDYPYDVPDYAGYPYDVPDYAGYPYDVPDYAGIRIQDLRTLGYSQQQQEKIKPKVRSTVAQHHEALVGHGFTHAHIVALSQHPAALGTVAVKYQDMIAALPEATHEAIVGVGKQWSGARALEALLTVAGELRGPPLQLDTGQLLKIAKRGGVTAVEAVHAWRNALTGAPLNLTPDQVVAIASHDGGKQALETVQRLLPVLCQAHGLTPDQVVAIASNGGGKQALETVQRLLPVLCQDHGLTPAQVVAIASNIGGKQALETVQRLLPVLCQDHGLTPDQVVAIASNNGGKQALETVQRLLPVLCQAHGLTPDQVVAIASHDGGKQALETVQRLLPVLCQDHGLTPDQVVAIASHDGGKQALETVQRLLPVLCQAHGLTPAQVVAIASNGGGKQALETVQRLLPVLCQDHGLTPAQVVAIASNIGGKQALETVQRLLPVLCQAHGLTPDQVVAIASNNGGKQALETVQRLLPVLCQAHGLTPAQVVAIASHDGGKQALETVQRLLPVLCQDHGLTPDQVVAIASHDGGKQALETVQRLLPVLCQAHGLTPEQVVAIASNNGGKQALETVQRLLPVLCQAHGLTPAQVVAIASNGGGKQALETVQRLLPVLCQAHGLTPAQVVAIASNGGGKQALETVQRLLPVLCQAHGLTPEQVVAIASNGGGKQALESIVAQLSRPDPALAALTNDHLVALACLGGRPALDAVKKGLGGSGSPTPYPNYANAGHVEGQSALFMRDNGISEGLVFHNNPEGTCGFCVNMTETLLPENAKMTVVPPEGAIPVKRGATGETKVFTGNSNSPKSPTKGGC

SEQ ID NO: 429 - protein, 849 aa, Artificial Sequence
  Synthetic Sequence
MALSRAVCGTSRQLAPVLGYLGSRQKHSLPDYPYDVPDYAGYPYDVPDYAGYPYDVPDYAGIRIQDLRTLGYSQQQQEKIKPKVRSTVAQHHEALVGHGFTHAHIVALSQHPAALGTVAVKYQDMIAALPEATHEAIVGVGKQWSGARALEALLTVAGELRGPPLQLDTGQLLKIAKRGGVTAVEAVHAWRNALTGAPLNLTPDQVVAIASHDGGKQALETVQRLLPVLCQAHGLTPDQVVAIASNGGGKQALETVQRLLPVLCQDHGLTPAQVVAIASNIGGKQALETVQRLLPVLCQDHGLTPDQVVAIASNNGGKQALETVQRLLPVLCQAHGLTPDQVVAIASHDGGKQALETVQRLLPVLCQDHGLTPDQVVAIASHDGGKQALETVQRLLPVLCQAHGLTPAQVVAIASNGGGKQALETVQRLLPVLCQDHGLTPAQVVAIASNIGGKQALETVQRLLPVLCQAHGLTPDQVVAIASNNGGKQALETVQRLLPVLCQAHGLTPAQVVAIASHDGGKQALETVQRLLPVLCQDHGLTPDQVVAIASHDGGKQALETVQRLLPVLCQAHGLTPEQVVAIASNNGGKQALETVQRLLPVLCQAHGLTPAQVVAIASNGGGKQALETVQRLLPVLCQAHGLTPAQVVAIASNGGGKQALETVQRLLPVLCQAHGLTPEQVVAIASNGGGKQALESIVAQLSRPDPALAALTNDHLVALACLGGRPALDAVKKGLGGSGSGSYALGPYQISAPQLPAYNGQTVGTFYYVNDAGGLESKVFSSGGPTPYPNYANAGHVEGQSALFMRDNGISEGLVFHNNPEGTCGFCVNMTETLLPENAKMTVVPPEG

SEQ ID NO: 430 - protein, 854 aa, Artificial Sequence
  Synthetic Sequence
MASVLTPLLLRGLTGSARRLPVPRAKIHSLDYKDHDGDYKDHDIDYKDDDDKGIRIQDLRTLGYSQQQQEKIKPKVRSTVAQHHEALVGHGFTHAHIVALSQHPAALGTVAVKYQDMIAALPEATHEAIVGVGKQWSGARALEALLTVAGELRGPPLQLDTGQLLKIAKRGGVTAVEAVHAWRNALTGAPLNLTPDQVVAIASNNGGKQALETVQRLLPVLCQDHGLTPAQVVAIASNIGGKQALETVQRLLPVLCQAHGLTPEQVVAIASNNGGKQALETVQRLLPVLCQAHGLTPDQVVAIASNGGGKQALETVQRLLPVLCQAHGLTPAQVVAIASNGGGKQALETVQRLLPVLCQAHGLTPEQVVAIASNGGGKQALETVQRLLPVLCQAHGLTPAQVVAIASNNGGKQALETVQRLLPVLCQDHGLTPAQVVAIASNIGGKQALETVQRLLPVLCQAHGLTPEQVVAIASNGGGKQALETVQRLLPVLCQAHGLTPDQVVAIASNNGGKQALETVQRLLPVLCQAHGLTPAQVVAIASHDGGKQALETVQRLLPVLCQDHGLTPDQVVAIASNGGGKQALETVQRLLPVLCQAHGLTPDQVVAIASHDGGKQALETVQRLLPVLCQAHGLTPDQVVAIASNIGGKQALETVQRLLPVLCQAHGLTPAQVVAIASHDGGKQALETVQRLLPVLCQAHGLTPAQVVAIASHDGGKQALETVQRLLPVLCQDHGLTPAQVVAIASHDGGKQALETVQRLLPVLCQAHGLTPEQVVAIASNGGGKQALESIVAQLSRPDPALAALLVGSGSYALGPYQISAPQLPAYNGQTVGTFYYVNDAGGLESKVFSSGG

SEQ ID NO: 431 - protein, 904 aa, Artificial Sequence
  Synthetic Sequence
MASVLTPLLLRGLTGSARRLPVPRAKIHSLDYKDHDGDYKDHDIDYKDDDDKGIRIQDLRTLGYSQQQQEKIKPKVRSTVAQHHEALVGHGFTHAHIVALSQHPAALGTVAVKYQDMIAALPEATHEAIVGVGKQWSGARALEALLTVAGELRGPPLQLDTGQLLKIAKRGGVTAVEAVHAWRNALTGAPLNLTPDQVVAIASNNGGKQALETVQRLLPVLCQDHGLTPAQVVAIASNIGGKQALETVQRLLPVLCQAHGLTPEQVVAIASNNGGKQALETVQRLLPVLCQAHGLTPDQVVAIASNGGGKQALETVQRLLPVLCQAHGLTPAQVVAIASNGGGKQALETVQRLLPVLCQAHGLTPEQVVAIASNGGGKQALETVQRLLPVLCQAHGLTPAQVVAIASNNGGKQALETVQRLLPVLCQDHGLTPAQVVAIASNIGGKQALETVQRLLPVLCQAHGLTPEQVVAIASNGGGKQALETVQRLLPVLCQAHGLTPDQVVAIASNNGGKQALETVQRLLPVLCQAHGLTPAQVVAIASHDGGKQALETVQRLLPVLCQDHGLTPDQVVAIASNGGGKQALETVQRLLPVLCQAHGLTPDQVVAIASHDGGKQALETVQRLLPVLCQAHGLTPDQVVAIASNIGGKQALETVQRLLPVLCQAHGLTPAQVVAIASHDGGKQALETVQRLLPVLCQAHGLTPAQVVAIASHDGGKQALETVQRLLPVLCQDHGLTPAQVVAIASHDGGKQALETVQRLLPVLCQAHGLTPEQVVAIASNGGGKQALESIVAQLSRPDPALAALLVGSPTPYPNYANAGHVEGQSALFMRDNGISEGLVFHNNPEGTCGFCVNMTETLLPENAKMTVVPPEGAIPVKRGATGETKVFTGNSNSPKSPTKGGC

SEQ ID NO: 432 - protein, 918 aa, Artificial Sequence
  Synthetic Sequence
MASVLTPLLLRGLTGSARRLPVPRAKIHSLDYKDHDGDYKDHDIDYKDDDDKGIRIQDLRTLGYSQQQQEKIKPKVRSTVAQHHEALVGHGFTHAHIVALSQHPAALGTVAVKYQDMIAALPEATHEAIVGVGKQWSGARALEALLTVAGELRGPPLQLDTGQLLKIAKRGGVTAVEAVHAWRNALTGAPLNLTPDQVVAIASNNGGKQALETVQRLLPVLCQDHGLTPAQVVAIASNIGGKQALETVQRLLPVLCQAHGLTPEQVVAIASNNGGKQALETVQRLLPVLCQAHGLTPDQVVAIASNGGGKQALETVQRLLPVLCQAHGLTPAQVVAIASNGGGKQALETVQRLLPVLCQAHGLTPEQVVAIASNGGGKQALETVQRLLPVLCQAHGLTPAQVVAIASNNGGKQALETVQRLLPVLCQDHGLTPAQVVAIASNIGGKQALETVQRLLPVLCQAHGLTPEQVVAIASNGGGKQALETVQRLLPVLCQAHGLTPDQVVAIASNNGGKQALETVQRLLPVLCQAHGLTPAQVVAIASHDGGKQALETVQRLLPVLCQDHGLTPDQVVAIASNGGGKQALETVQRLLPVLCQAHGLTPDQVVAIASHDGGKQALETVQRLLPVLCQAHGLTPDQVVAIASNIGGKQALETVQRLLPVLCQAHGLTPAQVVAIASHDGGKQALETVQRLLPVLCQAHGLTPAQVVAIASHDGGKQALETVQRLLPVLCQDHGLTPAQVVAIASHDGGKQALETVQRLLPVLCQAHGLTPEQVVAIASNGGGKQALESIVAQLSRPDPALAALLVGSGSYALGPYQISAPQLPAYNGQTVGTFYYVNDAGGLESKVFSSGGPTPYPNYANAGHVEGQSALFMRDNGISEGLVFHNNPEGTCGFCVNMTETLLPENAKMTVVPPEG

SEQ ID NO: 433 - protein, 1032 aa, Artificial Sequence
  Synthetic Sequence
MALSRAVCGTSRQLAPVLGYLGSRQKHSLPDYPYDVPDYAGYPYDVPDYAGYPYDVPDYAMDIADLRTLGYSQQQQEKIKPKVRSTVAQHHEALVGHGFTHAHIVALSQHPAALGTVAVKYQDMIAALPEATHEAIVGVGKQWSGARALEALLTVAGELRGPPLQLDTGQLLKIAKRGGVTAVEAVHAWRNALTGAPLNLTPEQVVAIASNNGGKQALETVQALLPVLCQAHGLTPQQVVAIASHDGGKQALETVQRLLPVLCQAHGLTPQQVVAIASNGGGKQALETVQRLLPVLCQAHGLTPEQVVAIASNIGGKQALETVQALLPVLCQAHGLTPEQVVAIASNNGGKQALETVQALLPVLCQAHGLTPEQVVAIASNGGGKQALETVQALLPVLCQAHGLTPEQVVAIASNIGGKQALETVQRLLPVLCQAHGLTPEQVVAIASNIGGKQALETVQALLPVLCQAHGLTPEQVVAIASHDGGKQALETVQRLLPVLCQAHGLTPEQVVAIASHDGGKQALETVQALLPVLCQAHGLTPEQVVAIASNIGGKQALETVQALLPVLCQAHGLTPEQVVAIASHDGGKQALETVQALLPVLCQAHGLTPEQVVAIASNNGGKQALETVQRLLPVLCQAHGLTPQQVVAIASNGGGKQALETVQRLLPVLCQAHGLTPEQVVAIASNGGGKQALETVQALLPVLCQAHGLTPEQVVAIASHDGGKQALETVQALLPVLCQAHGLTPQQVVAIASNGGGRPALESIVAQLSRPDPALAALTNDHLVALACLGGRPALDAVKKGLGGSGSYALGPYQISAPQLPAYNGQTVGTFYYVNDAGGLESKVFSSGGSGSETPGTSESATPESSEVEFSHEYWMRHALTLAKRARDEREVPVGAVLVLNNRVIGEGWNRAIGLHDPTAHAEIMALRQGGLVMQNYRLIDATLYVTFEPCVMCAGAMIHSRIGRVVFGVRNSKRGAAGSLMNVLNYPGMNHRVEITEGILADECAALLCDFYRMPRQVFNAQKKAQSSIN

SEQ ID NO: 434 - protein, 1082 aa, Artificial Sequence
  Synthetic Sequence
MALSRAVCGTSRQLAPVLGYLGSRQKHSLPDYPYDVPDYAGYPYDVPDYAGYPYDVPDYAMDIADLRTLGYSQQQQEKIKPKVRSTVAQHHEALVGHGFTHAHIVALSQHPAALGTVAVKYQDMIAALPEATHEAIVGVGKQWSGARALEALLTVAGELRGPPLQLDTGQLLKIAKRGGVTAVEAVHAWRNALTGAPLNLTPEQVVAIASNNGGKQALETVQALLPVLCQAHGLTPQQVVAIASHDGGKQALETVQRLLPVLCQAHGLTPQQVVAIASNGGGKQALETVQRLLPVLCQAHGLTPEQVVAIASNIGGKQALETVQALLPVLCQAHGLTPEQVVAIASNNGGKQALETVQALLPVLCQAHGLTPEQVVAIASNGGGKQALETVQALLPVLCQAHGLTPEQVVAIASNIGGKQALETVQRLLPVLCQAHGLTPEQVVAIASNIGGKQALETVQALLPVLCQAHGLTPEQVVAIASHDGGKQALETVQRLLPVLCQAHGLTPEQVVAIASHDGGKQALETVQALLPVLCQAHGLTPEQVVAIASNIGGKQALETVQALLPVLCQAHGLTPEQVVAIASHDGGKQALETVQALLPVLCQAHGLTPEQVVAIASNNGGKQALETVQRLLPVLCQAHGLTPQQVVAIASNGGGKQALETVQRLLPVLCQAHGLTPEQVVAIASNGGGKQALETVQALLPVLCQAHGLTPEQVVAIASHDGGKQALETVQALLPVLCQAHGLTPQQVVAIASNGGGRPALESIVAQLSRPDPALAALTNDHLVALACLGGRPALDAVKKGLGGSPTPYPNYANAGHVEGQSALFMRDNGISEGLVFHNNPEGTCGFCVNMTETLLPENAKMTVVPPEGAIPVKRGATGETKVFTGNSNSPKSPTKGGCSGSETPGTSESATPESSEVEFSHEYWMRHALTLAKRARDEREVPVGAVLVLNNRVIGEGWNRAIGLHDPTAHAEIMALRQGGLVMQNYRLIDATLYVTFEPCVMCAGAMIHSRIGRVVFGVRNSKRGAAGSLMNVLNYPGMNHRVEITEGILADECAALLCDFYRMPRQVFNAQKKAQSSIN

SEQ ID NO: 435 - protein, 1020 aa, Artificial Sequence
  Synthetic Sequence
MALSRAVCGTSRQLAPVLGYLGSRQKHSLPDYPYDVPDYAGYPYDVPDYAGYPYDVPDYAMDIADLRTLGYSQQQQEKIKPKVRSTVAQHHEALVGHGFTHAHIVALSQHPAALGTVAVKYQDMIAALPEATHEAIVGVGKQWSGARALEALLTVAGELRGPPLQLDTGQLLKIAKRGGVTAVEAVHAWRNALTGAPLNLTPEQVVAIASNNGGKQALETVQALLPVLCQAHGLTPQQVVAIASHDGGKQALETVQRLLPVLCQAHGLTPQQVVAIASNGGGKQALETVQRLLPVLCQAHGLTPEQVVAIASNIGGKQALETVQALLPVLCQAHGLTPEQVVAIASNNGGKQALETVQALLPVLCQAHGLTPEQVVAIASNGGGKQALETVQALLPVLCQAHGLTPEQVVAIASNIGGKQALETVQRLLPVLCQAHGLTPEQVVAIASNIGGKQALETVQALLPVLCQAHGLTPEQVVAIASHDGGKQALETVQRLLPVLCQAHGLTPEQVVAIASHDGGKQALETVQALLPVLCQAHGLTPEQVVAIASNIGGKQALETVQALLPVLCQAHGLTPEQVVAIASHDGGKQALETVQALLPVLCQAHGLTPEQVVAIASNNGGKQALETVQRLLPVLCQAHGLTPQQVVAIASNGGGKQALETVQRLLPVLCQAHGLTPEQVVAIASNGGGKQALETVQALLPVLCQAHGLTPEQVVAIASHDGGKQALETVQALLPVLCQAHGLTPQQVVAIASNGGGRPALESIVAQLSRPDPALAALTNDHLVALACLGGRPALDAVKKGLGGSGSAIPVKRGATGETKVFTGNSNSPKSPTKGGCSGSETPGTSESATPESSEVEFSHEYWMRHALTLAKRARDEREVPVGAVLVLNNRVIGEGWNRAIGLHDPTAHAEIMALRQGGLVMQNYRLIDATLYVTFEPCVMCAGAMIHSRIGRVVFGVRNSKRGAAGSLMNVLNYPGMNHRVEITEGILADECAALLCDFYRMPRQVFNAQKKAQSSIN

SEQ ID NO: 436 - protein, 1024 aa, Artificial Sequence
  Synthetic Sequence
MASVLTPLLLRGLTGSARRLPVPRAKIHSLDYKDHDGDYKDHDIDYKDDDDKMDIADLRTLGYSQQQQEKIKPKVRSTVAQHHEALVGHGFTHAHIVALSQHPAALGTVAVKYQDMIAALPEATHEAIVGVGKQWSGARALEALLTVAGELRGPPLQLDTGQLLKIAKRGGVTAVEAVHAWRNALTGAPLNLTPEQVVAIASHDGGKQALETVQALLPVLCQAHGLTPQQVVAIASHDGGKQALETVQRLLPVLCQAHGLTPQQVVAIASNGGGKQALETVQRLLPVLCQAHGLTPEQVVAIASNNGGKQALETVQALLPVLCQAHGLTPEQVVAIASNGGGKQALETVQALLPVLCQAHGLTPEQVVAIASNIGGKQALETVQALLPVLCQAHGLTPEQVVAIASNIGGKQALETVQRLLPVLCQAHGLTPEQVVAIASNNGGKQALETVQALLPVLCQAHGLTPEQVVAIASNGGGKQALETVQRLLPVLCQAHGLTPEQVVAIASNIGGKQALETVQRLLPVLCQAHGLTPEQVVAIASNNGGKQALETVQALLPVLCQAHGLTPEQVVAIASNNGGKQALETVQALLPVLCQAHGLTPEQVVAIASNIGGKQALETVQALLPVLCQAHGLTPEQVVAIASNNGGKQALETVQRLLPVLCQAHGLTPQQVVAIASNIGGKQALETVQRLLPVLCQAHGLTPQQVVAIASNNGGKQALETVQRLLPVLCQAHGLTPQQVVAIASNGGGRPALESIVAQLSRPDPALAALTNDHLVALACLGGRPALDAVKKGLGGSGSYALGPYQISAPQLPAYNGQTVGTFYYVNDAGGLESKVFSSGGSGSETPGTSESATPESSEVEFSHEYWMRHALTLAKRARDEREVPVGAVLVLNNRVIGEGWNRAIGLHDPTAHAEIMALRQGGLVMQNYRLIDATLYVTFEPCVMCAGAMIHSRIGRVVFGVRNSKRGAAGSLMNVLNYPGMNHRVEITEGILADECAALLCDFYRMPRQVFNAQKKAQSSIN

SEQ ID NO: 437 - protein, 1074 aa, Artificial Sequence
  Synthetic Sequence
MASVLTPLLLRGLTGSARRLPVPRAKIHSLDYKDHDGDYKDHDIDYKDDDDKMDIADLRTLGYSQQQQEKIKPKVRSTVAQHHEALVGHGFTHAHIVALSQHPAALGTVAVKYQDMIAALPEATHEAIVGVGKQWSGARALEALLTVAGELRGPPLQLDTGQLLKIAKRGGVTAVEAVHAWRNALTGAPLNLTPEQVVAIASHDGGKQALETVQALLPVLCQAHGLTPQQVVAIASHDGGKQALETVQRLLPVLCQAHGLTPQQVVAIASNGGGKQALETVQRLLPVLCQAHGLTPEQVVAIASNNGGKQALETVQALLPVLCQAHGLTPEQVVAIASNGGGKQALETVQALLPVLCQAHGLTPEQVVAIASNIGGKQALETVQALLPVLCQAHGLTPEQVVAIASNIGGKQALETVQRLLPVLCQAHGLTPEQVVAIASNNGGKQALETVQALLPVLCQAHGLTPEQVVAIASNGGGKQALETVQRLLPVLCQAHGLTPEQVVAIASNIGGKQALETVQRLLPVLCQAHGLTPEQVVAIASNNGGKQALETVQALLPVLCQAHGLTPEQVVAIASNNGGKQALETVQALLPVLCQAHGLTPEQVVAIASNIGGKQALETVQALLPVLCQAHGLTPEQVVAIASNNGGKQALETVQRLLPVLCQAHGLTPQQVVAIASNIGGKQALETVQRLLPVLCQAHGLTPQQVVAIASNNGGKQALETVQRLLPVLCQAHGLTPQQVVAIASNGGGRPALESIVAQLSRPDPALAALTNDHLVALACLGGRPALDAVKKGLGGSPTPYPNYANAGHVEGQSALFMRDNGISEGLVFHNNPEGTCGFCVNMTETLLPENAKMTVVPPEGAIPVKRGATGETKVFTGNSNSPKSPTKGGCSGSETPGTSESATPESSEVEFSHEYWMRHALTLAKRARDEREVPVGAVLVLNNRVIGEGWNRAIGLHDPTAHAEIMALRQGGLVMQNYRLIDATLYVTFEPCVMCAGAMIHSRIGRVVFGVRNSKRGAAGSLMNVLNYPGMNHRVEITEGILADECAALLCDFYRMPRQVFNAQKKAQSSIN

SEQ ID NO: 438 - protein, 1012 aa, Artificial Sequence
  Synthetic Sequence
MASVLTPLLLRGLTGSARRLPVPRAKIHSLDYKDHDGDYKDHDIDYKDDDDKMDIADLRTLGYSQQQQEKIKPKVRSTVAQHHEALVGHGFTHAHIVALSQHPAALGTVAVKYQDMIAALPEATHEAIVGVGKQWSGARALEALLTVAGELRGPPLQLDTGQLLKIAKRGGVTAVEAVHAWRNALTGAPLNLTPEQVVAIASHDGGKQALETVQALLPVLCQAHGLTPQQVVAIASHDGGKQALETVQRLLPVLCQAHGLTPQQVVAIASNGGGKQALETVQRLLPVLCQAHGLTPEQVVAIASNNGGKQALETVQALLPVLCQAHGLTPEQVVAIASNGGGKQALETVQALLPVLCQAHGLTPEQVVAIASNIGGKQALETVQALLPVLCQAHGLTPEQVVAIASNIGGKQALETVQRLLPVLCQAHGLTPEQVVAIASNNGGKQALETVQALLPVLCQAHGLTPEQVVAIASNGGGKQALETVQRLLPVLCQAHGLTPEQVVAIASNIGGKQALETVQRLLPVLCQAHGLTPEQVVAIASNNGGKQALETVQALLPVLCQAHGLTPEQVVAIASNNGGKQALETVQALLPVLCQAHGLTPEQVVAIASNIGGKQALETVQALLPVLCQAHGLTPEQVVAIASNNGGKQALETVQRLLPVLCQAHGLTPQQVVAIASNIGGKQALETVQRLLPVLCQAHGLTPQQVVAIASNNGGKQALETVQRLLPVLCQAHGLTPQQVVAIASNGGGRPALESIVAQLSRPDPALAALTNDHLVALACLGGRPALDAVKKGLGGSGSAIPVKRGATGETKVFTGNSNSPKSPTKGGCSGSETPGTSESATPESSEVEFSHEYWMRHALTLAKRARDEREVPVGAVLVLNNRVIGEGWNRAIGLHDPTAHAEIMALRQGGLVMQNYRLIDATLYVTFEPCVMCAGAMIHSRIGRVVFGVRNSKRGAAGSLMNVLNYPGMNHRVEITEGILADECAALLCDFYRMPRQVFNAQKKAQSSIN

SEQ ID NO: 439 - protein, 1038 aa, Artificial Sequence
  Synthetic Sequence
MALSRAVCGTSRQLAPVLGYLGSRQKHSLPDYPYDVPDYAGYPYDVPDYAGYPYDVPDYAGIRIQDLRTLGYSQQQQEKIKPKVRSTVAQHHEALVGHGFTHAHIVALSQHPAALGTVAVKYQDMIAALPEATHEAIVGVGKQWSGARALEALLTVAGELRGPPLQLDTGQLLKIAKRGGVTAVEAVHAWRNALTGAPLNLTPDQVVAIASHDGGKQALETVQRLLPVLCQAHGLTPDQVVAIASNGGGKQALETVQRLLPVLCQDHGLTPAQVVAIASNIGGKQALETVQRLLPVLCQDHGLTPDQVVAIASNNGGKQALETVQRLLPVLCQAHGLTPDQVVAIASHDGGKQALETVQRLLPVLCQDHGLTPDQVVAIASHDGGKQALETVQRLLPVLCQAHGLTPAQVVAIASNGGGKQALETVQRLLPVLCQDHGLTPAQVVAIASNIGGKQALETVQRLLPVLCQAHGLTPDQVVAIASNNGGKQALETVQRLLPVLCQAHGLTPAQVVAIASHDGGKQALETVQRLLPVLCQDHGLTPDQVVAIASHDGGKQALETVQRLLPVLCQAHGLTPEQVVAIASNNGGKQALETVQRLLPVLCQAHGLTPAQVVAIASNGGGKQALETVQRLLPVLCQAHGLTPAQVVAIASNGGGKQALETVQRLLPVLCQAHGLTPEQVVAIASNGGGKQALESIVAQLSRPDPALAALLVSGSETPGTSESATPESSEVEFSHEYWMRHALTLAKRARDEREVPVGAVLVLNNRVIGEGWNRAIGLHDPTAHAEIMALRQGGLVMQNYRLIDATLYVTFEPCVMCAGAMIHSRIGRVVFGVRNSKRGAAGSLMNVLNYPGMNHRVEITEGILADECAALLCDFYRMPRQVFNAQKKAQSSINLVGSGSYALGPYQISAPQLPAYNGQTVGTFYYVNDAGGLEGKVFSSGGPTPYPNYANAGHVESQSALFMRDNGISEGLVFHNNPEGTCGFCVNMTETLLPENAKMTVVPPEGVIPVKRGATGETKVFTGNSNGPKSPTKGGC

SEQ ID NO: 440 - protein, 1038 aa, Artificial Sequence
  Synthetic Sequence
MALSRAVCGTSRQLAPVLGYLGSRQKHSLPDYPYDVPDYAGYPYDVPDYAGYPYDVPDYAGIRIQDLRTLGYSQQQQEKIKPKVRSTVAQHHEALVGHGFTHAHIVALSQHPAALGTVAVKYQDMIAALPEATHEAIVGVGKQWSGARALEALLTVAGELRGPPLQLDTGQLLKIAKRGGVTAVEAVHAWRNALTGAPLNLTPDQVVAIASHDGGKQALETVQRLLPVLCQAHGLTPDQVVAIASNGGGKQALETVQRLLPVLCQDHGLTPAQVVAIASNIGGKQALETVQRLLPVLCQDHGLTPDQVVAIASNNGGKQALETVQRLLPVLCQAHGLTPDQVVAIASHDGGKQALETVQRLLPVLCQDHGLTPDQVVAIASHDGGKQALETVQRLLPVLCQAHGLTPAQVVAIASNGGGKQALETVQRLLPVLCQDHGLTPAQVVAIASNIGGKQALETVQRLLPVLCQAHGLTPDQVVAIASNNGGKQALETVQRLLPVLCQAHGLTPAQVVAIASHDGGKQALETVQRLLPVLCQDHGLTPDQVVAIASHDGGKQALETVQRLLPVLCQAHGLTPEQVVAIASNNGGKQALETVQRLLPVLCQAHGLTPAQVVAIASNGGGKQALETVQRLLPVLCQAHGLTPAQVVAIASNGGGKQALETVQRLLPVLCQAHGLTPEQVVAIASNGGGKQALESIVAQLSRPDPALAALLVSGSETPGTSESATPESSEVEFSHEYWMRHALTLAKRARDEREVPVGAVLVLNNRVIGEGWNRAIGLHDPTAHAEIMALRQGGLVMQNYRLIDATLYVTFEPCVMCAGAMIHSRIGRVVFGVRNSKRGAAGSLMNVLNYPGMNHRVEITEGILADECAALLCDFYRMPRQVFNAQKKAQSSINLVGSGSYALGPYQISAPQLPAYNGQTVGTFYYVNDAGGLESKVFSSGGPTPYPNYANAGHVAGQSALFMRDNGISEGLVFHNNPEGTCGFCVNMTETLLPENAKMTVVPPEGAIPVKRGATGETKVFTGNSNSPKSPTKGGC

SEQ ID NO: 441 - protein, 1038 aa, Artificial Sequence
  Synthetic Sequence
MALSRAVCGTSRQLAPVLGYLGSRQKHSLPDYPYDVPDYAGYPYDVPDYAGYPYDVPDYAGIRIQDLRTLGYSQQQQEKIKPKVRSTVAQHHEALVGHGFTHAHIVALSQHPAALGTVAVKYQDMIAALPEATHEAIVGVGKQWSGARALEALLTVAGELRGPPLQLDTGQLLKIAKRGGVTAVEAVHAWRNALTGAPLNLTPDQVVAIASHDGGKQALETVQRLLPVLCQAHGLTPDQVVAIASNGGGKQALETVQRLLPVLCQDHGLTPAQVVAIASNIGGKQALETVQRLLPVLCQDHGLTPDQVVAIASNNGGKQALETVQRLLPVLCQAHGLTPDQVVAIASHDGGKQALETVQRLLPVLCQDHGLTPDQVVAIASHDGGKQALETVQRLLPVLCQAHGLTPAQVVAIASNGGGKQALETVQRLLPVLCQDHGLTPAQVVAIASNIGGKQALETVQRLLPVLCQAHGLTPDQVVAIASNNGGKQALETVQRLLPVLCQAHGLTPAQVVAIASHDGGKQALETVQRLLPVLCQDHGLTPDQVVAIASHDGGKQALETVQRLLPVLCQAHGLTPEQVVAIASNNGGKQALETVQRLLPVLCQAHGLTPAQVVAIASNGGGKQALETVQRLLPVLCQAHGLTPAQVVAIASNGGGKQALETVQRLLPVLCQAHGLTPEQVVAIASNGGGKQALESIVAQLSRPDPALAALLVSGSETPGTSESATPESSEVEFSHEYWMRHALTLAKRARDEREVPVGAVLVLNNRVIGEGWNRAIGLHDPTAHAEIMALRQGGLVMQNYRLIDATLYVTFEPCVMCAGAMIHSRIGRVVFGVRNSKRGAAGSLMNVLNYPGMNHRVEITEGILADECAALLCDFYRMPRQVFNAQKKAQSSINLVGSGSYALGPYQISAPQLPAYNGQTVGTFYYVNDAGGLESKVFSSGGPTPYPNYANAGHVEGQSALFMRDNGISEGLVFHNNPEGTCGFCVNMTETLLPENAKMTVVPPEGAIPVAAGATGETAVFTGNSNSPASPTAGGC

SEQ ID NO: 442 - protein, 990 aa, Artificial Sequence
  Synthetic Sequence
MASVLTPLLLRGLTGSARRLPVPRAKIHSLDYKDHDGDYKDHDIDYKDDDDKGIRIQDLRTLGYSQQQQEKIKPKVRSTVAQHHEALVGHGFTHAHIVALSQHPAALGTVAVKYQDMIAALPEATHEAIVGVGKQWSGARALEALLTVAGELRGPPLQLDTGQLLKIAKRGGVTAVEAVHAWRNALTGAPLNLTPDQVVAIASNNGGKQALETVQRLLPVLCQDHGLTPAQVVAIASNIGGKQALETVQRLLPVLCQAHGLTPEQVVAIASNNGGKQALETVQRLLPVLCQAHGLTPDQVVAIASNGGGKQALETVQRLLPVLCQAHGLTPAQVVAIASNGGGKQALETVQRLLPVLCQAHGLTPEQVVAIASNGGGKQALETVQRLLPVLCQAHGLTPAQVVAIASNNGGKQALETVQRLLPVLCQDHGLTPAQVVAIASNIGGKQALETVQRLLPVLCQAHGLTPEQVVAIASNGGGKQALETVQRLLPVLCQAHGLTPDQVVAIASNNGGKQALETVQRLLPVLCQAHGLTPAQVVAIASHDGGKQALETVQRLLPVLCQDHGLTPDQVVAIASNGGGKQALETVQRLLPVLCQAHGLTPDQVVAIASHDGGKQALETVQRLLPVLCQAHGLTPDQVVAIASNIGGKQALETVQRLLPVLCQAHGLTPAQVVAIASHDGGKQALETVQRLLPVLCQAHGLTPAQVVAIASHDGGKQALETVQRLLPVLCQDHGLTPAQVVAIASHDGGKQALETVQRLLPVLCQAHGLTPEQVVAIASNGGGKQALESIVAQLSRPDPALAALLVSGSETPGTSESATPESSEVEFSHEYWMRHALTLAKRARDEREVPVGAVLVLNNRVIGEGWNRAIGLHDPTAHAEIMALRQGGLVMQNYRLIDATLYVTFEPCVMCAGAMIHSRIGRVVFGVRNSKRGAAGSLMNVLNYPGMNHRVEITEGILADECAALLCDFYRMPRQVFNAQKKAQSSIN

SEQ ID NO: 443 - protein, 854 aa, Artificial Sequence
  Synthetic Sequence
MALSRAVCGTSRQLAPVLGYLGSRQKHSLPDYPYDVPDYAGYPYDVPDYAGYPYDVPDYAGIRIQDLRTLGYSQQQQEKIKPKVRSTVAQHHEALVGHGFTHAHIVALSQHPAALGTVAVKYQDMIAALPEATHEAIVGVGKQWSGARALEALLTVAGELRGPPLQLDTGQLLKIAKRGGVTAVEAVHAWRNALTGAPLNLTPDQVVAIASHDGGKQALETVQRLLPVLCQAHGLTPDQVVAIASNGGGKQALETVQRLLPVLCQDHGLTPAQVVAIASNIGGKQALETVQRLLPVLCQDHGLTPDQVVAIASNNGGKQALETVQRLLPVLCQAHGLTPDQVVAIASHDGGKQALETVQRLLPVLCQDHGLTPDQVVAIASHDGGKQALETVQRLLPVLCQAHGLTPAQVVAIASNGGGKQALETVQRLLPVLCQDHGLTPAQVVAIASNIGGKQALETVQRLLPVLCQAHGLTPDQVVAIASNNGGKQALETVQRLLPVLCQAHGLTPAQVVAIASHDGGKQALETVQRLLPVLCQDHGLTPDQVVAIASHDGGKQALETVQRLLPVLCQAHGLTPEQVVAIASNNGGKQALETVQRLLPVLCQAHGLTPAQVVAIASNGGGKQALETVQRLLPVLCQAHGLTPAQVVAIASNGGGKQALETVQRLLPVLCQAHGLTPEQVVAIASNGGGKQALESIVAQLSRPDPALAALLVGSGSYALGPYQISAPQLPAYNGQTVGTFYYVNDAGGLEGKVFSSGGPTPYPNYANAGHVESQSALFMRDNGISEGLVFHNNPEGTCGFCVNMTETLLPENAKMTVVPPEGVIPVKRGATGETKVFTGNSNGPKSPTKGGC

SEQ ID NO: 444 - protein, 854 aa, Artificial Sequence
  Synthetic Sequence
MALSRAVCGTSRQLAPVLGYLGSRQKHSLPDYPYDVPDYAGYPYDVPDYAGYPYDVPDYAGIRIQDLRTLGYSQQQQEKIKPKVRSTVAQHHEALVGHGFTHAHIVALSQHPAALGTVAVKYQDMIAALPEATHEAIVGVGKQWSGARALEALLTVAGELRGPPLQLDTGQLLKIAKRGGVTAVEAVHAWRNALTGAPLNLTPDQVVAIASHDGGKQALETVQRLLPVLCQAHGLTPDQVVAIASNGGGKQALETVQRLLPVLCQDHGLTPAQVVAIASNIGGKQALETVQRLLPVLCQDHGLTPDQVVAIASNNGGKQALETVQRLLPVLCQAHGLTPDQVVAIASHDGGKQALETVQRLLPVLCQDHGLTPDQVVAIASHDGGKQALETVQRLLPVLCQAHGLTPAQVVAIASNGGGKQALETVQRLLPVLCQDHGLTPAQVVAIASNIGGKQALETVQRLLPVLCQAHGLTPDQVVAIASNNGGKQALETVQRLLPVLCQAHGLTPAQVVAIASHDGGKQALETVQRLLPVLCQDHGLTPDQVVAIASHDGGKQALETVQRLLPVLCQAHGLTPEQVVAIASNNGGKQALETVQRLLPVLCQAHGLTPAQVVAIASNGGGKQALETVQRLLPVLCQAHGLTPAQVVAIASNGGGKQALETVQRLLPVLCQAHGLTPEQVVAIASNGGGKQALESIVAQLSRPDPALAALLVGSGSYALGPYQISAPQLPAYNGQTVGTFYYVNDAGGLESKVFSSGGPTPYPNYANAGHVAGQSALFMRDNGISEGLVFHNNPEGTCGFCVNMTETLLPENAKMTVVPPEGAIPVKRGATGETKVFTGNSNSPKSPTKGGC

SEQ ID NO: 445 - protein, 854 aa, Artificial Sequence
  Synthetic Sequence
MALSRAVCGTSRQLAPVLGYLGSRQKHSLPDYPYDVPDYAGYPYDVPDYAGYPYDVPDYAGIRIQDLRTLGYSQQQQEKIKPKVRSTVAQHHEALVGHGFTHAHIVALSQHPAALGTVAVKYQDMIAALPEATHEAIVGVGKQWSGARALEALLTVAGELRGPPLQLDTGQLLKIAKRGGVTAVEAVHAWRNALTGAPLNLTPDQVVAIASHDGGKQALETVQRLLPVLCQAHGLTPDQVVAIASNGGGKQALETVQRLLPVLCQDHGLTPAQVVAIASNIGGKQALETVQRLLPVLCQDHGLTPDQVVAIASNNGGKQALETVQRLLPVLCQAHGLTPDQVVAIASHDGGKQALETVQRLLPVLCQDHGLTPDQVVAIASHDGGKQALETVQRLLPVLCQAHGLTPAQVVAIASNGGGKQALETVQRLLPVLCQDHGLTPAQVVAIASNIGGKQALETVQRLLPVLCQAHGLTPDQVVAIASNNGGKQALETVQRLLPVLCQAHGLTPAQVVAIASHDGGKQALETVQRLLPVLCQDHGLTPDQVVAIASHDGGKQALETVQRLLPVLCQAHGLTPEQVVAIASNNGGKQALETVQRLLPVLCQAHGLTPAQVVAIASNGGGKQALETVQRLLPVLCQAHGLTPAQVVAIASNGGGKQALETVQRLLPVLCQAHGLTPEQVVAIASNGGGKQALESIVAQLSRPDPALAALLVGSGSYALGPYQISAPQLPAYNGQTVGTFYYVNDAGGLESKVFSSGGPTPYPNYANAGHVEGQSALFMRDNGISEGLVFHNNPEGTCGFCVNMTETLLPENAKMTVVPPEGAIPVAAGATGETAVFTGNSNSPASPTAGGC

SEQ ID NO: 446 - protein, 647 aa, Artificial Sequence
  Synthetic Sequence
DLRTLGYSQQQQEKIKPKVRSTVAQHHEALVGHGFTHAHIVALSQHPAALGTVAVKYQDMIAALPEATHEAIVGVGKQWSGARALEALLTVAGELRGPPLQLDTGQLLKIAKRGGVTAVEAVHAWRNALTGAPLNLTPDQVVAIASHDGGKQALETVQRLLPVLCQAHGLTPDQVVAIASNGGGKQALETVQRLLPVLCQDHGLTPAQVVAIASNIGGKQALETVQRLLPVLCQDHGLTPDQVVAIASNNGGKQALETVQRLLPVLCQAHGLTPDQVVAIASHDGGKQALETVQRLLPVLCQDHGLTPDQVVAIASHDGGKQALETVQRLLPVLCQAHGLTPAQVVAIASNGGGKQALETVQRLLPVLCQDHGLTPAQVVAIASNIGGKQALETVQRLLPVLCQAHGLTPDQVVAIASNNGGKQALETVQRLLPVLCQAHGLTPAQVVAIASHDGGKQALETVQRLLPVLCQDHGLTPDQVVAIASHDGGKQALETVQRLLPVLCQAHGLTPEQVVAIASNNGGKQALETVQRLLPVLCQAHGLTPAQVVAIASNGGGKQALETVQRLLPVLCQAHGLTPAQVVAIASNGGGKQALETVQRLLPVLCQAHGLTPEQVVAIASNGGGKQALESIVAQLSRPDPALAAL

SEQ ID NO: 447 - protein, 749 aa, Artificial Sequence
  Synthetic Sequence
DLRTLGYSQQQQEKIKPKVRSTVAQHHEALVGHGFTHAHIVALSQHPAALGTVAVKYQDMIAALPEATHEAIVGVGKQWSGARALEALLTVAGELRGPPLQLDTGQLLKIAKRGGVTAVEAVHAWRNALTGAPLNLTPDQVVAIASNNGGKQALETVQRLLPVLCQDHGLTPAQVVAIASNIGGKQALETVQRLLPVLCQAHGLTPEQVVAIASNNGGKQALETVQRLLPVLCQAHGLTPDQVVAIASNGGGKQALETVQRLLPVLCQAHGLTPAQVVAIASNGGGKQALETVQRLLPVLCQAHGLTPEQVVAIASNGGGKQALETVQRLLPVLCQAHGLTPAQVVAIASNNGGKQALETVQRLLPVLCQDHGLTPAQVVAIASNIGGKQALETVQRLLPVLCQAHGLTPEQVVAIASNGGGKQALETVQRLLPVLCQAHGLTPDQVVAIASNNGGKQALETVQRLLPVLCQAHGLTPAQVVAIASHDGGKQALETVQRLLPVLCQDHGLTPDQVVAIASNGGGKQALETVQRLLPVLCQAHGLTPDQVVAIASHDGGKQALETVQRLLPVLCQAHGLTPDQVVAIASNIGGKQALETVQRLLPVLCQAHGLTPAQVVAIASHDGGKQALETVQRLLPVLCQAHGLTPAQVVAIASHDGGKQALETVQRLLPVLCQDHGLTPAQVVAIASHDGGKQALETVQRLLPVLCQAHGLTPEQVVAIASNGGGKQALESIVAQLSRPDPALAAL

SEQ ID NO: 448 - protein, 744 aa, Artificial Sequence
  Synthetic Sequence
MDIADLRTLGYSQQQQEKIKPKVRSTVAQHHEALVGHGFTHAHIVALSQHPAALGTVAVKYQDMIAALPEATHEAIVGVGKQWSGARALEALLTVAGELRGPPLQLDTGQLLKIAKRGGVTAVEAVHAWRNALTGAPLNLTPEQVVAIASNNGGKQALETVQALLPVLCQAHGLTPQQVVAIASHDGGKQALETVQRLLPVLCQAHGLTPQQVVAIASNGGGKQALETVQRLLPVLCQAHGLTPEQVVAIASNIGGKQALETVQALLPVLCQAHGLTPEQVVAIASNNGGKQALETVQALLPVLCQAHGLTPEQVVAIASNGGGKQALETVQALLPVLCQAHGLTPEQVVAIASNIGGKQALETVQRLLPVLCQAHGLTPEQVVAIASNIGGKQALETVQALLPVLCQAHGLTPEQVVAIASHDGGKQALETVQRLLPVLCQAHGLTPEQVVAIASHDGGKQALETVQALLPVLCQAHGLTPEQVVAIASNIGGKQALETVQALLPVLCQAHGLTPEQVVAIASHDGGKQALETVQALLPVLCQAHGLTPEQVVAIASNNGGKQALETVQRLLPVLCQAHGLTPQQVVAIASNGGGKQALETVQRLLPVLCQAHGLTPEQVVAIASNGGGKQALETVQALLPVLCQAHGLTPEQVVAIASHDGGKQALETVQALLPVLCQAHGLTPQQVVAIASNGGGRPALESIVAQLSRPDPALAALTNDHLVALACLGGRPALDAVKKGLG

SEQ ID NO: 449 - protein, 744 aa, Artificial Sequence
  Synthetic Sequence
MDIADLRTLGYSQQQQEKIKPKVRSTVAQHHEALVGHGFTHAHIVALSQHPAALGTVAVKYQDMIAALPEATHEAIVGVGKQWSGARALEALLTVAGELRGPPLQLDTGQLLKIAKRGGVTAVEAVHAWRNALTGAPLNLTPEQVVAIASHDGGKQALETVQALLPVLCQAHGLTPQQVVAIASHDGGKQALETVQRLLPVLCQAHGLTPQQVVAIASNGGGKQALETVQRLLPVLCQAHGLTPEQVVAIASNNGGKQALETVQALLPVLCQAHGLTPEQVVAIASNGGGKQALETVQALLPVLCQAHGLTPEQVVAIASNIGGKQALETVQALLPVLCQAHGLTPEQVVAIASNIGGKQALETVQRLLPVLCQAHGLTPEQVVAIASNNGGKQALETVQALLPVLCQAHGLTPEQVVAIASNGGGKQALETVQRLLPVLCQAHGLTPEQVVAIASNIGGKQALETVQRLLPVLCQAHGLTPEQVVAIASNNGGKQALETVQALLPVLCQAHGLTPEQVVAIASNNGGKQALETVQALLPVLCQAHGLTPEQVVAIASNIGGKQALETVQALLPVLCQAHGLTPEQVVAIASNNGGKQALETVQRLLPVLCQAHGLTPQQVVAIASNIGGKQALETVQRLLPVLCQAHGLTPQQVVAIASNNGGKQALETVQRLLPVLCQAHGLTPQQVVAIASNGGGRPALESIVAQLSRPDPALAALTNDHLVALACLGGRPALDAVKKGLG

SEQ ID NO: 450 - protein, 142 aa, Artificial Sequence
  Synthetic Sequence
FQCRICMRKFATSGSLTRHTKIHTGEKPFQCRICMRNFSRSDHLSTHIRTHTGEKPFACDICGRKFATSSNRTKHTKIHTHPRAPIPKPFQCRICMRNFSRSDNLSEHIRTHTGEKPFACDICGRKFAWHSSLRVHTKIHLR

SEQ ID NO: 451 - protein, 138 aa, Artificial Sequence
  Synthetic Sequence
FQCRICMRNFSRSDHLSTHIRTHTGEKPFACDICGRKFADRSHLARHTKIHTGSQKPFQCRICMRKFALKQHLNEHTKIHTGEKPFQCRICMRNFSQSGNLARHIRTHTGEKPFACDICGRKFAHNSSLKDHTKIHLR

SEQ ID NO: 452 - protein, 110 aa, Artificial Sequence
  Synthetic Sequence
FQCRICMRNFSDSGNLRVHIRTHTGEKPYKCPDCGKSFSQSSSLIRHQRTHTGEKPYECDHCGKSFSQSSHLNVHKRTHTGEKPYRCKYCDRSFSISSNLQRHVRNIHLR

SEQ ID NO: 453 - protein, 110 aa, Artificial Sequence
  Synthetic Sequence
YKCPECGKSFSTKNSLTEHQRTHTGEKPYKCPECGKSFSSKKALTEHQRTHTGEKPYECNYCGKTFSVSSTLIRHQRIHTGEKPYRCKYCDRSFSISSNLQRHVRNIHLR

SEQ ID NO: 454 - protein, 46 aa, Artificial Sequence
  Synthetic Sequence
GSGSYALGPYQISAPQLPAYNGQTVGTFYYVNDAGGLESKVFSSGG

SEQ ID NO: 455 - protein, 96 aa, Artificial Sequence
  Synthetic Sequence
GSPTPYPNYANAGHVEGQSALFMRDNGISEGLVFHNNPEGTCGFCVNMTETLLPENAKMTVVPPEGAIPVKRGATGETKVFTGNSNSPKSPTKGGC

SEQ ID NO: 456 - protein, 110 aa, Artificial Sequence
  Synthetic Sequence
GSGSYALGPYQISAPQLPAYNGQTVGTFYYVNDAGGLESKVFSSGGPTPYPNYANAGHVEGQSALFMRDNGISEGLVFHNNPEGTCGFCVNMTETLLPENAKMTVVPPEG

SEQ ID NO: 457 - protein, 32 aa, Artificial Sequence
  Synthetic Sequence
GSAIPVKRGATGETKVFTGNSNSPKSPTKGGC

SEQ ID NO: 458 - protein, 166 aa, Artificial Sequence
  Synthetic Sequence
SEVEFSHEYWMRHALTLAKRARDEREVPVGAVLVLNNRVIGEGWNRAIGLHDPTAHAEIMALRQGGLVMQNYRLIDATLYVTFEPCVMCAGAMIHSRIGRVVFGVRNSKRGAAGSLMNVLNYPGMNHRVEITEGILADECAALLCDFYRMPRQVFNAQKKAQSSIN

SEQ ID NO: 459 - protein, 140 aa, Artificial Sequence
  Synthetic Sequence
GSGSYALGPYQISAPQLPAYNGQTVGTFYYVNDAGGLEGKVFSSGGPTPYPNYANAGHVESQSALFMRDNGISEGLVFHNNPEGTCGFCVNMTETLLPENAKMTVVPPEGVIPVKRGATGETKVFTGNSNGPKSPTKGGC

SEQ ID NO: 460 - protein, 140 aa, Artificial Sequence
  Synthetic Sequence
GSGSYALGPYQISAPQLPAYNGQTVGTFYYVNDAGGLESKVFSSGGPTPYPNYANAGHVAGQSALFMRDNGISEGLVFHNNPEGTCGFCVNMTETLLPENAKMTVVPPEGAIPVKRGATGETKVFTGNSNSPKSPTKGGC

SEQ ID NO: 461 - protein, 140 aa, Artificial Sequence
  Synthetic Sequence
GSGSYALGPYQISAPQLPAYNGQTVGTFYYVNDAGGLESKVFSSGGPTPYPNYANAGHVEGQSALFMRDNGISEGLVFHNNPEGTCGFCVNMTETLLPENAKMTVVPPEGAIPVAAGATGETAVFTGNSNSPASPTAGGC

SEQ ID NO: 462 - protein, 83 aa, Artificial Sequence
  Synthetic Sequence
TNLSDIIEKETGKQLVIQESILMLPEEVEEVIGNKPESDILVHTAYDESTDENVMLLTSDAPEYKPWALVIQDSNGENKIKML

SEQ ID NO: 463 - protein, 324 aa, Artificial Sequence
  Synthetic Sequence
SGSETPGTSESATPESSEVEFSHEYWMRHALTLAKRARDEREVPVGAVLVLNNRVIGEGWNRAIGLHDPTAHAEIMALRQGGLVMQNYRLIDATLYVTFEPCVMCAGAMIHSRIGRVVFGVRNSKRGAAGSLMNVLNYPGMNHRVEITEGILADECAALLCDFYRMPRQVFNAQKKAQSSINLVGSGSYALGPYQISAPQLPAYNGQTVGTFYYVNDAGGLEGKVFSSGGPTPYPNYANAGHVESQSALFMRDNGISEGLVFHNNPEGTCGFCVNMTETLLPENAKMTVVPPEGVIPVKRGATGETKVFTGNSNGPKSPTKGGC

SEQ ID NO: 464 - protein, 324 aa, Artificial Sequence
  Synthetic Sequence
SGSETPGTSESATPESSEVEFSHEYWMRHALTLAKRARDEREVPVGAVLVLNNRVIGEGWNRAIGLHDPTAHAEIMALRQGGLVMQNYRLIDATLYVTFEPCVMCAGAMIHSRIGRVVFGVRNSKRGAAGSLMNVLNYPGMNHRVEITEGILADECAALLCDFYRMPRQVFNAQKKAQSSINLVGSGSYALGPYQISAPQLPAYNGQTVGTFYYVNDAGGLESKVFSSGGPTPYPNYANAGHVAGQSALFMRDNGISEGLVFHNNPEGTCGFCVNMTETLLPENAKMTVVPPEGAIPVKRGATGETKVFTGNSNSPKSPTKGGC

SEQ ID NO: 465 - protein, 324 aa, Artificial Sequence
  Synthetic Sequence
SGSETPGTSESATPESSEVEFSHEYWMRHALTLAKRARDEREVPVGAVLVLNNRVIGEGWNRAIGLHDPTAHAEIMALRQGGLVMQNYRLIDATLYVTFEPCVMCAGAMIHSRIGRVVFGVRNSKRGAAGSLMNVLNYPGMNHRVEITEGILADECAALLCDFYRMPRQVFNAQKKAQSSINLVGSGSYALGPYQISAPQLPAYNGQTVGTFYYVNDAGGLESKVFSSGGPTPYPNYANAGHVEGQSALFMRDNGISEGLVFHNNPEGTCGFCVNMTETLLPENAKMTVVPPEGAIPVAAGATGETAVFTGNSNSPASPTAGGC

SEQ ID NO: 466 - protein, 182 aa, Artificial Sequence
  Synthetic Sequence
SGSETPGTSESATPESSEVEFSHEYWMRHALTLAKRARDEREVPVGAVLVLNNRVIGEGWNRAIGLHDPTAHAEIMALRQGGLVMQNYRLIDATLYVTFEPCVMCAGAMIHSRIGRVVFGVRNSKRGAAGSLMNVLNYPGMNHRVEITEGILADECAALLCDFYRMPRQVFNAQKKAQSSIN

SEQ ID NO: 467 - protein, 140 aa, Artificial Sequence; identical to SEQ ID NO: 459
  Synthetic Sequence

SEQ ID NO: 468 - protein, 140 aa, Artificial Sequence; identical to SEQ ID NO: 460
  Synthetic Sequence

SEQ ID NO: 469 - protein, 140 aa, Artificial Sequence; identical to SEQ ID NO: 461
  Synthetic Sequence

SEQ ID NO: 470 - protein, 214 aa, Artificial Sequence
  Synthetic Sequence
GSAIPVKRGATGETKVFTGNSNSPKSPTKGGCSGSETPGTSESATPESSEVEFSHEYWMRHALTLAKRARDEREVPVGAVLVLNNRVIGEGWNRAIGLHDPTAHAEIMALRQGGLVMQNYRLIDATLYVTFEPCVMCAGAMIHSRIGRVVFGVRNSKRGAAGSLMNVLNYPGMNHRVEITEGILADECAALLCDFYRMPRQVFNAQKKAQSSIN

SEQ ID NO: 471 - protein, 228 aa, Artificial Sequence
  Synthetic Sequence
GSGSYALGPYQISAPQLPAYNGQTVGTFYYVNDAGGLESKVFSSGGSGSETPGTSESATPESSEVEFSHEYWMRHALTLAKRARDEREVPVGAVLVLNNRVIGEGWNRAIGLHDPTAHAEIMALRQGGLVMQNYRLIDATLYVTFEPCVMCAGAMIHSRIGRVVFGVRNSKRGAAGSLMNVLNYPGMNHRVEITEGILADECAALLCDFYRMPRQVFNAQKKAQSSIN

SEQ ID NO: 472 - protein, 278 aa, Artificial Sequence
  Synthetic Sequence
GSPTPYPNYANAGHVEGQSALFMRDNGISEGLVFHNNPEGTCGFCVNMTETLLPENAKMTVVPPEGAIPVKRGATGETKVFTGNSNSPKSPTKGGCSGSETPGTSESATPESSEVEFSHEYWMRHALTLAKRARDEREVPVGAVLVLNNRVIGEGWNRAIGLHDPTAHAEIMALRQGGLVMQNYRLIDATLYVTFEPCVMCAGAMIHSRIGRVVFGVRNSKRGAAGSLMNVLNYPGMNHRVEITEGILADECAALLCDFYRMPRQVFNAQKKAQSSIN

SEQ ID NO: 473 - protein, 8 aa, Artificial Sequence
  Synthetic Sequence
SGGGLGST

SEQ ID NO: 474 - protein, 16 aa, Artificial Sequence
  Synthetic Sequence
SGSETPGTSESATPES

SEQ ID NO: 475 - protein, 32 aa, Artificial Sequence
  Synthetic Sequence
SGGSSGGSSGSETPGTSESATPESSGGSSGGS

SEQ ID NO: 476 - protein, 60 aa, Artificial Sequence
  Synthetic Sequence
MALSRAVCGTSRQLAPVLGYLGSRQKHSLPDYPYDVPDYAGYPYDVPDYAGYPYDVPDYA

SEQ ID NO: 477 - protein, 52 aa, Artificial Sequence
  Synthetic Sequence
MASVLTPLLLRGLTGSARRLPVPRAKIHSLDYKDHDGDYKDHDIDYKDDDDK

SEQ ID NO: 478 - protein, 7 aa, Artificial Sequence
  Synthetic Sequence
PKKKRKV

SEQ ID NO: 479 - protein, 5 aa, Artificial Sequence
  Synthetic Sequence
TGEKP

SEQ ID NO: 480 - protein, 4 aa, Artificial Sequence
  Synthetic Sequence
SGGS

SEQ ID NO: 481 - protein, 83 aa, Artificial Sequence; identical to SEQ ID NO: 462
  Synthetic Sequence

SEQ ID NO: 482 - protein, 123 aa, Artificial Sequence
  Synthetic Sequence
GIHGVPAAMAERPFQCRICMRNFSQSGDLRRHIRTHTGEKPFACDICGRKFARSDNLSVHTKIHTGSQKPFQCRICMRNFSQKINLQVHIRTHTGEKPFACDICGRKFARSDVLSEHTKIHLR

SEQ ID NO: 483 - protein, 123 aa, Artificial Sequence
  Synthetic Sequence
GIHGVPAAMAERPFQCRICMRNFSDQSNLRAHIRTHTGEKPFACDICGRKFATSSNRKTHTKIHTGSQKPFQCRICMRNFSLQQTLADHIRTHTGEKPFACDICGRKFAQSGNLARHTKIHLR

SEQ ID NO: 484 - protein, 142 aa, Artificial Sequence; identical to SEQ ID NO: 450
  Synthetic Sequence

SEQ ID NO: 485 - protein, 151 aa, Artificial Sequence
  Synthetic Sequence
GIHGVPAAMAERPFQCRICMRNFSRSDHLSTHIRTHTGEKPFACDICGRKFADRSHLARHTKIHTGSQKPFQCRICMRKFALKQHLNEHTKIHTGEKPFQCRICMRNFSQSGNLARHIRTHTGEKPFACDICGRKFAHNSSLKDHTKIHLR

SEQ ID NO: 486 - protein, 118 aa, Artificial Sequence
  Synthetic Sequence
GIRIPGEKPYSCGICGKSFSDSSAKRRHCILHTGEKPYTCSDCGKAFRDKSCLNRHRRTHTGEKPYKCMECGKAFNRRSHLTRHQRIHTGEKPYECNYCGKTFSVSSTLIRHQRIHLR

SEQ ID NO: 487 - protein, 117 aa, Artificial Sequence
  Synthetic Sequence
GIRERPYACPVESCDRRFSTSGSLVRHIRIHTGQKPFQCRICMRNFSRSDELTRHIRTHTGEKPFACDICGRKFARSDHLTTHTKIHTGEKPFQCRICMRKFAQSSNLVRHTKIHLR

SEQ ID NO: 488 - protein, 117 aa, Artificial Sequence
  Synthetic Sequence
GIRERPYACPVESCDRRFSDPGHLVRHIRIHTGQKPFQCRICMRNFSRSDELTRHIRTHTGEKPFACDICGRKFARSDHLTTHTKIHTGEKPFQCRICMRKFARSDKLVRHTKIHLR

SEQ ID NO: 489 - protein, 122 aa, Artificial Sequence
  Synthetic Sequence
GIRIPGEKPYECNYCGKTFSVSSTLIRHQRIHTGEKPYHCDWDGCGWKFARSDELTRHYRKHTGEKPFECKDCGKAFIQKSNLIRHQRTHTGEKPYHCDWDGCGWKFARSDELTRHYRKHLR

SEQ ID NO: 490 - protein, 117 aa, Artificial Sequence
  Synthetic Sequence
GIRERPYACPVESCDRRFSDCRDLARHIRIHTGQKPFQCRICMRNFSRSDELTRHIRTHTGEKPFACDICGRKFARSDHLTTHTKIHTGEKPFQCRICMRKFARSDKLVRHTKIHLR

SEQ ID NO: 491 - protein, 118 aa, Artificial Sequence
  Synthetic Sequence
GIRIPGEKPFECKDCGKAFIQKSNLIRHQRTHTGEKPYRCEECGKAFRWPSNLTRHKRIHTGEKPYRCEECGKAFRWPSNLTRHKRIHTGEKPYSCGICGKSFSDSSAKRRHCILHLR

SEQ ID NO: 492 - protein, 117 aa, Artificial Sequence; identical to SEQ ID NO: 490
  Synthetic Sequence

SEQ ID NO: 493 - protein, 120 aa, Artificial Sequence
  Synthetic Sequence
GIRIPGEKPYTCSDCGKAFRDKSCLNRHRRTHTGEKPYKCGQCGKFYSQVSHLTRHQKIHTGEKPFECKDCGKAFIQKSNLIRHQRTHTGEKPYHCDWDGCGWKFARSDELTRHYRKHLR

SEQ ID NO: 494 - protein, 117 aa, Artificial Sequence
  Synthetic Sequence
GIRERPYACPVESCDRRFSRSDKLVRHIRIHTGQKPFQCRICMRNFSRSDELTRHIRTHTGEKPFACDICGRKFARSDHLTTHTKIHTGEKPFQCRICMRKFARSDKLVRHTKIHLR

SEQ ID NO: 495 - protein, 118 aa, Artificial Sequence
  Synthetic Sequence
GIRIPGEKPYTCSDCGKAFRDKSCLNRHRRTHTGEKPYECNYCGKTFSVSSTLIRHQRIHTGEKPYTCSDCGKAFRDKSCLNRHRRTHTGEKPYTCSDCGKAFRDKSCLNRHRRTHLR

SEQ ID NO: 496 - protein, 117 aa, Artificial Sequence; identical to SEQ ID NO: 494
  Synthetic Sequence

SEQ ID NO: 497 - protein, 118 aa, Artificial Sequence
  Synthetic Sequence
GIRIPGEKPYECNYCGKTFSVSSTLIRHQRIHTGEKPYTCSDCGKAFRDKSCLNRHRRTHTGEKPYTCSDCGKAFRDKSCLNRHRRTHTGEKPYHCDWDGCGWKFARSDELTRHYRKH

SEQ ID NO: 498 - protein, 122 aa, Artificial Sequence
  Synthetic Sequence
GIHGVPAAMAERPFQCRICMRNFSTSGHLVRHIRTHTGEKPFACDICGRKFATSGHLVRHTKIHTGEKPFQCRICMRNFSTSGELVRHIRTHTGEKPFACDICGRKFAQSSNLVRHTKIHLR

SEQ ID NO: 499 - protein, 123 aa, Artificial Sequence; identical to SEQ ID NO: 2
  Synthetic Sequence

SEQ ID NO: 500 - protein, 23 aa, Artificial Sequence
  Synthetic Sequence
FQCRICMRNFSDSGNLRVHIRTH

SEQ ID NO: 501 - protein, 23 aa, Artificial Sequence
  Synthetic Sequence
YKCPECGKSFSTKNSLTEHQRTH

SEQ ID NO: 502 - protein, 23 aa, Artificial Sequence
  Synthetic Sequence
YKCPECGKSFSREDNLHTHQRTH

SEQ ID NO: 503 - protein, 23 aa, Artificial Sequence
  Synthetic Sequence
YECDHCGKSFSQSSHLNVHKRTH

SEQ ID NO: 504 - protein, 23 aa, Artificial Sequence
  Synthetic Sequence
YECHDCGKSFRQSTHLTQHRRIH

SEQ ID NO: 505 - protein, 23 aa, Artificial Sequence
  Synthetic Sequence
YKCPDCGKSFSQSSSLIRHQRTH

SEQ ID NO: 506 - protein, 23 aa, Artificial Sequence
  Synthetic Sequence
YKCPECGKSFSDPGHLVRHQRTH

SEQ ID NO: 507 - protein, 23 aa, Artificial Sequence
  Synthetic Sequence
YGCHLCGKAFSKSSNLRRHEMIH

SEQ ID NO: 508 - protein, 23 aa, Artificial Sequence
  Synthetic Sequence
YKCPECGKSFSDPGHLVRHQRTH

SEQ ID NO: 509 - protein, 23 aa, Artificial Sequence
  Synthetic Sequence
YKCPECGKSFSDPGHLVRHQRTH

SEQ ID NO: 510 - protein, 23 aa, Artificial Sequence
  Synthetic Sequence
FHCGYCEKSFSVKDYLTKHIRTH

SEQ ID NO: 511 - protein, 23 aa, Artificial Sequence
  Synthetic Sequence
FHCGYCEKSFSVKDYLTKHIRTH

SEQ ID NO: 512 - protein, 23 aa, Artificial Sequence
  Synthetic Sequence
FHCGYCEKSFSVKDYLTKHIRTH

SEQ ID NO: 513 - protein, 23 aa, Artificial Sequence
  Synthetic Sequence
FACPECPKRFMRSDNLTQHIKTH

SEQ ID NO: 514 - protein, 23 aa, Artificial Sequence
  Synthetic Sequence
YECHDCGKSFRQSTHLTQHRRIH

SEQ ID NO: 515 - protein, 23 aa, Artificial Sequence
  Synthetic Sequence
YRCEECGKAFRWPSNLTRHKRIH

SEQ ID NO: 516 - protein, 23 aa, Artificial Sequence
  Synthetic Sequence
FECKDCGKAFIQKSNLIRHQRTH

SEQ ID NO: 517 - protein, 23 aa, Artificial Sequence
  Synthetic Sequence
YTCSYCGKSFTQSNTLKQHTRIH

SEQ ID NO: 518 - protein, 23 aa, Artificial Sequence
  Synthetic Sequence
YKCPDCGKSFSQSSSLIRHQRTH

SEQ ID NO: 519 - protein, 23 aa, Artificial Sequence
  Synthetic Sequence
YKCPECGKSFSSKKALTEHQRTH

SEQ ID NO: 520 - protein, 25 aa, Artificial Sequence
  Synthetic Sequence
YHCDWDGCGWKFARSDELTRHYRKH

SEQ ID NO: 521 - protein, 25 aa, Artificial Sequence
  Synthetic Sequence
YHCDWDGCGWKFARSDELTRHYRKH

SEQ ID NO: 522 - protein, 23 aa, Artificial Sequence
  Synthetic Sequence
YSCGICGKSFSDSSAKRRHCILH

SEQ ID NO: 523 - protein, 23 aa, Artificial Sequence
  Synthetic Sequence
YKCGQCGKFYSQVSHLTRHQKIH

SEQ ID NO: 524 - protein, 24 aa, Artificial Sequence
  Synthetic Sequence
YRCKYCDRSFSISSNLQRHVRNIH

SEQ ID NO: 525 - protein, 23 aa, Artificial Sequence
  Synthetic Sequence
FQCKTCQRKFSRSDHLKTHTRTH

SEQ ID NO: 526 - protein, 23 aa, Artificial Sequence
  Synthetic Sequence
YKCPECGKSFSREDNLHTHQRTH

SEQ ID NO: 527 - protein, 23 aa, Artificial Sequence
  Synthetic Sequence
FHCGYCEKSFSVKDYLTKHIRTH

SEQ ID NO: 528 - protein, 23 aa, Artificial Sequence
  Synthetic Sequence
YECVQCGKGFTQSSNLITHQRVH

SEQ ID NO: 529 - protein, 23 aa, Artificial Sequence
  Synthetic Sequence
YKCPECGKSFSTHLDLIRHQRTH

SEQ ID NO: 530 - protein, 23 aa, Artificial Sequence
  Synthetic Sequence
YECDHCGKSFSQSSHLNVHKRTH

SEQ ID NO: 531 - protein, 23 aa, Artificial Sequence
  Synthetic Sequence
YECNYCGKTFSVSSTLIRHQRIH

SEQ ID NO: 532 - protein, 23 aa, Artificial Sequence
  Synthetic Sequence
YECHDCGKSFRQSTHLTQHRRIH

SEQ ID NO: 533 - protein, 23 aa, Artificial Sequence
  Synthetic Sequence
YKCPECGKSFSREDNLHTHQRTH

SEQ ID NO: 534 - protein, 23 aa, Artificial Sequence
  Synthetic Sequence
FHCGYCEKSFSVKDYLTKHIRTH

SEQ ID NO: 535 - protein, 23 aa, Artificial Sequence
  Synthetic Sequence
YKCDECGKNFTQSSNLIVHKRIH

SEQ ID NO: 536 - protein, 23 aa, Artificial Sequence
  Synthetic Sequence
YECDHCGKSFSQSSHLNVHKRTH

SEQ ID NO: 537 - protein, 23 aa, Artificial Sequence
  Synthetic Sequence
YECNYCGKTFSVSSTLIRHQRIH

SEQ ID NO: 538 - protein, 23 aa, Artificial Sequence
  Synthetic Sequence
YKCPECGKSFSREDNLHTHQRTH

SEQ ID NO: 539 - protein, 23 aa, Artificial Sequence
  Synthetic Sequence
YKCPDCGKSFSQSSSLIRHQRTH

SEQ ID NO: 540 - protein, 23 aa, Artificial Sequence
  Synthetic Sequence
YECHDCGKSFRQSTHLTQHRRIH

SEQ ID NO: 541 - protein, 23 aa, Artificial Sequence
  Synthetic Sequence
YKCPDCGKSFSQSSSLIRHQRTH

SEQ ID NO: 542 - protein, 24 aa, Artificial Sequence
  Synthetic Sequence
YRCKYCDRSFSISSNLQRHVRNIH

SEQ ID NO: 543 - protein, 23 aa, Artificial Sequence
  Synthetic Sequence
YKCGQCGKFYSQVSHLTRHQKIH

SEQ ID NO: 544 - protein, 23 aa, Artificial Sequence
  Synthetic Sequence
YKCPECGKSFSREDNLHTHQRTH

SEQ ID NO: 545 - protein, 23 aa, Artificial Sequence
  Synthetic Sequence
YKCPECGKSFSSPADLTRHQRTH

SEQ ID NO: 546 - protein, 23 aa, Artificial Sequence
  Synthetic Sequence
YTCSYCGKSFTQSNTLKQHTRIH

SEQ ID NO: 547 - protein, 23 aa, Artificial Sequence
  Synthetic Sequence
YKCPECGKSFSSKKALTEHQRTH

SEQ ID NO: 548 - protein, 23 aa, Artificial Sequence
  Synthetic Sequence
FQCRICMRNFSDSGNLRVHIRTH

SEQ ID NO: 549 - protein, 23 aa, Artificial Sequence
  Synthetic Sequence
YECDHCGKAFSVSSNLNVHRRIH

SEQ ID NO: 550 - protein, 23 aa, Artificial Sequence
  Synthetic Sequence
YKCGQCGKFYSQVSHLTRHQKIH

SEQ ID NO: 551 - protein, 23 aa, Artificial Sequence
  Synthetic Sequence
YGCHLCGKAFSKSSNLRRHEMIH

SEQ ID NO: 552 - protein, 23 aa, Artificial Sequence
  Synthetic Sequence
YTCSDCGKAFRDKSCLNRHRRTH

SEQ ID NO: 553 - protein, 23 aa, Artificial Sequence
  Synthetic Sequence
YKCPECGKSFSDPGHLVRHQRTH

SEQ ID NO: 554 - protein, 24 aa, Artificial Sequence
  Synthetic Sequence
YRCKYCDRSFSISSNLQRHVRNIH

SEQ ID NO: 555 - protein, 24 aa, Artificial Sequence
  Synthetic Sequence
YRCKYCDRSFSISSNLQRHVRNIH

SEQ ID NO: 556 - protein, 24 aa, Artificial Sequence
  Synthetic Sequence
YRCKYCDRSFSISSNLQRHVRNIH

SEQ ID NO: 557 - protein, 23 aa, Artificial Sequence
  Synthetic Sequence
YKCGQCGKFYSQVSHLTRHQKIH

SEQ ID NO: 558 - protein, 23 aa, Artificial Sequence
  Synthetic Sequence
YKCPDCGKSFSQSSSLIRHQRTH

SEQ ID NO: 559 - protein, 23 aa, Artificial Sequence
  Synthetic Sequence
YECDHCGKSFSQSSHLNVHKRTH

SEQ ID NO: 560 - protein, 23 aa, Artificial Sequence
  Synthetic Sequence
YKCPECGKSFSREDNLHTHQRTH

SEQ ID NO: 561 - protein, 23 aa, Artificial Sequence
  Synthetic Sequence
YKCPECGKSFSREDNLHTHQRTH

SEQ ID NO: 562 - protein, 24 aa, Artificial Sequence
  Synthetic Sequence
YRCKYCDRSFSDSSNLQRHVRNIH

SEQ ID NO: 563 - protein, 23 aa, Artificial Sequence
  Synthetic Sequence
FQCRICMRNFSDSGNLRVHIRTH

SEQ ID NO: 564 - protein, 24 aa, Artificial Sequence
  Synthetic Sequence
YRCKYCDRSFSISSNLQRHVRNIH

SEQ ID NO: 565 - protein, 23 aa, Artificial Sequence
  Synthetic Sequence
FQCRICMRNFSDSGNLRVHIRTH

SEQ ID NO: 566 - protein, 23 aa, Artificial Sequence
  Synthetic Sequence
YECDHCGKSFSQSSHLNVHKRTH

SEQ ID NO: 567 - protein, 23 aa, Artificial Sequence
  Synthetic Sequence
YECDHCGKAFSVSSNLNVHRRIH

SEQ ID NO: 568 - protein, 25 aa, Artificial Sequence
  Synthetic Sequence
YHCDWDGCGWKFARSDELTRHYRKH

SEQ ID NO: 569 - protein, 23 aa, Artificial Sequence
  Synthetic Sequence
YKCPECGKSFSREDNLHTHQRTH

SEQ ID NO: 570 - protein, 23 aa, Artificial Sequence
  Synthetic Sequence
YTCSYCGKSFTQSNTLKQHTRIH

SEQ ID NO: 571 - protein, 23 aa, Artificial Sequence
  Synthetic Sequence
YECDHCGKSFSQSSHLNVHKRTH